European Patent Application EP 4 438 736 A1, published October 2, 2024. Title: NOVEL METHOD FOR PRODUCING ECTOINE. Applicant: 350 PPM Biotech GmbH. Application EP. The sequence listing filed with the application follows.

SEQUENCE LISTING (35 sequences)

SEQ ID NO: 1 - DNA, 1402 bp, Hydrogenovibrio marinus
  source 1..1402: mol_type = genomic DNA
agagtttgatcctggctcagaatgaacgctggcggcaggcttaacacatgcaagtcgaacggtaacaggagaaagcttgctttcttgctgacgagtggcggacgggtgagtaatgtatgggaatctgccctctagttggggacaacatatggaaacgtatgctaataccgaatgtgatctacggattaaaggtgccctctccttggaaggtatcgctagaggatgagcccatattagattagctagttggtagggtaaaggcctaccaaggcgacgatctatagctggtttgagaggatgatcagccacactgggactgagacacggcccagactcctacgggaggcagcagtggggaatattgcacaatgagggaaaccttgatgcagccatgccgcgtgtgtgaagaaggcctgagggttgtaaagcactttcaattgtgaggaaagctaagtagttaatacctgcttagtgtgacgttaactttagaagaagcaccggctaactctgtgccagcagccgcggtaatacagagggtgcaagcgttattcggaattactgggcgtaaagcgcgcgtaggcggactgttaagtcggttgtgaaagccctgggctcaacctaggaattgcatccgatactggcaatctagagtttaagagagggaaggggaattccaggtgtagcagtgaaatgcgtagatatctggaggaacatcagtggcgaaggcgccttcctggcttaaaactgacgctgaggtgcgaaagcgtgggtagcgaacgggattagataccccggtagtccacgccgtaaacgatgtcaactagctgttggccttattaaaaaggttagtagcgcagctaacgcgataagttgaccgcctggggagtacggtcgcaagattaaaactcaaaggaattgacgggggcccgcacaagcggtggagcatgtggtttaattcgatgcaacgcgaagaaccttaccatcccttgacatcctgcgaactttctagagatagattggtgccttcgggaacgcagtgacaggtgctgcatggctgtcgtcagctcgtgtcgtgagatgttgggttaagtcccgcaacgagcgcaacccttatctttagttgctaccatttagttgagaactctaaagagactgccggtgataaaccggaggaaggcggggacgacgtcaagtcatcatggcccttatgggatgggctacacacgtgctacaatggggggtacaaagagcagctagctggcgacagtgcgcgaatctcataaaacccttcgtagtccggattggagtctgcaactcgactccatgaagtcggaatcgctagtaatcgtgaatcagaatgtcacggtgaatacgttcccgggccttgtacacaccgcccgtc

SEQ ID NO: 2 - DNA, 8410 bp, synthetic construct
  source 1..8410: mol_type = other DNA
agtcctcgtctcgccctcgaattagcccgcttaatgagcgggctttttttgaattaattctcgcgagctggcacgacaggtttcccgactggaaagcgggcagtgagcgcaacgcaattaatgtaagttagcgcgaattgcaagctggccgacgcgctgggctacgtcttgctggcgttcgggagcagaagagcatacatctggaagcaaagccaggaaagcggcctatggagctgtgcggcagcgctcagtaggcaatttttcaaaatattgttaagccttttctgagcatggtatttttcatggtattaccaattagcaggaaaataagccattgaatataaaagataaaaatgtcttgtttacaatagagtggggggggtcagcctgccgccttgggccgggtgatgtcgtacttgcccgccgcgaactcggttaccgtccagcccagcgcgaccagctccggcaacgcctcgcgcacccgctggcggcgcttgcgcatggtcgaaccactggcctctgacggccagacatagccgcacaaggtatctatggaagccttgccggttttgccggggtcgatccagccacacagccgctggtgcagcaggcgggcggtttcgctgtccagcgcccgcacctcgtccatgctgatgcgcacatgctggccgccacccatgacggcctgcgcgatcaaggggttcagggccacgtacaggcgcccgtccgcctcgtcgctggcgtactccgacagcagccgaaacccctgccgcttgcggccattctgggcgatgatggataccttccaaaggcgctcgatgcagtcctgtatgtgcttgagcgccccaccactatcgacctctgccccgatttcctttgccagcgcccgatagctacctttgaccaccatggcatcagcggtgacggcctcccacttgggttccaggaacagccggagctgccgtccgccttcggtcttgggttccgggccaagcactaggccattaggcccagccatggccaccagcccttgcaggatgcgcagatcatcagcgcccagcggctccgggccgctgaactcgatccgcttgccgtcgccgtagtcatacgtcacgtccagcttgctgcgcttgcgctcgccccgcttgagggcacggaacaggccgggggccagacagtgcgccgggtcgtgtcggacgtggctgaggctgtgcttgttcttaggcttcaccacggggcacccccttgctcttgcgctgcctctccagcacggcgggcttgagcaccccgccgtcatgccgcctgaaccaccgatcagcgaacggtgcgccatagttggccttgctcacaccgaagcggacgaagaaccggcgctggtcgtcgtccacaccccattcctcggcctcggcgctggtcatgctcgacaggtaggactgccagcggatgttatcgaccagtaccgagctgccccggctggcctgctgctggtcgcctgcgcccatcatggccgcgcccttgctggcatggtgcaggaacacgatagagcacccggtatcggcggcgatggcctccatgcgaccgatgacctgggccatggggccgctggcgttttcttcctcgatgtggaaccggcgcagcgtgtccagcaccatcaggcggcggccctcggcggcgcgcttgaggccgtcgaaccactccggggccatgatgttgggcaggctgccgatcagcggctggatcagcaggccgtcagccacggcttgccgttcctcggcgctgaggtgcgccccaagggcgtgcaggcggtgatgaatggcggtgggcgggtcttcggcgggcaggtagatcaccgggccggtgggcagttcgcccacctccagcagatccggcccgcctgcaatctgtgcggccagttgcagggccagcatggatttaccggcaccaccgggcgacaccagcgccccgaccgtaccggccaccatgttgggcaaaacgtagtccagcggtggcggcgctgctgcgaacgcctccagaatattgataggcttatgggtagccattgattgcctcctttgcaggcagttggtggttaggcgctggcggggtcactacccccgccctgcgccgctctgagttcttccaggcactcgcgcagcgcctcgtattcgtcgtcggtcagccagaacttgcgctgacgcatccctttggccttcatgcgctcggcatatcgcgcttggcgtacagcgtcagggctggccagcaggtcgccggtctgcttgtccttttggtctttcatatcagtcaccgagaaacttgccggggccgaaaggcttgtcttcgcggaacaaggacaaggtgcagccgtcaaggttaaggctggccatatcagcgactgaaaagcggccagcctcggccttgtttgacgtataaccaaagccaccgggcaaccaatagcccttgtcacttttgatcaggtagaccgaccctgaagcgcttttttcgtattccataaaacccccttctgtgcgtgagtactcatagtataacaggcgtgagtaccaacgcaagcactacatgctgaaatctggcccgcccctgtccatgcctcgctggcggggtgccggtgcccgtgccagctcggcccgcgcaagctggacgctgggcagacccatgaccttgctgacggtgcgctcgatgtaatccgcttcgtggccgggcttgcgctctgccagcgctgggctggcctcggccatggccttgccgatttcctcggcactgcggccccggctggccagcttctgcgcggcgataaagtcgcacttgctgaggtcatcaccgaagcgcttgaccagcccggccatctcgctgcggtactcgtccagcgccgtgcgccggtggcggctaagctgccgctcggacagttcgaggctggccagcctgcgggccttctcctgctgccgctgggcctgctcgatctgctggccagcctgctgcaccagcgccgggccagcggtggcggtcttgcccttggattcacgcagcagcacccacggctgataaccggcgcgggtggtgtgcttgtccttgcggttggtgaagcccgccaagcggccatagtggcggctgtcggcgctggccgggtcggcgtcgtactcgctggccagcgtccgggcaatctgcccccgaagttcaccgcctgcggcgtcggccaccttgacccatgcctgatagttcttcgggctggtttccactaccagggcaggctcccggccctcggctttcatgtcatccaggtcaaactcgctgaggtcgtccaccagcaccagaccatgccgctcctgctcggcgggcctgatatacacgtcattgccctgggcattcatccgcttgagccatggcgtgttctggagcacttcggcggctgaccattcccggttcatcatctggccggtggtggcgtccctgacgccgatatcgaagcgctcacagcccatggccttgagctgtcggcctatggcctgcaaagtcctgtcgttcttcatcgggccaccaagcgcagccagatcgagccgtcctcggttgtcagtggcgtcaggtcgagcaagagcaacgatgcgatcagcagcaccaccgtaggcatcatggaagccagcatcacggttagccatagcttccagtgccacccccgcgacgcgctccgggcgctctgcgcggcgctgctcacctcggcggctacctcccgcaactctttggccagctccacccatgccgcccctgtctggcgctgggctttcagccactccgccgcctgcgcctcgctggcctgctgggtctggctcatgacctgccgggcttcgtcggccagtgtcgccatgctctgggccagcggttcgatctgctccgctaactcgttgatgcctctggatttcttcactctgtcgattgcgttcatggtctattgcctcccggtattcctgtaagtcgatgatctgggcgttggcggtgtcgatgttcagggccacgtctgcccggtcggtgcggatgccccggccttccatctccaccacgttcggccccaggtgaacaccgggcaggcgctcgatgccctgcgcctcaagtgttctgtggtcaatgcgggcgtcgtggcctgcccgctctaatgcccggttggcatggtcggcccatgcctcgcgggtctgctcaagccatgccttgggcttgagcgcttcggtcttctgtgccccgcccttctccggggtcttgccgttgtaccgcttgaaccactgagcggcgggccgctcgatgccgtcattgatccgctcggagatcatcaggtggcagtgcgggttctcgccgccaccggcatggatggccagcgtatacggcaggcgctcggcaccggtcaggtgctgggcgaactcggacgccagcgccttctgctggtcgagggtcagctcgaccggcagggcaaattcgacctccttgaacagccgcccattggcgcgttcatacaggtcggcagcatcccagtagtcggcgggccgctcgacgaactccggcatgtgcccggattcggcgtgcaagacttcatccatgtcgcgggcatacttgccttcgcgctggatgaagtcggccttggccctggccgattggccgcccgacctgctgccggttttcgccgtaaggtgataaatcgccatgctgcctcgctgttgcttttgcttttcggctccatgcaatggccctcggagagcgcaccgcccgaagggtggccgttaggccagtttctcgaagagaaaccggtaagtgcgccctcccctacaaagtagggtcgggattgccgccgctgtgcctccatgatagcctacgagacagcacattaacaatggggtgtcaagatggttaaggggagcaacaaggcggcggatcggctggccaagctcgaagaacaacgagcgcgaatcaatgccgaaattcagcgggtgcgggcaagggaacagcagcaagagcgcaagaacgaaacaaggcgcaaggtgctggtgggggccatgattttggccaaggtgaacagcagcgagtggccggaggatcggctcatggcggcaatggatgcgtaccttgaacgcgaccacgaccgcgccttgttcggtctgccgccacgccagaaggatgagccgggctgaatgatcgaccgagacaggccctgcggggctgcacacgcgcccccacccttcgggtagggggaaaggccgctaaagcggctaaaagcgctccagcgtatttctgcggggtttggtgtggggtttagcgggctttgcccgcctttccccctgccgcgcagcggtggggcggtgtgtagcctagcgcagcgaatagaccagctatccggcctctggccgggcatattgggcaagggcagcagcgccccacaagggcgctgataaccgcgcctagtggattattcttagataatcatggatggatttttccaacaccccgccagcccccgcccctgctgggtttgcaggtttgggggcgtgacagttattgcaggggttcgtgacagttattgcaggggggcgtgacagttattgcaggggttcgtgacagttagtacgggagtgacgggcactggctggcaatgtctagcaacggcaggcatttcggctgagggtaaaagaactttccgctaagcgatagactgtatgtaaacacagtattgcaaggacgcggaacatgcctcatgtggcggccctcgcgagaattaattcagataaaaaaaatccttagctttcgctaaggatgatttctagcgatgaccctgctgattggttcgctgaccgtagactggttggcttggtttcatcagccatccgcttgccctcatctgttacgccggcggtagccggccagcctcgcagagcaggattcccgttgagcaccgccaggtgcgaataagggacagtgaagaaggaacacccgctcgcgggtgggcctacttcacctatcctgcccggctgacgccgttggatacaccaaggaaagtctacacgaaccctttggcaaaatcctgtatatcgtgcgacatcgcgcgcgcgcgcgcggatgctagtacgttgtgtctcaaaatctctgatgttacattgcacaagataaaaatatatcatcatgaacaataaaactgtctgcttacataaacagtaatacaaggggtgttatgagccatattcaacgggaaacgtcttgctcgaggccgcgattaaattccaacatggatgctgatttatatgggtataaatgggctcgcgataatgtcgggcaatcaggtgcgacaatctatcgattgtatgggaagcccgatgcgccagagttgtttctgaaacatggcaaaggtagcgttgccaatgatgttacagatgagatggtcagactaaactggctgacggaatttatgcctcttccgaccatcaagcattttatccgtactcctgatgatgcatggttactcaccactgcgatccccgggaaaacagcattccaggtattagaagaatatcctgattcaggtgaaaatattgttgatgcgctggcagtgttcctgcgccggttgcattcgattcctgtttgtaattgtccttttaacagcgatcgcgtatttcgtctcgctcaggcgcaatcacgaatgaataacggtttggttgatgcgagtgattttgatgacgagcgtaatggctggcctgttgaacaagtctggaaagaaatgcataagcttttgccattctcaccggattcagtcgtcactcatggtgatttctcacttgataaccttatttttgacgaggggaaattaataggttgtattgatgttggacgagtcggaatcgcagaccgataccaggatcttgccatcctatggaactgcctcggtgagttttctccttcattacagaaacggctttttcaaaaatatggtattgataatcctgatatgaataaattgcagtttcatttgatgctcgatgagtttttctaatcagaattggttaattggttgtaacactggcagagcattacgctgacttgacgggacggcggctttgttgaataaatcgaacttttgctgagttgaaggatcagatcacgcatcttcccgacaacgcagaccgttccgtggcaaagcaaaagttcaaaatcaccaactggtccacctacaacaaagctctcatcaaccgtggctccctcactttctggctggatgatggggcgattcaggcctggtatgagtcagcaacaccttcttcacgaggcagacctcagcgctattctgaccttgccatcacgactgtgctggtcattaaacgcgtattcaggctgaccctgcgcgctgcgcagggctttattgattccatttttacactgatgaatgttccgttgcgctgcccggattacagatcctctagataatgaattctataggtaccttgacagctagctcagtcctaggtataatgctagcactagagaaagaggagaaatactagtatgtggagccacccgcagttcgaaaaaggatcaagcaaaggagaagaacttttcactggagttgtcccaattcttgttgaattagatggtgatgttaatgggcacaaattttctgtccgtggagagggtgaaggtgatgctacaaacggaaaacttacccttaaatttatttgcactactggaaaactacctgttccatggccaacacttgtcactactctcacttatggtgttcaatgcttttcccgttatccggatcatatgaaacggcatgactttttcaagagtgccatgcccgaaggttatgtacaggaacgcactatatctttcaaagatgacgggacttacaagacgcgtgctgaagtcaagtttgaaggtgatacccttgttaatcgtatcgagttaaaaggtattgattttaaagaagatggaaacattctcggacacaaacttgagtacaactttaactcacacaatgtatacatcacggcagacaaacaaaagaatggaatcaaagctaacttcaaaattcgccacaacgttgaagatggttccgttcaactagcagaccattatcaacaaaatactccaattggcgatggccctgtccttttaccagacaaccattacctgtctacacaatctgtcctttcgaaagatcccaacgaaaagcgtgaccacatggtccttcttgagtttgtaactgctgctgggattacacatggcatggatgagctctacaaataaggatcctgaagatccaacgctcggttgccgccgggcgttttttattctgcaggagcagaagagcatacatctggaagctttctagaatcgggggcccccggggggattctagaacaatgga

SEQ ID NO: 3 - DNA, 8410 bp, synthetic construct
  source 1..8410: mol_type = other DNA
agtcctcgtctcgccctcgaattagcccgcttaatgagcgggctttttttgaattaattctcgcgagctggcacgacaggtttcccgactggaaagcgggcagtgagcgcaacgcaattaatgtaagttagcgcgaattgcaagctggccgacgcgctgggctacgtcttgctggcgttcgggagcagaagagcatacatctggaagcaaagccaggaaagcggcctatggagctgtgcggcagcgctcagtaggcaatttttcaaaatattgttaagccttttctgagcatggtatttttcatggtattaccaattagcaggaaaataagccattgaatataaaagataaaaatgtcttgtttacaatagagtggggggggtcagcctgccgccttgggccgggtgatgtcgtacttgcccgccgcgaactcggttaccgtccagcccagcgcgaccagctccggcaacgcctcgcgcacccgctggcggcgcttgcgcatggtcgaaccactggcctctgacggccagacatagccgcacaaggtatctatggaagccttgccggttttgccggggtcgatccagccacacagccgctggtgcagcaggcgggcggtttcgctgtccagcgcccgcacctcgtccatgctgatgcgcacatgctggccgccacccatgacggcctgcgcgatcaaggggttcagggccacgtacaggcgcccgtccgcctcgtcgctggcgtactccgacagcagccgaaacccctgccgcttgcggccattctgggcgatgatggataccttccaaaggcgctcgatgcagtcctgtatgtgcttgagcgccccaccactatcgacctctgccccgatttcctttgccagcgcccgatagctacctttgaccaccatggcatcagcggtgacggcctcccacttgggttccaggaacagccggagctgccgtccgccttcggtcttgggttccgggccaagcactaggccattaggcccagccatggccaccagcccttgcaggatgcgcagatcatcagcgcccagcggctccgggccgctgaactcgatccgcttgccgtcgccgtagtcatacgtcacgtccagcttgctgcgcttgcgctcgccccgcttgagggcacggaacaggccgggggccagacagtgcgccgggtcgtgtcggacgtggctgaggctgtgcttgttcttaggcttcaccacggggcacccccttgctcttgcgctgcctctccagcacggcgggcttgagcaccccgccgtcatgccgcctgaaccaccgatcagcgaacggtgcgccatagttggccttgctcacaccgaagcggacgaagaaccggcgctggtcgtcgtccacaccccattcctcggcctcggcgctggtcatgctcgacaggtaggactgccagcggatgttatcgaccagtaccgagctgccccggctggcctgctgctggtcgcctgcgcccatcatggccgcgcccttgctggcatggtgcaggaacacgatagagcacccggtatcggcggcgatggcctccatgcgaccgatgacctgggccatggggccgctggcgttttcttcctcgatgtggaaccggcgcagcgtgtccagcaccatcaggcggcggccctcggcggcgcgcttgaggccgtcgaaccactccggggccatgatgttgggcaggctgccgatcagcggctggatcagcaggccgtcagccacggcttgccgttcctcggcgctgaggtgcgccccaagggcgtgcaggcggtgatgaatggcggtgggcgggtcttcggcgggcaggtagatcaccgggccggtgggcagttcgcccacctccagcagatccggcccgcctgcaatctgtgcggccagttgcagggccagcatggatttaccggcaccaccgggcgacaccagcgccccgaccgtaccggccaccatgttgggcaaaacgtagtccagcggtggcggcgctgctgcgaacgcctccagaatattgataggcttatgggtagccattgattgcctcctttgcaggcagttggtggttaggcgctggcggggtcactacccccgccctgcgccgctctgagttcttccaggcactcgcgcagcgcctcgtattcgtcgtcggtcagccagaacttgcgctgacgcatccctttggccttcatgcgctcggcatatcgcgcttggcgtacagcgtcagggctggccagcaggtcgccggtctgcttgtccttttggtctttcatatcagtcaccgagaaacttgccggggccgaaaggcttgtcttcgcggaacaaggacaaggtgcagccgtcaaggttaaggctggccatatcagcgactgaaaagcggccagcctcggccttgtttgacgtataaccaaagccaccgggcaaccaatagcccttgtcacttttgatcaggtagaccgaccctgaagcgcttttttcgtattccataaaacccccttctgtgcgtgagtactcatagtataacaggcgtgagtaccaacgcaagcactacatgctgaaatctggcccgcccctgtccatgcctcgctggcggggtgccggtgcccgtgccagctcggcccgcgcaagctggacgctgggcagacccatgaccttgctgacggtgcgctcgatgtaatccgcttcgtggccgggcttgcgctctgccagcgctgggctggcctcggccatggccttgccgatttcctcggcactgcggccccggctggccagcttctgcgcggcgataaagtcgcacttgctgaggtcatcaccgaagcgcttgaccagcccggccatctcgctgcggtactcgtccagcgccgtgcgccggtggcggctaagctgccgctcggacagttcgaggctggccagcctgcgggccttctcctgctgccgctgggcctgctcgatctgctggccagcctgctgcaccagcgccgggccagcggtggcggtcttgcccttggattcacgcagcagcacccacggctgataaccggcgcgggtggtgtgcttgtccttgcggttggtgaagcccgccaagcggccatagtggcggctgtcggcgctggccgggtcggcgtcgtactcgctggccagcgtccgggcaatctgcccccgaagttcaccgcctgcggcgtcggccaccttgacccatgcctgatagttcttcgggctggtttccactaccagggcaggctcccggccctcggctttcatgtcatccaggtcaaactcgctgaggtcgtccaccagcaccagaccatgccgctcctgctcggcgggcctgatatacacgtcattgccctgggcattcatccgcttgagccatggcgtgttctggagcacttcggcggctgaccattcccggttcatcatctggccggtggtggcgtccctgacgccgatatcgaagcgctcacagcccatggccttgagctgtcggcctatggcctgcaaagtcctgtcgttcttcatcgggccaccaagcgcagccagatcgagccgtcctcggttgtcagtggcgtcaggtcgagcaagagcaacgatgcgatcagcagcaccaccgtaggcatcatggaagccagcatcacggttagccatagcttccagtgccacccccgcgacgcgctccgggcgctctgcgcggcgctgctcacctcggcggctacctcccgcaactctttggccagctccacccatgccgcccctgtctggcgctgggctttcagccactccgccgcctgcgcctcgctggcctgctgggtctggctcatgacctgccgggcttcgtcggccagtgtcgccatgctctgggccagcggttcgatctgctccgctaactcgttgatgcctctggatttcttcactctgtcgattgcgttcatggtctattgcctcccggtattcctgtaagtcgatgatctgggcgttggcggtgtcgatgttcagggccacgtctgcccggtcggtgcggatgccccggccttccatctccaccacgttcggccccaggtgaacaccgggcaggcgctcgatgccctgcgcctcaagtgttctgtggtcaatgcgggcgtcgtggcctgcccgctctaatgcccggttggcatggtcggcccatgcctcgcgggtctgctcaagccatgccttgggcttgagcgcttcggtcttctgtgccccgcccttctccggggtcttgccgttgtaccgcttgaaccactgagcggcgggccgctcgatgccgtcattgatccgctcggagatcatcaggtggcagtgcgggttctcgccgccaccggcatggatggccagcgtatacggcaggcgctcggcaccggtcaggtgctgggcgaactcggacgccagcgccttctgctggtcgagggtcagctcgaccggcagggcaaattcgacctccttgaacagccgcccattggcgcgttcatacaggtcggcagcatcccagtagtcggcgggccgctcgacgaactccggcatgtgcccggattcggcgtgcaagacttcatccatgtcgcgggcatacttgccttcgcgctggatgaagtcggccttggccctggccgattggccgcccgacctgctgccggttttcgccgtaaggtgataaatcgccatgctgcctcgctgttgcttttgcttttcggctccatgcaatggccctcggagagcgcaccgcccgaagggtggccgttaggccagtttctcgaagagaaaccggtaagtgcgccctcccctacaaagtagggtcgggattgccgccgctgtgcctccatgatagcctacgagacagcacattaacaatggggtgtcaagatggttaaggggagcaacaaggcggcggatcggctggccaagctcgaagaacaacgagcgcgaatcaatgccgaaattcagcgggtgcgggcaagggaacagcagcaagagcgcaagaacgaaacaaggcgcaaggtgctggtgggggccatgattttggccaaggtgaacagcagcgagtggccggaggatcggctcatggcggcaatggatgcgtaccttgaacgcgaccacgaccgcgccttgttcggtctgccgccacgccagaaggatgagccgggctgaatgatcgaccgagacaggccctgcggggctgcacacgcgcccccacccttcgggtagggggaaaggccgctaaagcggctaaaagcgctccagcgtatttctgcggggtttggtgtggggtttagcgggctttgcccgcctttccccctgccgcgcagcggtggggcggtgtgtagcctagcgcagcgaatagaccagctatccggcctctggccgggcatattgggcaagggcagcagcgccccacaagggcgctgataaccgcgcctagtggattattcttagataatcatggatggatttttccaacaccccgccagcccccgcccctgctgggtttgcaggtttgggggcgtgacagttattgcaggggttcgtgacagttattgcaggggggcgtgacagttattgcaggggttcgtgacagttagtacgggagtgacgggcactggctggcaatgtctagcaacggcaggcatttcggctgagggtaaaagaactttccgctaagcgatagactgtatgtaaacacagtattgcaaggacgcggaacatgcctcatgtggcggccctcgcgagaattaattcagataaaaaaaatccttagctttcgctaaggatgatttctagcgatgaccctgctgattggttcgctgaccgtagactggttggcttggtttcatcagccatccgcttgccctcatctgttacgccggcggtagccggccagcctcgcagagcaggattcccgttgagcaccgccaggtgcgaataagggacagtgaagaaggaacacccgctcgcgggtgggcctacttcacctatcctgcccggctgacgccgttggatacaccaaggaaagtctacacgaaccctttggcaaaatcctgtatatcgtgcgacatcgcgcgcgcgcgcgcggatgctagtacgttgtgtctcaaaatctctgatgttacattgcacaagataaaaatatatcatcatgaacaataaaactgtctgcttacataaacagtaatacaaggggtgttatgagccatattcaacgggaaacgtcttgctcgaggccgcgattaaattccaacatggatgctgatttatatgggtataaatgggctcgcgataatgtcgggcaatcaggtgcgacaatctatcgattgtatgggaagcccgatgcgccagagttgtttctgaaacatggcaaaggtagcgttgccaatgatgttacagatgagatggtcagactaaactggctgacggaatttatgcctcttccgaccatcaagcattttatccgtactcctgatgatgcatggttactcaccactgcgatccccgggaaaacagcattccaggtattagaagaatatcctgattcaggtgaaaatattgttgatgcgctggcagtgttcctgcgccggttgcattcgattcctgtttgtaattgtccttttaacagcgatcgcgtatttcgtctcgctcaggcgcaatcacgaatgaataacggtttggttgatgcgagtgattttgatgacgagcgtaatggctggcctgttgaacaagtctggaaagaaatgcataagcttttgccattctcaccggattcagtcgtcactcatggtgatttctcacttgataaccttatttttgacgaggggaaattaataggttgtattgatgttggacgagtcggaatcgcagaccgataccaggatcttgccatcctatggaactgcctcggtgagttttctccttcattacagaaacggctttttcaaaaatatggtattgataatcctgatatgaataaattgcagtttcatttgatgctcgatgagtttttctaatcagaattggttaattggttgtaacactggcagagcattacgctgacttgacgggacggcggctttgttgaataaatcgaacttttgctgagttgaaggatcagatcacgcatcttcccgacaacgcagaccgttccgtggcaaagcaaaagttcaaaatcaccaactggtccacctacaacaaagctctcatcaaccgtggctccctcactttctggctggatgatggggcgattcaggcctggtatgagtcagcaacaccttcttcacgaggcagacctcagcgctattctgaccttgccatcacgactgtgctggtcattaaacgcgtattcaggctgaccctgcgcgctgcgcagggctttattgattccatttttacactgatgaatgttccgttgcgctgcccggattacagatcctctagataatgaattctataggtaccttgacggctagctcagtcctaggtatagtgctagcactagagaaagaggggaaatactagtatgtggagccacccgcagttcgaaaaaggatcaagcaaaggagaagaacttttcactggagttgtcccaattcttgttgaattagatggtgatgttaatgggcacaaattttctgtccgtggagagggtgaaggtgatgctacaaacggaaaacttacccttaaatttatttgcactactggaaaactacctgttccatggccaacacttgtcactactctcacttatggtgttcaatgcttttcccgttatccggatcatatgaaacggcatgactttttcaagagtgccatgcccgaaggttatgtacaggaacgcactatatctttcaaagatgacgggacttacaagacgcgtgctgaagtcaagtttgaaggtgatacccttgttaatcgtatcgagttaaaaggtattgattttaaagaagatggaaacattctcggacacaaacttgagtacaactttaactcacacaatgtatacatcacggcagacaaacaaaagaatggaatcaaagctaacttcaaaattcgccacaacgttgaagatggttccgttcaactagcagaccattatcaacaaaatactccaattggcgatggccctgtccttttaccagacaaccattacctgtctacacaatctgtcctttcgaaagatcccaacgaaaagcgtgaccacatggtccttcttgagtttgtaactgctgctgggattacacatggcatggatgagctctacaaataaggatcctgaagatccaacgctcggttgccgccgggcgttttttattctgcaggagcagaagagcatacatctggaagctttctagaatcgggggcccccggggggattctagaacaatgga

SEQ ID NO: 4 - DNA, 8411 bp, synthetic construct
  source 1..8411: mol_type = other DNA
agtcctcgtctcgccctcgaattagcccgcttaatgagcgggctttttttgaattaattctcgcgagctggcacgacaggtttcccgactggaaagcgggcagtgagcgcaacgcaattaatgtaagttagcgcgaattgcaagctggccgacgcgctgggctacgtcttgctggcgttcgggagcagaagagcatacatctggaagcaaagccaggaaagcggcctatggagctgtgcggcagcgctcagtaggcaatttttcaaaatattgttaagccttttctgagcatggtatttttcatggtattaccaattagcaggaaaataagccattgaatataaaagataaaaatgtcttgtttacaatagagtggggggggtcagcctgccgccttgggccgggtgatgtcgtacttgcccgccgcgaactcggttaccgtccagcccagcgcgaccagctccggcaacgcctcgcgcacccgctggcggcgcttgcgcatggtcgaaccactggcctctgacggccagacatagccgcacaaggtatctatggaagccttgccggttttgccggggtcgatccagccacacagccgctggtgcagcaggcgggcggtttcgctgtccagcgcccgcacctcgtccatgctgatgcgcacatgctggccgccacccatgacggcctgcgcgatcaaggggttcagggccacgtacaggcgcccgtccgcctcgtcgctggcgtactccgacagcagccgaaacccctgccgcttgcggccattctgggcgatgatggataccttccaaaggcgctcgatgcagtcctgtatgtgcttgagcgccccaccactatcgacctctgccccgatttcctttgccagcgcccgatagctacctttgaccaccatggcatcagcggtgacggcctcccacttgggttccaggaacagccggagctgccgtccgccttcggtcttgggttccgggccaagcactaggccattaggcccagccatggccaccagcccttgcaggatgcgcagatcatcagcgcccagcggctccgggccgctgaactcgatccgcttgccgtcgccgtagtcatacgtcacgtccagcttgctgcgcttgcgctcgccccgcttgagggcacggaacaggccgggggccagacagtgcgccgggtcgtgtcggacgtggctgaggctgtgcttgttcttaggcttcaccacggggcacccccttgctcttgcgctgcctctccagcacggcgggcttgagcaccccgccgtcatgccgcctgaaccaccgatcagcgaacggtgcgccatagttggccttgctcacaccgaagcggacgaagaaccggcgctggtcgtcgtccacaccccattcctcggcctcggcgctggtcatgctcgacaggtaggactgccagcggatgttatcgaccagtaccgagctgccccggctggcctgctgctggtcgcctgcgcccatcatggccgcgcccttgctggcatggtgcaggaacacgatagagcacccggtatcggcggcgatggcctccatgcgaccgatgacctgggccatggggccgctggcgttttcttcctcgatgtggaaccggcgcagcgtgtccagcaccatcaggcggcggccctcggcggcgcgcttgaggccgtcgaaccactccggggccatgatgttgggcaggctgccgatcagcggctggatcagcaggccgtcagccacggcttgccgttcctcggcgctgaggtgcgccccaagggcgtgcaggcggtgatgaatggcggtgggcgggtcttcggcgggcaggtagatcaccgggccggtgggcagttcgcccacctccagcagatccggcccgcctgcaatctgtgcggccagttgcagggccagcatggatttaccggcaccaccgggcgacaccagcgccccgaccgtaccggccaccatgttgggcaaaacgtagtccagcggtggcggcgctgctgcgaacgcctccagaatattgataggcttatgggtagccattgattgcctcctttgcaggcagttggtggttaggcgctggcggggtcactacccccgccctgcgccgctctgagttcttccaggcactcgcgcagcgcctcgtattcgtcgtcggtcagccagaacttgcgctgacgcatccctttggccttcatgcgctcggcatatcgcgcttggcgtacagcgtcagggctggccagcaggtcgccggtctgcttgtccttttggtctttcatatcagtcaccgagaaacttgccggggccgaaaggcttgtcttcgcggaacaaggacaaggtgcagccgtcaaggttaaggctggccatatcagcgactgaaaagcggccagcctcggccttgtttgacgtataaccaaagccaccgggcaaccaatagcccttgtcacttttgatcaggtagaccgaccctgaagcgcttttttcgtattccataaaacccccttctgtgcgtgagtactcatagtataacaggcgtgagtaccaacgcaagcactacatgctgaaatctggcccgcccctgtccatgcctcgctggcggggtgccggtgcccgtgccagctcggcccgcgcaagctggacgctgggcagacccatgaccttgctgacggtgcgctcgatgtaatccgcttcgtggccgggcttgcgctctgccagcgctgggctggcctcggccatggccttgccgatttcctcggcactgcggccccggctggccagcttctgcgcggcgataaagtcgcacttgctgaggtcatcaccgaagcgcttgaccagcccggccatctcgctgcggtactcgtccagcgccgtgcgccggtggcggctaagctgccgctcggacagttcgaggctggccagcctgcgggccttctcctgctgccgctgggcctgctcgatctgctggccagcctgctgcaccagcgccgggccagcggtggcggtcttgcccttggattcacgcagcagcacccacggctgataaccggcgcgggtggtgtgcttgtccttgcggttggtgaagcccgccaagcggccatagtggcggctgtcggcgctggccgggtcggcgtcgtactcgctggccagcgtccgggcaatctgcccccgaagttcaccgcctgcggcgtcggccaccttgacccatgcctgatagttcttcgggctggtttccactaccagggcaggctcccggccctcggctttcatgtcatccaggtcaaactcgctgaggtcgtccaccagcaccagaccatgccgctcctgctcggcgggcctgatatacacgtcattgccctgggcattcatccgcttgagccatggcgtgttctggagcacttcggcggctgaccattcccggttcatcatctggccggtggtggcgtccctgacgccgatatcgaagcgctcacagcccatggccttgagctgtcggcctatggcctgcaaagtcctgtcgttcttcatcgggccaccaagcgcagccagatcgagccgtcctcggttgtcagtggcgtcaggtcgagcaagagcaacgatgcgatcagcagcaccaccgtaggcatcatggaagccagcatcacggttagccatagcttccagtgccacccccgcgacgcgctccgggcgctctgcgcggcgctgctcacctcggcggctacctcccgcaactctttggccagctccacccatgccgcccctgtctggcgctgggctttcagccactccgccgcctgcgcctcgctggcctgctgggtctggctcatgacctgccgggcttcgtcggccagtgtcgccatgctctgggccagcggttcgatctgctccgctaactcgttgatgcctctggatttcttcactctgtcgattgcgttcatggtctattgcctcccggtattcctgtaagtcgatgatctgggcgttggcggtgtcgatgttcagggccacgtctgcccggtcggtgcggatgccccggccttccatctccaccacgttcggccccaggtgaacaccgggcaggcgctcgatgccctgcgcctcaagtgttctgtggtcaatgcgggcgtcgtggcctgcccgctctaatgcccggttggcatggtcggcccatgcctcgcgggtctgctcaagccatgccttgggcttgagcgcttcggtcttctgtgccccgcccttctccggggtcttgccgttgtaccgcttgaaccactgagcggcgggccgctcgatgccgtcattgatccgctcggagatcatcaggtggcagtgcgggttctcgccgccaccggcatggatggccagcgtatacggcaggcgctcggcaccggtcaggtgctgggcgaactcggacgccagcgccttctgctggtcgagggtcagctcgaccggcagggcaaattcgacctccttgaacagccgcccattggcgcgttcatacaggtcggcagcatcccagtagtcggcgggccgctcgacgaactccggcatgtgcccggattcggcgtgcaagacttcatccatgtcgcgggcatacttgccttcgcgctggatgaagtcggccttggccctggccgattggccgcccgacctgctgccggttttcgccgtaaggtgataaatcgccatgctgcctcgctgttgcttttgcttttcggctccatgcaatggccctcggagagcgcaccgcccgaagggtggccgttaggccagtttctcgaagagaaaccggtaagtgcgccctcccctacaaagtagggtcgggattgccgccgctgtgcctccatgatagcctacgagacagcacattaacaatggggtgtcaagatggttaaggggagcaacaaggcggcggatcggctggccaagctcgaagaacaacgagcgcgaatcaatgccgaaattcagcgggtgcgggcaagggaacagcagcaagagcgcaagaacgaaacaaggcgcaaggtgctggtgggggccatgattttggccaaggtgaacagcagcgagtggccggaggatcggctcatggcggcaatggatgcgtaccttgaacgcgaccacgaccgcgccttgttcggtctgccgccacgccagaaggatgagccgggctgaatgatcgaccgagacaggccctgcggggctgcacacgcgcccccacccttcgggtagggggaaaggccgctaaagcggctaaaagcgctccagcgtatttctgcggggtttggtgtggggtttagcgggctttgcccgcctttccccctgccgcgcagcggtggggcggtgtgtagcctagcgcagcgaatagaccagctatccggcctctggccgggcatattgggcaagggcagcagcgccccacaagggcgctgataaccgcgcctagtggattattcttagataatcatggatggatttttccaacaccccgccagcccccgcccctgctgggtttgcaggtttgggggcgtgacagttattgcaggggttcgtgacagttattgcaggggggcgtgacagttattgcaggggttcgtgacagttagtacgggagtgacgggcactggctggcaatgtctagcaacggcaggcatttcggctgagggtaaaagaactttccgctaagcgatagactgtatgtaaacacagtattgcaaggacgcggaacatgcctcatgtggcggccctcgcgagaattaattcagataaaaaaaatccttagctttcgctaaggatgatttctagcgatgaccctgctgattggttcgctgaccgtagactggttggcttggtttcatcagccatccgcttgccctcatctgttacgccggcggtagccggccagcctcgcagagcaggattcccgttgagcaccgccaggtgcgaataagggacagtgaagaaggaacacccgctcgcgggtgggcctacttcacctatcctgcccggctgacgccgttggatacaccaaggaaagtctacacgaaccctttggcaaaatcctgtatatcgtgcgacatcgcgcgcgcgcgcgcggatgctagtacgttgtgtctcaaaatctctgatgttacattgcacaagataaaaatatatcatcatgaacaataaaactgtctgcttacataaacagtaatacaaggggtgttatgagccatattcaacgggaaacgtcttgctcgaggccgcgattaaattccaacatggatgctgatttatatgggtataaatgggctcgcgataatgtcgggcaatcaggtgcgacaatctatcgattgtatgggaagcccgatgcgccagagttgtttctgaaacatggcaaaggtagcgttgccaatgatgttacagatgagatggtcagactaaactggctgacggaatttatgcctcttccgaccatcaagcattttatccgtactcctgatgatgcatggttactcaccactgcgatccccgggaaaacagcattccaggtattagaagaatatcctgattcaggtgaaaatattgttgatgcgctggcagtgttcctgcgccggttgcattcgattcctgtttgtaattgtccttttaacagcgatcgcgtatttcgtctcgctcaggcgcaatcacgaatgaataacggtttggttgatgcgagtgattttgatgacgagcgtaatggctggcctgttgaacaagtctggaaagaaatgcataagcttttgccattctcaccggattcagtcgtcactcatggtgatttctcacttgataaccttatttttgacgaggggaaattaataggttgtattgatgttggacgagtcggaatcgcagaccgataccaggatcttgccatcctatggaactgcctcggtgagttttctccttcattacagaaacggctttttcaaaaatatggtattgataatcctgatatgaataaattgcagtttcatttgatgctcgatgagtttttctaatcagaattggttaattggttgtaacactggcagagcattacgctgacttgacgggacggcggctttgttgaataaatcgaacttttgctgagttgaaggatcagatcacgcatcttcccgacaacgcagaccgttccgtggcaaagcaaaagttcaaaatcaccaactggtccacctacaacaaagctctcatcaaccgtggctccctcactttctggctggatgatggggcgattcaggcctggtatgagtcagcaacaccttcttcacgaggcagacctcagcgctattctgaccttgccatcacgactgtgctggtcattaaacgcgtattcaggctgaccctgcgcgctgcgcagggctttattgattccatttttacactgatgaatgttccgttgcgctgcccggattacagatcctctagataatgaattctataggtacctttatggctagctcagtcctaggtacaatgctagcactagagtcacacaggaaaccactagtatgtggagccacccgcagttcgaaaaaggatcaagcaaaggagaagaacttttcactggagttgtcccaattcttgttgaattagatggtgatgttaatgggcacaaattttctgtccgtggagagggtgaaggtgatgctacaaacggaaaacttacccttaaatttatttgcactactggaaaactacctgttccatggccaacacttgtcactactctcacttatggtgttcaatgcttttcccgttatccggatcatatgaaacggcatgactttttcaagagtgccatgcccgaaggttatgtacaggaacgcactatatctttcaaagatgacgggacttacaagacgcgtgctgaagtcaagtttgaaggtgatacccttgttaatcgtatcgagttaaaaggtattgattttaaagaagatggaaacattctcggacacaaacttgagtacaactttaactcacacaatgtatacatcacggcagacaaacaaaagaatggaatcaaagctaacttcaaaattcgccacaacgttgaagatggttccgttcaactagcagaccattatcaacaaaatactccaattggcgatggccctgtccttttaccagacaaccattacctgtctacacaatctgtcctttcgaaagatcccaacgaaaagcgtgaccacatggtccttcttgagtttgtaactgctgctgggattacacatggcatggatgagctctacaaataaggatcctgaagatccaacgctcggttgccgccgggcgttttttattctgcaggagcagaagagcatacatctggaagctttctagaatcgggggcccccggggggattctagaacaatgga

SEQ ID NO: 5 - DNA, 7632 bp, synthetic construct
  source 1..7632: mol_type = other DNA
agtcctcgtctcgccctcgaattagcccgcttaatgagcgggctttttttgaattaattctcgcgagctggcacgacaggtttcccgactggaaagcgggcagtgagcgcaacgcaattaatgtaagttagcgcgaattgcaagctggccgacgcgctgggctacgtcttgctggcgttcgggagcagaagagcatacatctggaagcaaagccaggaaagcggcctatggagctgtgcggcagcgctcagtaggcaatttttcaaaatattgttaagccttttctgagcatggtatttttcatggtattaccaattagcaggaaaataagccattgaatataaaagataaaaatgtcttgtttacaatagagtggggggggtcagcctgccgccttgggccgggtgatgtcgtacttgcccgccgcgaactcggttaccgtccagcccagcgcgaccagctccggcaacgcctcgcgcacccgctggcggcgcttgcgcatggtcgaaccactggcctctgacggccagacatagccgcacaaggtatctatggaagccttgccggttttgccggggtcgatccagccacacagccgctggtgcagcaggcgggcggtttcgctgtccagcgcccgcacctcgtccatgctgatgcgcacatgctggccgccacccatgacggcctgcgcgatcaaggggttcagggccacgtacaggcgcccgtccgcctcgtcgctggcgtactccgacagcagccgaaacccctgccgcttgcggccattctgggcgatgatggataccttccaaaggcgctcgatgcagtcctgtatgtgcttgagcgccccaccactatcgacctctgccccgatttcctttgccagcgcccgatagctacctttgaccaccatggcatcagcggtgacggcctcccacttgggttccaggaacagccggagctgccgtccgccttcggtcttgggttccgggccaagcactaggccattaggcccagccatggccaccagcccttgcaggatgcgcagatcatcagcgcccagcggctccgggccgctgaactcgatccgcttgccgtcgccgtagtcatacgtcacgtccagcttgctgcgcttgcgctcgccccgcttgagggcacggaacaggccgggggccagacagtgcgccgggtcgtgtcggacgtggctgaggctgtgcttgttcttaggcttcaccacggggcacccccttgctcttgcgctgcctctccagcacggcgggcttgagcaccccgccgtcatgccgcctgaaccaccgatcagcgaacggtgcgccatagttggccttgctcacaccgaagcggacgaagaaccggcgctggtcgtcgtccacaccccattcctcggcctcggcgctggtcatgctcgacaggtaggactgccagcggatgttatcgaccagtaccgagctgccccggctggcctgctgctggtcgcctgcgcccatcatggccgcgcccttgctggcatggtgcaggaacacgatagagcacccggtatcggcggcgatggcctccatgcgaccgatgacctgggccatggggccgctggcgttttcttcctcgatgtggaaccggcgcagcgtgtccagcaccatcaggcggcggccctcggcggcgcgcttgaggccgtcgaaccactccggggccatgatgttgggcaggctgccgatcagcggctggatcagcaggccgtcagccacggcttgccgttcctcggcgctgaggtgcgccccaagggcgtgcaggcggtgatgaatggcggtgggcgggtcttcggcgggcaggtagatcaccgggccggtgggcagttcgcccacctccagcagatccggcccgcctgcaatctgtgcggccagttgcagggccagcatggatttaccggcaccaccgggcgacaccagcgccccgaccgtaccggccaccatgttgggcaaaacgtagtccagcggtggcggcgctgctgcgaacgcctccagaatattgataggcttatgggtagccattgattgcctcctttgcaggcagttggtggttaggcgctggcggggtcactacccccgccctgcgccgctctgagttcttccaggcactcgcgcagcgcctcgtattcgtcgtcggtcagccagaacttgcgctgacgcatccctttggccttcatgcgctcggcatatcgcgcttggcgtacagcgtcagggctggccagcaggtcgccggtctgcttgtccttttggtctttcatatcagtcaccgagaaacttgccggggccgaaaggcttgtcttcgcggaacaaggacaaggtgcagccgtcaaggttaaggctggccatatcagcgactgaaaagcggccagcctcggccttgtttgacgtataaccaaagccaccgggcaaccaatagcccttgtcacttttgatcaggtagaccgaccctgaagcgcttttttcgtattccataaaacccccttctgtgcgtgagtactcatagtataacaggcgtgagtaccaacgcaagcactacatgctgaaatctggcccgcccctgtccatgcctcgctggcggggtgccggtgcccgtgccagctcggcccgcgcaagctggacgctgggcagacccatgaccttgctgacggtgcgctcgatgtaatccgcttcgtggccgggcttgcgctctgccagcgctgggctggcctcggccatggccttgccgatttcctcggcactgcggccccggctggccagcttctgcgcggcgataaagtcgcacttgctgaggtcatcaccgaagcgcttgaccagcccggccatctcgctgcggtactcgtccagcgccgtgcgccggtggcggctaagctgccgctcggacagttcgaggctggccagcctgcgggccttctcctgctgccgctgggcctgctcgatctgctggccagcctgctgcaccagcgccgggccagcggtggcggtcttgcccttggattcacgcagcagcacccacggctgataaccggcgcgggtggtgtgcttgtccttgcggttggtgaagcccgccaagcggccatagtggcggctgtcggcgctggccgggtcggcgtcgtactcgctggccagcgtccgggcaatctgcccccgaagttcaccgcctgcggcgtcggccaccttgacccatgcctgatagttcttcgggctggtttccactaccagggcaggctcccggccctcggctttcatgtcatccaggtcaaactcgctgaggtcgtccaccagcaccagaccatgccgctcctgctcggcgggcctgatatacacgtcattgccctgggcattcatccgcttgagccatggcgtgttctggagcacttcggcggctgaccattcccggttcatcatctggccggtggtggcgtccctgacgccgatatcgaagcgctcacagcccatggccttgagctgtcggcctatggcctgcaaagtcctgtcgttcttcatcgggccaccaagcgcagccagatcgagccgtcctcggttgtcagtggcgtcaggtcgagcaagagcaacgatgcgatcagcagcaccaccgtaggcatcatggaagccagcatcacggttagccatagcttccagtgccacccccgcgacgcgctccgggcgctctgcgcggcgctgctcacctcggcggctacctcccgcaactctttggccagctccacccatgccgcccctgtctggcgctgggctttcagccactccgccgcctgcgcctcgctggcctgctgggtctggctcatgacctgccgggcttcgtcggccagtgtcgccatgctctgggccagcggttcgatctgctccgctaactcgttgatgcctctggatttcttcactctgtcgattgcgttcatggtctattgcctcccggtattcctgtaagtcgatgatctgggcgttggcggtgtcgatgttcagggccacgtctgcccggtcggtgcggatgccccggccttccatctccaccacgttcggccccaggtgaacaccgggcaggcgctcgatgccctgcgcctcaagtgttctgtggtcaatgcgggcgtcgtggcctgcccgctctaatgcccggttggcatggtcggcccatgcctcgcgggtctgctcaagccatgccttgggcttgagcgcttcggtcttctgtgccccgcccttctccggggtcttgccgttgtaccgcttgaaccactgagcggcgggccgctcgatgccgtcattgatccgctcggagatcatcaggtggcagtgcgggttctcgccgccaccggcatggatggccagcgtatacggcaggcgctcggcaccggtcaggtgctgggcgaactcggacgccagcgccttctgctggtcgagggtcagctcgaccggcagggcaaattcgacctccttgaacagccgcccattggcgcgttcatacaggtcggcagcatcccagtagtcggcgggccgctcgacgaactccggcatgtgcccggattcggcgtgcaagacttcatccatgtcgcgggcatacttgccttcgcgctggatgaagtcggccttggccctggccgattggccgcccgacctgctgccggttttcgccgtaaggtgataaatcgccatgctgcctcgctgttgcttttgcttttcggctccatgcaatggccctcggagagcgcaccgcccgaagggtggccgttaggccagtttctcgaagagaaaccggtaagtgcgccctcccctacaaagtagggtcgggattgccgccgctgtgcctccatgatagcctacgagacagcacattaacaatggggtgtcaagatggttaaggggagcaacaaggcggcggatcggctggccaagctcgaagaacaacgagcgcgaatcaatgccgaaattcagcgggtgcgggcaagggaacagcagcaagagcgcaagaacgaaacaaggcgcaaggtgctggtgggggccatgattttggccaaggtgaacagcagcgagtggccggaggatcggctcatggcggcaatggatgcgtaccttgaacgcgaccacgaccgcgccttgttcggtctgccgccacgccagaaggatgagccgggctgaatgatcgaccgagacaggccctgcggggctgcacacgcgcccccacccttcgggtagggggaaaggccgctaaagcggctaaaagcgctccagcgtatttctgcggggtttggtgtggggtttagcgggctttgcccgcctttccccctgccgcgcagcggtggggcggtgtgtagcctagcgcagcgaatagaccagctatccggcctctggccgggcatattgggcaagggcagcagcgccccacaagggcgctgataaccgcgcctagtggattattcttagataatcatggatggatttttccaacaccccgccagcccccgcccctgctgggtttgcaggtttgggggcgtgacagttattgcaggggttcgtgacagttattgcaggggggcgtgacagttattgcaggggttcgtgacagttagtacgggagtgacgggcactggctggcaatgtctagcaacggcaggcatttcggctgagggtaaaagaactttccgctaagcgatagactgtatgtaaacacagtattgcaaggacgcggaacatgcctcatgtggcggccctcgcgagaattaattcagataaaaaaaatccttagctttcgctaaggatgatttctagcgatgaccctgctgattggttcgctgaccgtagactggttggcttggtttcatcagccatccgcttgccctcatctgttacgccggcggtagccggccagcctcgcagagcaggattcccgttgagcaccgccaggtgcgaataagggacagtgaagaaggaacacccgctcgcgggtgggcctacttcacctatcctgcccggctgacgccgttggatacaccaaggaaagtctacacgaaccctttggcaaaatcctgtatatcgtgcgacatcgcgcgcgcgcgcgcggatgctagtacgttgtgtctcaaaatctctgatgttacattgcacaagataaaaatatatcatcatgaacaataaaactgtctgcttacataaacagtaatacaaggggtgttatgagccatattcaacgggaaacgtcttgctcgaggccgcgattaaattccaacatggatgctgatttatatgggtataaatgggctcgcgataatgtcgggcaatcaggtgcgacaatctatcgattgtatgggaagcccgatgcgccagagttgtttctgaaacatggcaaaggtagcgttgccaatgatgttacagatgagatggtcagactaaactggctgacggaatttatgcctcttccgaccatcaagcattttatccgtactcctgatgatgcatggttactcaccactgcgatccccgggaaaacagcattccaggtattagaagaatatcctgattcaggtgaaaatattgttgatgcgctggcagtgttcctgcgccggttgcattcgattcctgtttgtaattgtccttttaacagcgatcgcgtatttcgtctcgctcaggcgcaatcacgaatgaataacggtttggttgatgcgagtgattttgatgacgagcgtaatggctggcctgttgaacaagtctggaaagaaatgcataagcttttgccattctcaccggattcagtcgtcactcatggtgatttctcacttgataaccttatttttgacgaggggaaattaataggttgtattgatgttggacgagtcggaatcgcagaccgataccaggatcttgccatcctatggaactgcctcggtgagttttctccttcattacagaaacggctttttcaaaaatatggtattgataatcctgatatgaataaattgcagtttcatttgatgctcgatgagtttttctaatcagaattggttaattggttgtaacactggcagagcattacgctgacttgacgggacggcggctttgttgaataaatcgaacttttgctgagttgaaggatcagatcacgcatcttcccgacaacgcagaccgttccgtggcaaagcaaaagttcaaaatcaccaactggtccacctacaacaaagctctcatcaaccgtggctccctcactttctggctggatgatggggcgattcaggcctggtatgagtcagcaacaccttcttcacgaggcagacctcagcgctattctgaccttgccatcacgactgtgctggtcattaaacgcgtattcaggctgaccctgcgcgctgcgcagggctttattgattccatttttacactgatgaatgttccgttgcgctgcccggattacagatcctctagataatgaattctataggtaccataaataaggttttcccctgatgctgccacgcgtgactagtatgtggagccacccgcagttcgaaaaaggatcaagcaaaggagaagaacttttcactggatccaagctttctagaatcgggggcccccggggggattctagaacaatgga

SEQ ID NO: 6 - DNA, 35 bp, synthetic construct
  source 1..35: mol_type = other DNA
ttgacagctagctcagtcctaggtataatgctagc

SEQ ID NO: 7 - DNA, 35 bp, synthetic construct
  source 1..35: mol_type = other DNA
ttgacggctagctcagtcctaggtatagtgctagc

SEQ ID NO: 8 - DNA, 35 bp, synthetic construct
  source 1..35: mol_type = other DNA
tttatggctagctcagtcctaggtacaatgctagc

SEQ ID NO: 9 - DNA, 28 bp, synthetic construct
  source 1..28: mol_type = other DNA
tctagagaaagaggagaaatactagatg

SEQ ID NO: 10 - DNA, 28 bp, synthetic construct
  source 1..28: mol_type = other DNA
tctagagaaagaggggaaatactagatg

SEQ ID NO: 11 - DNA, 30 bp, synthetic construct
  source 1..30: mol_type = other DNA
tctagagtcacacaggaaacctactagatg

SEQ ID NO: 12 - DNA, 33 bp, synthetic construct
  source 1..33: mol_type = other DNA
tgtcttactagtatggagagtcataccgaaacc

SEQ ID NO: 13 - DNA, 39 bp, synthetic construct
  source 1..39: mol_type = other DNA
tgtcttggatccttattccttcaccaaagtataagaacc

SEQ ID NO: 14 - DNA, 34 bp, synthetic construct
  source 1..34: mol_type = other DNA
tgtcttggatccttctttagtgttcccatatcgc

SEQ ID NO: 15 - DNA, 36 bp, synthetic construct
  source 1..36: mol_type = other DNA
tgtcttggatccctagttactagcttgcttttgaag

SEQ ID NO: 16 - DNA, 34 bp, synthetic construct
  source 1..34: mol_type = other DNA
tgtcttgaattcgatgaaaaattcgttgcttcgg

SEQ ID NO: 17 - DNA, 39 bp, synthetic construct
  source 1..39: mol_type = other DNA
tgtcttactagtatgaaaacttttgaactgaatgaatcc

SEQ ID NO: 18 - DNA, 31 bp, synthetic construct
  source 1..31: mol_type = other DNA
taccttggatcctcaggaagcttggttctcg

SEQ ID NO: 19 - DNA, 9952 bp, synthetic construct
  source 1..9952: mol_type = other DNA
agtcctcgtctcgccctcgaattagcccgcttaatgagcgggctttttttgaattaattctcgcgagctggcacgacaggtttcccgactggaaagcgggcagtgagcgcaacgcaattaatgtaagttagcgcgaattgcaagctggccgacgcgctgggctacgtcttgctggcgttcgggagcagaagagcatacatctggaagcaaagccaggaaagcggcctatggagctgtgcggcagcgctcagtaggcaatttttcaaaatattgttaagccttttctgagcatggtatttttcatggtattaccaattagcaggaaaataagccattgaatataaaagataaaaatgtcttgtttacaatagagtggggggggtcagcctgccgccttgggccgggtgatgtcgtacttgcccgccgcgaactcggttaccgtccagcccagcgcgaccagctccggcaacgcctcgcgcacccgctggcggcgcttgcgcatggtcgaaccactggcctctgacggccagacatagccgcacaaggtatctatggaagccttgccggttttgccggggtcgatccagccacacagccgctggtgcagcaggcgggcggtttcgctgtccagcgcccgcacctcgtccatgctgatgcgcacatgctggccgccacccatgacggcctgcgcgatcaaggggttcagggccacgtacaggcgcccgtccgcctcgtcgctggcgtactccgacagcagccgaaacccctgccgcttgcggccattctgggcgatgatggataccttccaaaggcgctcgatgcagtcctgtatgtgcttgagcgccccaccactatcgacctctgccccgatttcctttgccagcgcccgatagctacctttgaccaccatggcatcagcggtgacggcctcccacttgggttccaggaacagccggagctgccgtccgccttcggtcttgggttccgggccaagcactaggccattaggcccagccatggccaccagcccttgcaggatgcgcagatcatcagcgcccagcggctccgggccgctgaactcgatccgcttgccgtcgccgtagtcatacgtcacgtccagcttgctgcgcttgcgctcgccccgcttgagggcacggaacaggccgggggccagacagtgcgccgggtcgtgtcggacgtggctgaggctgtgcttgttcttaggcttcaccacggggcacccccttgctcttgcgctgcctctccagcacggcgggcttgagcaccccgccgtcatgccgcctgaaccaccgatcagcgaacggtgcgccatagttggccttgctcacaccgaagcggacgaagaaccggcgctggtcgtcgtccacaccccattcctcggcctcggcgctggtcatgctcgacaggtaggactgccagcggatgttatcgaccagtaccgagctgccccggctggcctgctgctggtcgcctgcgcccatcatggccgcgcccttgctggcatggtgcaggaacacgatagagcacccggtatcggcggcgatggcctccatgcgaccgatgacctgggccatggggccgctggcgttttcttcctcgatgtggaaccggcgcagcgtgtccagcaccatcaggcggcggccctcggcggcgcgcttgaggccgtcgaaccactccggggccatgatgttgggcaggctgccgatcagcggctggatcagcaggccgtcagccacggcttgccgttcctcggcgctgaggtgcgccccaagggcgtgcaggcggtgatgaatggcggtgggcgggtcttcggcgggcaggtagatcaccgggccggtgggcagttcgcccacctccagcagatccggcccgcctgcaatctgtgcggccagttgcagggccagcatggatttaccggcaccaccgggcgacaccagcgccccgaccgtaccggccaccatgttgggcaaaacgtagtccagcggtggcggcgctgctgcgaacgcctccagaatattgataggcttatgggtagccattgattgcctcctttgcaggcagttggtggttaggcgctggcggggtcactacccccgccctgcgccgctctgagttcttccaggcactcgcgcagcgcctcgtattcgtcgtcggtcagccagaacttgcgctgacgcatccctttggccttcatgcgctcggcatatcgcgcttggcgtacagcgtcagggctggccagcaggtcgccggtctgcttgtccttttggtctttcatatcagtcaccgagaaacttgccggggccgaaaggcttgtcttcgcggaacaaggacaaggtgcagccgtcaaggttaaggctggccatatcagcgactgaaaagcggccagcctcggccttgtttgacgtataaccaaagccaccgggcaaccaatagcccttgtcacttttgatcaggtagaccgaccctgaagcgcttttttcgtattccataaaacccccttctgtgcgtgagtactcatagtataacaggcgtgagtaccaacgcaagcactacatgctgaaatctggcccgcccctgtccatgcctcgctggcggggtgccggtgcccgtgccagctcggcccgcgcaagctggacgctgggcagacccatgaccttgctgacggtgcgctcgatgtaatccgcttcgtggccgggcttgcgctctgccagcgctgggctggcctcggccatggccttgccgatttcctcggcactgcggccccggctggccagcttctgcgcggcgataaagtcgcacttgctgaggtcatcaccgaagcgcttgaccagcccggccatctcgctgcggtactcgtccagcgccgtgcgccggtggcggctaagctgccgctcggacagttcgaggctggccagcctgcgggccttctcctgctgccgctgggcctgctcgatctgctggccagcctgctgcaccagcgccgggccagcggtggcggtcttgcccttggattcacgcagcagcacccacggctgataaccggcgcgggtggtgtgcttgtccttgcggttggtgaagcccgccaagcggccatagtggcggctgtcggcgctggccgggtcggcgtcgtactcgctggccagcgtccgggcaatctgcccccgaagttcaccgcctgcggcgtcggccaccttgacccatgcctgatagttcttcgggctggtttccactaccagggcaggctcccggccctcggctttcatgtcatccaggtcaaactcgctgaggtcgtccaccagcaccagaccatgccgctcctgctcggcgggcctgatatacacgtcattgccctgggcattcatccgcttgagccatggcgtgttctggagcacttcggcggctgaccattcccggttcatcatctggccggtggtggcgtccctgacgccgatatcgaagcgctcacagcccatggccttgagctgtcggcctatggcctgcaaagtcctgtcgttcttcatcgggccaccaagcgcagccagatcgagccgtcctcggttgtcagtggcgtcaggtcgagcaagagcaacgatgcgatcagcagcaccaccgtaggcatcatggaagccagcatcacggttagccatagcttccagtgccacccccgcgacgcgctccgggcgctctgcgcggcgctgctcacctcggcggctacctcccgcaactctttggccagctccacccatgccgcccctgtctggcgctgggctttcagccactccgccgcctgcgcctcgctggcctgctgggtctggctcatgacctgccgggcttcgtcggccagtgtcgccatgctctgggccagcggttcgatctgctccgctaactcgttgatgcctctggatttcttcactctgtcgattgcgttcatggtctattgcctcccggtattcctgtaagtcgatgatctgggcgttggcggtgtcgatgttcagggccacgtctgcccggtcggtgcggatgccccggccttccatctccaccacgttcggccccaggtgaacaccgggcaggcgctcgatgccctgcgcctcaagtgttctgtggtcaatgcgggcgtcgtggcctgcccgctctaatgcccggttggcatggtcggcccatgcctcgcgggtctgctcaagccatgccttgggcttgagcgcttcggtcttctgtgccccgcccttctccggggtcttgccgttgtaccgcttgaaccactgagcggcgggccgctcgatgccgtcattgatccgctcggagatcatcaggtggcagtgcgggttctcgccgccaccggcatggatggccagcgtatacggcaggcgctcggcaccggtcaggtgctgggcgaactcggacgccagcgccttctgctggtcgagggtcagctcgaccggcagggcaaattcgacctccttgaacagccgcccattggcgcgttcatacaggtcggcagcatcccagtagtcggcgggccgctcgacgaactccggcatgtgcccggattcggcgtgcaagacttcatccatgtcgcgggcatacttgccttcgcgctggatgaagtcggccttggccctggccgattggccgcccgacctgctgccggttttcgccgtaaggtgataaatcgccatgctgcctcgctgttgcttttgcttttcggctccatgcaatggccctcggagagcgcaccgcccgaagggtggccgttaggccagtttctcgaagagaaaccggtaagtgcgccctcccctacaaagtagggtcgggattgccgccgctgtgcctccatgatagcctacgagacagcacattaacaatggggtgtcaagatggttaaggggagcaacaaggcggcggatcggctggccaagctcgaagaacaacgagcgcgaatcaatgccgaaattcagcgggtgcgggcaagggaacagcagcaagagcgcaagaacgaaacaaggcgcaaggtgctggtgggggccatgattttggccaaggtgaacagcagcgagtggccggaggatcggctcatggcggcaatggatgcgtaccttgaacgcgaccacgaccgcgccttgttcggtctgccgccacgccagaaggatgagccgggctgaatgatcgaccgagacaggccctgcggggctgcacacgcgcccccacccttcgggtagggggaaaggccgctaaagcggctaaaagcgctccagcgtatttctgcggggtttggtgtggggtttagcgggctttgcccgcctttccccctgccgcgcagcggtggggcggtgtgtagcctagcgcagcgaatagaccagctatccggcctctggccgggcatattgggcaagggcagcagcgccccacaagggcgctgataaccgcgcctagtggattattcttagataatcatggatggatttttccaacaccccgccagcccccgcccctgctgggtttgcaggtttgggggcgtgacagttattgcaggggttcgtgacagttattgcaggggggcgtgacagttattgcaggggttcgtgacagttagtacgggagtgacgggcactggctggcaatgtctagcaacggcaggcatttcggctgagggtaaaagaactttccgctaagcgatagactgtatgtaaacacagtattgcaaggacgcggaacatgcctcatgtggcggccctcgcgagaattaattcagataaaaaaaatccttagctttcgctaaggatgatttctagcgatgaccctgctgattggttcgctgaccgtagactggttggcttggtttcatcagccatccgcttgccctcatctgttacgccggcggtagccggccagcctcgcagagcaggattcccgttgagcaccgccaggtgcgaataagggacagtgaagaaggaacacccgctcgcgggtgggcctacttcacctatcctgcccggctgacgccgttggatacaccaaggaaagtctacacgaaccctttggcaaaatcctgtatatcgtgcgacatcgcgcgcgcgcgcgcggatgctagtacgttgtgtctcaaaatctctgatgttacattgcacaagataaaaatatatcatcatgaacaataaaactgtctgcttacataaacagtaatacaaggggtgttatgagccatattcaacgggaaacgtcttgctcgaggccgcgattaaattccaacatggatgctgatttatatgggtataaatgggctcgcgataatgtcgggcaatcaggtgcgacaatctatcgattgtatgggaagcccgatgcgccagagttgtttctgaaacatggcaaaggtagcgttgccaatgatgttacagatgagatggtcagactaaactggctgacggaatttatgcctcttccgaccatcaagcattttatccgtactcctgatgatgcatggttactcaccactgcgatccccgggaaaacagcattccaggtattagaagaatatcctgattcaggtgaaaatattgttgatgcgctggcagtgttcctgcgccggttgcattcgattcctgtttgtaattgtccttttaacagcgatcgcgtatttcgtctcgctcaggcgcaatcacgaatgaataacggtttggttgatgcgagtgattttgatgacgagcgtaatggctggcctgttgaacaagtctggaaagaaatgcataagcttttgccattctcaccggattcagtcgtcactcatggtgatttctcacttgataaccttatttttgacgaggggaaattaataggttgtattgatgttggacgagtcggaatcgcagaccgataccaggatcttgccatcctatggaactgcctcggtgagttttctccttcattacagaaacggctttttcaaaaatatggtattgataatcctgatatgaataaattgcagtttcatttgatgctcgatgagtttttctaatcagaattggttaattggttgtaacactggcagagcattacgctgacttgacgggacggcggctttgttgaataaatcgaacttttgctgagttgaaggatcagatcacgcatcttcccgacaacgcagaccgttccgtggcaaagcaaaagttcaaaatcaccaactggtccacctacaacaaagctctcatcaaccgtggctccctcactttctggctggatgatggggcgattcaggcctggtatgagtcagcaacaccttcttcacgaggcagacctcagcgctattctgaccttgccatcacgactgtgctggtcattaaacgcgtattcaggctgaccctgcgcgctgcgcagggctttattgattccatttttacactgatgaatgttccgttgcgctgcccggattacagatcctctagataatgaattctataggtaccttgacggctagctcagtcctaggtatagtgctagcactagagaaagaggggaaatactagtatggagagtcataccgaaacctttaattctcataaaacaaaacccaaacctgatattcagttcagaaaaccgacgctggcggatggtgaagccatctatcgcttgattgagcgatgcccgccgttggatttgaactcgagttatctctatttcctgcaggcatcgcattttgccgatacctgtgtggttgcagaaatggacggtgagctggtgggcttcgtttccgcctattacttgcctgaagagccgcgctcattgtttgtttggcagattgccgtagacgaaatcgcgcgaggccaaggcttagcgaagcgattgattcgtcaattactggcgaaccagagcaaaagctatgtcaccgaaattctctgcaccatcagtccatccaacaaggcctcccaagcgttgttcaacggctttgccaatgacgaaggcttgaaggtagtcgttgaaccctttttaaccgaagcgcacttttccagtcttggacacgaggctgaagaactttatcgcttggcagcaccaaagcatcagaacctgtttgcctactggcgataagaaaaactattaaaaatctaaggaaagctaacatgacaacagaaaaattaagtgtatttaatcaatacgaatcggaagtgagaggctatatccgctctttcccaaccctattttcaaaatcgaaaatggcagaaatctgggacgatgacggtaaacgttacgtcgatttctttgccggcgcgggcgcgttgaactacgggcacaacaatccggttatcaacgatgcggtcatcaagtatttgcaggaagacggtatcggccatgcactggatatggcgacagtagcgaaacgcgactttattgagtcgttcgtcaataacatcctcaagccacgaaatctggattacaaaattcaattcgtaggaccaaccggtaccaatgccatcgaaaccgcattgaaaatcgccagaaaggtcaagggtcgtaaacaagtgatgtctttcactaacggcttccatggtatgtcgatgggatcgctgagtatcaccggtaacagttactaccacgacgaaagctatggtgtgccgggttacaccactcaggtgcctttccataactacctgggcgacaaggtcgataccatcgcttatctacacaaaattctagaagatgcttccagtgggacggaactgcctgccgccatcgttttggaaaccattcaggcggaagggggcatcaacgttgccggcgcgccttggctgaaatcgctgagagagatttgtgacaaattcgatatcttgttgatcgtcgatgacattcaagctggtaacggacgctcaagtgatttcttcagcttcgaacgtgctggtatcgtccctgatattgtcactttatcgaaatctgtcgggggtgggcatccgatgtcgattgttttgatgaaaccagagttggacaaatggagtccgggtgaacactcaggaactttccgtgggtttaacttggcgtttgtcgcggcgaaggcagcgattgacaaatattggtcaaacaaagacttccaagcggaaatcaaacaaaaatctgagtgggtgcaacagcgtatgcagcaactggcgttgaaattcccgaaagcgattcgtgaaattcgcggtcacggcatgatctggggtgcggagttcagagaccctgaagtcgcgtcaaaagtctgtgaggcgtcattccatgaaggcttggtggtggaaaccgccggcgcggaaggtgaagtcatcaaattcctcgggcctttgatcatcaccaaagagttgatcgacgaaggtttcgacattctggaatcagcgaccacaaaagtgctcgccaagaaataacccttttagtaaccaatttagacaggagtaaatcatgattgtaagaaatctatacgacgatattatcggaaccgaagcggatgtagatggtgggcaatgggtcagccgccgcttgttgctggggaaagatgggatgggattctctttccatgacaccatcatcaaagaaggtgagatttgccatttttggtataaaaaccatcttgaagcggtgtattgcattgcgggtgaaggggaaatctacgacaaggcgaccggtatcacgcacccgattcgtgaagggacgatctatgcattgaacgagcatgatcgccatatccttagcgccaacaaaggcactgaactgcgtttggtgtgtgccttcaatccaccggtcacggggcgcgaaacccatgatgaagatggttcttatactttggtgaaggaataaggatcctgaagatccaacgctcggttgccgccgggcgttttttattctgcaggagcagaagagcatacatctggaagctttctagaatcgggggcccccggggggattctagaacaatgga

SEQ ID NO: 20 - DNA, 11444 bp, synthetic construct
  source 1..11444: mol_type = other DNA
agtcctcgtctcgccctcgaattagcccgcttaatgagcgggctttttttgaattaattctcgcgagctggcacgacaggtttcccgactggaaagcgggcagtgagcgcaacgcaattaatgtaagttagcgcgaattgcaagctggccgacgcgctgggctacgtcttgctggcgttcgggagcagaagagcatacatctggaagcaaagccaggaaagcggcctatggagctgtgcggcagcgctcagtaggcaatttttcaaaatattgttaagccttttctgagcatggtatttttcatggtattaccaattagcaggaaaataagccattgaatataaaagataaaaatgtcttgtttacaatagagtggggggggtcagcctgccgccttgggccgggtgatgtcgtacttgcccgccgcgaactcggttaccgtccagcccagcgcgaccagctccggcaacgcctcgcgcacccgctggcggcgcttgcgcatggtcgaaccactggcctctgacggccagacatagccgcacaaggtatctatggaagccttgccggttttgccggggtcgatccagccacacagccgctggtgcagcaggcgggcggtttcgctgtccagcgcccgcacctcgtccatgctgatgcgcacatgctggccgccacccatgacggcctgcgcgatcaaggggttcagggccacgtacaggcgcccgtccgcctcgtcgctggcgtactccgacagcagccgaaacccctgccgcttgcggccattctgggcgatgatggataccttccaaaggcgctcgatgcagtcctgtatgtgcttgagcgccccaccactatcgacctctgccccgatttcctttgccagcgcccgatagctacctttgaccaccatggcatcagcggtgacggcctcccacttgggttccaggaacagccggagctgccgtccgccttcggtcttgggttccgggccaagcactaggccattaggcccagccatggccaccagcccttgcaggatgcgcagatcatcagcgcccagcggctccgggccgctgaactcgatccgcttgccgtcgccgtagtcatacgtcacgtccagcttgctgcgcttgcgctcgccccgcttgagggcacggaacaggccgggggccagacagtgcgccgggtcgtgtcggacgtggctgaggctgtgcttgttcttaggcttcaccacggggcacccccttgctcttgcgctgcctctccagcacggcgggcttgagcaccccgccgtcatgccgcctgaaccaccgatcagcgaacggtgcgccatagttggccttgctcacaccgaagcggacgaagaaccggcgctggtcgtcgtccacaccccattcctcggcctcggcgctggtcatgctcgacaggtaggactgccagcggatgttatcgaccagtaccgagctgccccggctggcctgctgctggtcgcctgcgcccatcatggccgcgcccttgctggcatggtgcaggaacacgatagagcacccggtatcggcggcgatggcctccatgcgaccgatgacctgggccatggggccgctggcgttttcttcctcgatgtggaaccggcgcagcgtgtccagcaccatcaggcggcggccctcggcggcgcgcttgaggccgtcgaaccactccggggccatgatgttgggcaggctgccgatcagcggctggatcagcaggccgtcagccacggcttgccgttcctcggcgctgaggtgcgccccaagggcgtgcaggcggtgatgaatggcggtgggcgggtcttcggcgggcaggtagatcaccgggccggtgggcagttcgcccacctccagcagatccggcccgcctgcaatctgtgcggccagttgcagggccagcatggatttaccggcaccaccgggcgacaccagcgccccgaccgtaccggccaccatgttgggcaaaacgtagtccagcggtggcggcgctgctgcgaacgcctccagaatattgataggcttatgggtagccattgattgcctcctttgcaggcagttggtggttaggcgctggcggggtcactacccccgccctgcgccgctctgagttcttccaggcactcgcgcagcgcctcgtattcgtcgtcggtcagccagaacttgcgctgacgcatccctttggccttcatgcgctcggcatatcgcgcttggcgtacagcgtcagggctggccagcaggtcgccggtctgcttgtccttttggtctttcatatcagtcaccgagaaacttgccggggccgaaaggcttgtcttcgcggaacaaggacaaggtgcagccgtcaaggttaaggctggccatatcagcgactgaaaagcggccagcctcggccttgtttgacgtataaccaaagccaccgggcaaccaatagcccttgtcacttttgatcaggtagaccgaccctgaagcgcttttttcgtattccataaaacccccttctgtgcgtgagtactcatagtataacaggcgtgagtaccaacgcaagcactacatgctgaaatctggcccgcccctgtccatgcctcgctggcggggtgccggtgcccgtgccagctcggcccgcgcaagctggacgctgggcagacccatgaccttgctgacggtgcgctcgatgtaatccgcttcgtggccgggcttgcgctctgccagcgctgggctggcctcggccatggccttgccgatttcctcggcactgcggccccggctggccagcttctgcgcggcgataaagtcgcacttgctgaggtcatcaccgaagcgcttgaccagcccggccatctcgctgcggtactcgtccagcgccgtgcgccggtggcggctaagctgccgctcggacagttcgaggctggccagcctgcgggccttctcctgctgccgctgggcctgctcgatctgctggccagcctgctgcaccagcgccgggccagcggtggcggtcttgcccttggattcacgcagcagcacccacggctgataaccggcgcgggtggtgtgcttgtccttgcggttggtgaagcccgccaagcggccatagtggcggctgtcggcgctggccgggtcggcgtcgtactcgctggccagcgtccgggcaatctgcccccgaagttcaccgcctgcggcgtcggccaccttgacccatgcctgatagttcttcgggctggtttccactaccagggcaggctcccggccctcggctttcatgtcatccaggtcaaactcgctgaggtcgtccaccagcaccagaccatgccgctcctgctcggcgggcctgatatacacgtcattgccctgggcattcatccgcttgagccatggcgtgttctggagcacttcggcggctgaccattcccggttcatcatctggccggtggtggcgtccctgacgccgatatcgaagcgctcacagcccatggccttgagctgtcggcctatggcctgcaaagtcctgtcgttcttcatcgggccaccaagcgcagccagatcgagccgtcctcggttgtcagtggcgtcaggtcgagcaagagcaacgatgcgatcagcagcaccaccgtaggcatcatggaagccagcatcacggttagccatagcttccagtgccacccccgcgacgcgctccgggcgctctgcgcggcgctgctcacctcggcggctacctcccgcaactctttggccagctccacccatgccgcccctgtctggcgctgggctttcagccactccgccgcctgcgcctcgctggcctgctgggtctggctcatgacctgccgggcttcgtcggccagtgtcgccatgctctgggccagcggttcgatctgctccgctaactcgttgatgcctctggatttcttcactctgtcgattgcgttcatggtctattgcctcccggtattcctgtaagtcgatgatctgggcgttggcggtgtcgatgttcagggccacgtctgcccggtcggtgcggatgccccggccttccatctccaccacgttcggccccaggtgaacaccgggcaggcgctcgatgccctgcgcctcaagtgttctgtggtcaatgcgggcgtcgtggcctgcccgctctaatgcccggttggcatggtcggcccatgcctcgcgggtctgctcaagccatgccttgggcttgagcgcttcggtcttctgtgccccgcccttctccggggtcttgccgttgtaccgcttgaaccactgagcggcgggccgctcgatgccgtcattgatccgctcggagatcatcaggtggcagtgcgggttctcgccgccaccggcatggatggccagcgtatacggcaggcgctcggcaccggtcaggtgctgggcgaactcggacgccagcgccttctgctggtcgagggtcagctcgaccggcagggcaaattcgacctccttgaacagccgcccattggcgcgttcatacaggtcggcagcatcccagtagtcggcgggccgctcgacgaactccggcatgtgcccggattcggcgtgcaagacttcatccatgtcgcgggcatacttgccttcgcgctggatgaagtcggccttggccctggccgattggccgcccgacctgctgccggttttcgccgtaaggtgataaatcgccatgctgcctcgctgttgcttttgcttttcggctccatgcaatggccctcggagagcgcaccgcccgaagggtggccgttaggccagtttctcgaagagaaaccggtaagtgcgccctcccctacaaagtagggtcgggattgccgccgctgtgcctccatgatagcctacgagacagcacattaacaatggggtgtcaagatggttaaggggagcaacaaggcggcggatcggctggccaagctcgaagaacaacgagcgcgaatcaatgccgaaattcagcgggtgcgggcaagggaacagcagcaagagcgcaagaacgaaacaaggcgcaaggtgctggtgggggccatgattttggccaaggtgaacagcagcgagtggccggaggatcggctcatggcggcaatggatgcgtaccttgaacgcgaccacgaccgcgccttgttcggtctgccgccacgccagaaggatgagccgggctgaatgatcgaccgagacaggccctgcggggctgcacacgcgcccccacccttcgggtagggggaaaggccgctaaagcggctaaaagcgctccagcgtatttctgcggggtttggtgtggggtttagcgggctttgcccgcctttccccctgccgcgcagcggtggggcggtgtgtagcctagcgcagcgaatagaccagctatccggcctctggccgggcatattgggcaagggcagcagcgccccacaagggcgctgataaccgcgcctagtggattattcttagataatcatggatggatttttccaacaccccgccagcccccgcccctgctgggtttgcaggtttgggggcgtgacagttattgcaggggttcgtgacagttattgcaggggggcgtgacagttattgcaggggttcgtgacagttagtacgggagtgacgggcactggctggcaatgtctagcaacggcaggcatttcggctgagggtaaaagaactttccgctaagcgatagactgtatgtaaacacagtattgcaaggacgcggaacatgcctcatgtggcggccctcgcgagaattaattcagataaaaaaaatccttagctttcgctaaggatgatttctagcgatgaccctgctgattggttcgctgaccgtagactggttggcttggtttcatcagccatccgcttgccctcatctgttacgccggcggtagccggccagcctcgcagagcaggattcccgttgagcaccgccaggtgcgaataagggacagtgaagaaggaacacccgctcgcgggtgggcctacttcacctatcctgcccggctgacgccgttggatacaccaaggaaagtctacacgaaccctttggcaaaatcctgtatatcgtgcgacatcgcgcgcgcgcgcgcggatgctagtacgttgtgtctcaaaatctctgatgttacattgcacaagataaaaatatatcatcatgaacaataaaactgtctgcttacataaacagtaatacaaggggtgttatgagccatattcaacgggaaacgtcttgctcgaggccgcgattaaattccaacatggatgctgatttatatgggtataaatgggctcgcgataatgtcgggcaatcaggtgcgacaatctatcgattgtatgggaagcccgatgcgccagagttgtttctgaaacatggcaaaggtagcgttgccaatgatgttacagatgagatggtcagactaaactggctgacggaatttatgcctcttccgaccatcaagcattttatccgtactcctgatgatgcatggttactcaccactgcgatccccgggaaaacagcattccaggtattagaagaatatcctgattcaggtgaaaatattgttgatgcgctggcagtgttcctgcgccggttgcattcgattcctgtttgtaattgtccttttaacagcgatcgcgtatttcgtctcgctcaggcgcaatcacgaatgaataacggtttggttgatgcgagtgattttgatgacgagcgtaatggctggcctgttgaacaagtctggaaagaaatgcataagcttttgccattctcaccggattcagtcgtcactcatggtgatttctcacttgataaccttatttttgacgaggggaaattaataggttgtattgatgttggacgagtcggaatcgcagaccgataccaggatcttgccatcctatggaactgcctcggtgagttttctccttcattacagaaacggctttttcaaaaatatggtattgataatcctgatatgaataaattgcagtttcatttgatgctcgatgagtttttctaatcagaattggttaattggttgtaacactggcagagcattacgctgacttgacgggacggcggctttgttgaataaatcgaacttttgctgagttgaaggatcagatcacgcatcttcccgacaacgcagaccgttccgtggcaaagcaaaagttcaaaatcaccaactggtccacctacaacaaagctctcatcaaccgtggctccctcactttctggctggatgatggggcgattcaggcctggtatgagtcagcaacaccttcttcacgaggcagacctcagcgctattctgaccttgccatcacgactgtgctggtcattaaacgcgtattcaggctgaccctgcgcgctgcgcagggctttattgattccatttttacactgatgaatgttccgttgcgctgcccggattacagatcctctagataatgaattctataggtaccttgacggctagctcagtcctaggtatagtgctagcactagagaaagaggggaaatactagtatggagagtcataccgaaacctttaattctcataaaacaaaacccaaacctgatattcagttcagaaaaccgacgctggcggatggtgaagccatctatcgcttgattgagcgatgcccgccgttggatttgaactcgagttatctctatttcctgcaggcatcgcattttgccgatacctgtgtggttgcagaaatggacggtgagctggtgggcttcgtttccgcctattacttgcctgaagagccgcgctcattgtttgtttggcagattgccgtagacgaaatcgcgcgaggccaaggcttagcgaagcgattgattcgtcaattactggcgaaccagagcaaaagctatgtcaccgaaattctctgcaccatcagtccatccaacaaggcctcccaagcgttgttcaacggctttgccaatgacgaaggcttgaaggtagtcgttgaaccctttttaaccgaagcgcacttttccagtcttggacacgaggctgaagaactttatcgcttggcagcaccaaagcatcagaacctgtttgcctactggcgataagaaaaactattaaaaatctaaggaaagctaacatgacaacagaaaaattaagtgtatttaatcaatacgaatcggaagtgagaggctatatccgctctttcccaaccctattttcaaaatcgaaaatggcagaaatctgggacgatgacggtaaacgttacgtcgatttctttgccggcgcgggcgcgttgaactacgggcacaacaatccggttatcaacgatgcggtcatcaagtatttgcaggaagacggtatcggccatgcactggatatggcgacagtagcgaaacgcgactttattgagtcgttcgtcaataacatcctcaagccacgaaatctggattacaaaattcaattcgtaggaccaaccggtaccaatgccatcgaaaccgcattgaaaatcgccagaaaggtcaagggtcgtaaacaagtgatgtctttcactaacggcttccatggtatgtcgatgggatcgctgagtatcaccggtaacagttactaccacgacgaaagctatggtgtgccgggttacaccactcaggtgcctttccataactacctgggcgacaaggtcgataccatcgcttatctacacaaaattctagaagatgcttccagtgggacggaactgcctgccgccatcgttttggaaaccattcaggcggaagggggcatcaacgttgccggcgcgccttggctgaaatcgctgagagagatttgtgacaaattcgatatcttgttgatcgtcgatgacattcaagctggtaacggacgctcaagtgatttcttcagcttcgaacgtgctggtatcgtccctgatattgtcactttatcgaaatctgtcgggggtgggcatccgatgtcgattgttttgatgaaaccagagttggacaaatggagtccgggtgaacactcaggaactttccgtgggtttaacttggcgtttgtcgcggcgaaggcagcgattgacaaatattggtcaaacaaagacttccaagcggaaatcaaacaaaaatctgagtgggtgcaacagcgtatgcagcaactggcgttgaaattcccgaaagcgattcgtgaaattcgcggtcacggcatgatctggggtgcggagttcagagaccctgaagtcgcgtcaaaagtctgtgaggcgtcattccatgaaggcttggtggtggaaaccgccggcgcggaaggtgaagtcatcaaattcctcgggcctttgatcatcaccaaagagttgatcgacgaaggtttcgacattctggaatcagcgaccacaaaagtgctcgccaagaaataacccttttagtaaccaatttagacaggagtaaatcatgattgtaagaaatctatacgacgatattatcggaaccgaagcggatgtagatggtgggcaatgggtcagccgccgcttgttgctggggaaagatgggatgggattctctttccatgacaccatcatcaaagaaggtgagatttgccatttttggtataaaaaccatcttgaagcggtgtattgcattgcgggtgaaggggaaatctacgacaaggcgaccggtatcacgcacccgattcgtgaagggacgatctatgcattgaacgagcatgatcgccatatccttagcgccaacaaaggcactgaactgcgtttggtgtgtgccttcaatccaccggtcacggggcgcgaaacccatgatgaagatggttcttatactttggtgaaggaataagttatcgccatgcagcataagaatgagcagggaaaacctgttgatagaacattgagcgtcgagaaaatcggcggaacctccatgagtgactatcaggcggttagggacaatattgttttctatccgcaaaacccgtatcgacgtattctggtggtgtccgcttacggcggcatgaccaacgacttgttggaacacaagaaaaccgggcaaccgggtgtctatgggttgtttgcatacaatgacgagagtgatgatggtacggagcattcctggcgcgaagctttgcgagacctctcggcaaagatgcaacagttcaacgaagagctgtttgatgaagatgacatgaaagcggcggcaaaccgctttatctccgagcgcattgaacacaccgaaaacttgttgatgcatttgcagaacctttgtcaccatggacatttttcactggaagatcatttgttgacggtgcgtgaactcttagcgagcatcggcgaagcgcacagtgcatggaacctgacgcagttgttgaaatcagaaggcatcaatgcaatttggattgatttgaccggctggcaggacgatgaaaaactgccgctggatgaagtgattcacaacaaattgtgccacctcaattatgacgaagtgctgccgattgtaaccggctatgctcactgcgaagagaacctcatgaacacctttgaccgtggctatagcgaaatgacgttcagtcgtattgcggtgttgtgtcaggcgacgcaagcggtcattcataaggaatatcatttgagtagtgccgacccgcgcttggtgggagaggaacaggcagttcccattggtaagaccaattatgacatcgctgaccagttggcgaaccttggcatggaagcgattcaccccaaagcggcaaaagggttgcgacaagcacagatccctctgttgattaaaaacacctttgagcccgagcaccacggcaccattattcgcgaagactacgtgagcgagttcccgcaagtcgagattatcgccggcaggcagaatttgatcgccgtagaagtgttcgatgccgaaatgatggggcagcagacagactatgagcaagccatttgggaaatcaccaaacgtctcagatgccaggtgctgactaaagatttcaacgccaataccatcaccctgtatctgcaagcatccttgcgaaaagccaaacgacttgccggacaattggaggtgcgtttgccgaccgccaagatttccaccagcaaagtctcattggtttcggcgatgggaagtgatatgcgtatcaaagggcttttggcgcaagctgtacagacgctatttgaagcgggcatcaatattcaagcgttgcatcaaaacctcagacaggtggaaatgcagtttttcgtcaaagagcaagattacgagcgcgcggtcaaacgcctacacgctagtttaatcgaagttcataaccatggaaaagcgatatgggaacactaaagaaggatcctgaagatccaacgctcggttgccgccgggcgttttttattctgcaggagcagaagagcatacatctggaagctttctagaatcgggggcccccggggggattctagaacaatgga

SEQ ID NO: 21 - DNA, 10608 bp, synthetic construct
  source 1..10608: mol_type = other DNA
agtcctcgtctcgccctcgaattagcccgcttaatgagcgggctttttttgaattaattctcgcgagctggcacgacaggtttcccgactggaaagcgggcagtgagcgcaacgcaattaatgtaagttagcgcgaattgcaagctggccgacgcgctgggctacgtcttgctggcgttcgggagcagaagagcatacatctggaagcaaagccaggaaagcggcctatggagctgtgcggcagcgctcagtaggcaatttttcaaaatattgttaagccttttctgagcatggtatttttcatggtattaccaattagcaggaaaataagccattgaatataaaagataaaaatgtcttgtttacaatagagtggggggggtcagcctgccgccttgggccgggtgatgtcgtacttgcccgccgcgaactcggttaccgtccagcccagcgcgaccagctccggcaacgcctcgcgcacccgctggcggcgcttgcgcatggtcgaaccactggcctctgacggccagacatagccgcacaaggtatctatggaagccttgccggttttgccggggtcgatccagccacacagccgctggtgcagcaggcgggcggtttcgctgtccagcgcccgcacctcgtccatgctgatgcgcacatgctggccgccacccatgacggcctgcgcgatcaaggggttcagggccacgtacaggcgcccgtccgcctcgtcgctggcgtactccgacagcagccgaaacccctgccgcttgcggccattctgggcgatgatggataccttccaaaggcgctcgatgcagtcctgtatgtgcttgagcgccccaccactatcgacctctgccccgatttcctttgccagcgcccgatagctacctttgaccaccatggcatcagcggtgacggcctcccacttgggttccaggaacagccggagctgccgtccgccttcggtcttgggttccgggccaagcactaggccattaggcccagccatggccaccagcccttgcaggatgcgcagatcatcagcgcccagcggctccgggccgctgaactcgatccgcttgccgtcgccgtagtcatacgtcacgtccagcttgctgcgcttgcgctcgccccgcttgagggcacggaacaggccgggggccagacagtgcgccgggtcgtgtcggacgtggctgaggctgtgcttgttcttaggcttcaccacggggcacccccttgctcttgcgctgcctctccagcacggcgggcttgagcaccccgccgtcatgccgcctgaaccaccgatcagcgaacggtgcgccatagttggccttgctcacaccgaagcggacgaagaaccggcgctggtcgtcgtccacaccccattcctcggcctcggcgctggtcatgctcgacaggtaggactgccagcggatgttatcgaccagtaccgagctgccccggctggcctgctgctggtcgcctgcgcccatcatggccgcgcccttgctggcatggtgcaggaacacgatagagcacccggtatcggcggcgatggcctccatgcgaccgatgacctgggccatggggccgctggcgttttcttcctcgatgtggaaccggcgcagcgtgtccagcaccatcaggcggcggccctcggcggcgcgcttgaggccgtcgaaccactccggggccatgatgttgggcaggctgccgatcagcggctggatcagcaggccgtcagccacggcttgccgttcctcggcgctgaggtgcgccccaagggcgtgcaggcggtgatgaatggcggtgggcgggtcttcggcgggcaggtagatcaccgggccggtgggcagttcgcccacctccagcagatccggcccgcctgcaatctgtgcggccagttgcagggccagcatggatttaccggcaccaccgggcgacaccagcgccccgaccgtaccggccaccatgttgggcaaaacgtagtccagcggtggcggcgctgctgcgaacgcctccagaatattgataggcttatgggtagccattgattgcctcctttgcaggcagttggtggttaggcgctggcggggtcactacccccgccctgcgccgctctgagttcttccaggcactcgcgcagcgcctcgtattcgtcgtcggtcagccagaacttgcgctgacgcatccctttggccttcatgcgctcggcatatcgcgcttggcgtacagcgtcagggctggccagcaggtcgccggtctgcttgtccttttggtctttcatatcagtcaccgagaaacttgccggggccgaaaggcttgtcttcgcggaacaaggacaaggtgcagccgtcaaggttaaggctggccatatcagcgactgaaaagcggccagcctcggccttgtttgacgtataaccaaagccaccgggcaaccaatagcccttgtcacttttgatcaggtagaccgaccctgaagcgcttttttcgtattccataaaacccccttctgtgcgtgagtactcatagtataacaggcgtgagtaccaacgcaagcactacatgctgaaatctggcccgcccctgtccatgcctcgctggcggggtgccggtgcccgtgccagctcggcccgcgcaagctggacgctgggcagacccatgaccttgctgacggtgcgctcgatgtaatccgcttcgtggccgggcttgcgctctgccagcgctgggctggcctcggccatggccttgccgatttcctcggcactgcggccccggctggccagcttctgcgcggcgataaagtcgcacttgctgaggtcatcaccgaagcgcttgaccagcccggccatctcgctgcggtactcgtccagcgccgtgcgccggtggcggctaagctgccgctcggacagttcgaggctggccagcctgcgggccttctcctgctgccgctgggcctgctcgatctgctggccagcctgctgcaccagcgccgggccagcggtggcggtcttgcccttggattcacgcagcagcacccacggctgataaccggcgcgggtggtgtgcttgtccttgcggttggtgaagcccgccaagcggccatagtggcggctgtcggcgctggccgggtcggcgtcgtactcgctggccagcgtccgggcaatctgcccccgaagttcaccgcctgcggcgtcggccaccttgacccatgcctgatagttcttcgggctggtttccactaccagggcaggctcccggccctcggctttcatgtcatccaggtcaaactcgctgaggtcgtccaccagcaccagaccatgccgctcctgctcggcgggcctgatatacacgtcattgccctgggcattcatccgcttgagccatggcgtgttctggagcacttcggcggctgaccattcccggttcatcatctggccggtggtggcgtccctgacgccgatatcgaagcgctcacagcccatggccttgagctgtcggcctatggcctgcaaagtcctgtcgttcttcatcgggccaccaagcgcagccagatcgagccgtcctcggttgtcagtggcgtcaggtcgagcaagagcaacgatgcgatcagcagcaccaccgtaggcatcatggaagccagcatcacggttagccatagcttccagtgccacccccgcgacgcgctccgggcgctctgcgcggcgctgctcacctcggcggctacctcccgcaactctttggccagctccacccatgccgcccctgtctggcgctgggctttcagccactccgccgcctgcgcctcgctggcctgctgggtctggctcatgacctgccgggcttcgtcggccagtgtcgccatgctctgggccagcggttcgatctgctccgctaactcgttgatgcctctggatttcttcactctgtcgattgcgttcatggtctattgcctcccggtattcctgtaagtcgatgatctgggcgttggcggtgtcgatgttcagggccacgtctgcccggtcggtgcggatgccccggccttccatctccaccacgttcggccccaggtgaacaccgggcaggcgctcgatgccctgcgcctcaagtgttctgtggtcaatgcgggcgtcgtggcctgcccgctctaatgcccggttggcatggtcggcccatgcctcgcgggtctgctcaagccatgccttgggcttgagcgcttcggtcttctgtgccccgcccttctccggggtcttgccgttgtaccgcttgaaccactgagcggcgggccgctcgatgccgtcattgatccgctcggagatcatcaggtggcagtgcgggttctcgccgccaccggcatggatggccagcgtatacggcaggcgctcggcaccggtcaggtgctgggcgaactcggacgccagcgccttctgctggtcgagggtcagctcgaccggcagggcaaattcgacctccttgaacagccgcccattggcgcgttcatacaggtcggcagcatcccagtagtcggcgggccgctcgacgaactccggcatgtgcccggattcggcgtgcaagacttcatccatgtcgcgggcatacttgccttcgcgctggatgaagtcggccttggccctggccgattggccgcccgacctgctgccggttttcgccgtaaggtgataaatcgccatgctgcctcgctgttgcttttgcttttcggctccatgcaatggccctcggagagcgcaccgcccgaagggtggccgttaggccagtttctcgaagagaaaccggtaagtgcgccctcccctacaaagtagggtcgggattgccgccgctgtgcctccatgatagcctacgagacagcacattaacaatggggtgtcaagatggttaaggggagcaacaaggcggcggatcggctggccaagctcgaagaacaacgagcgcgaatcaatgccgaaattcagcgggtgcgggcaagggaacagcagcaagagcgcaagaacgaaacaaggcgcaaggtgctggtgggggccatgattttggccaaggtgaacagcagcgagtggccggaggatcggctcatggcggcaatggatgcgtaccttgaacgcgaccacgaccgcgccttgttcggtctgccgccacgccagaaggatgagccgggctgaatgatcgaccgagacaggccctgcggggctgcacacgcgcccccacccttcgggtagggggaaaggccgctaaagcggctaaaagcgctccagcgtatttctgcggggtttggtgtggggtttagcgggctttgcccgcctttccccctgccgcgcagcggtggggcggtgtgtagcctagcgcagcgaatagaccagctatccggcctctggccgggcatattgggcaagggcagcagcgccccacaagggcgctgataaccgcgcctagtggattattcttagataatcatggatggatttttccaacaccccgccagcccccgcccctgctgggtttgcaggtttgggggcgtgacagttattgcaggggttcgtgacagttattgcaggggggcgtgacagttattgcaggggttcgtgacagttagtacgggagtgacgggcactggctggcaatgtctagcaacggcaggcatttcggctgagggtaaaagaactttccgctaagcgatagactgtatgtaaacacagtattgcaaggacgcggaacatgcctcatgtggcggccctcgcgagaattaattcagataaaaaaaatccttagctttcgctaaggatgatttctagcgatgaccctgctgattggttcgctgaccgtagactggttggcttggtttcatcagccatccgcttgccctcatctgttacgccggcggtagccggccagcctcgcagagcaggattcccgttgagcaccgccaggtgcgaataagggacagtgaagaaggaacacccgctcgcgggtgggcctacttcacctatcctgcccggctgacgccgttggatacaccaaggaaagtctacacgaaccctttggcaaaatcctgtatatcgtgcgacatcgcgcgcgcgcgcgcggatgctagtacgttgtgtctcaaaatctctgatgttacattgcacaagataaaaatatatcatcatgaacaataaaactgtctgcttacataaacagtaatacaaggggtgttatgagccatattcaacgggaaacgtcttgctcgaggccgcgattaaattccaacatggatgctgatttatatgggtataaatgggctcgcgataatgtcgggcaatcaggtgcgacaatctatcgattgtatgggaagcccgatgcgccagagttgtttctgaaacatggcaaaggtagcgttgccaatgatgttacagatgagatggtcagactaaactggctgacggaatttatgcctcttccgaccatcaagcattttatccgtactcctgatgatgcatggttactcaccactgcgatccccgggaaaacagcattccaggtattagaagaatatcctgattcaggtgaaaatattgttgatgcgctggcagtgttcctgcgccggttgcattcgattcctgtttgtaattgtccttttaacagcgatcgcgtatttcgtctcgctcaggcgcaatcacgaatgaataacggtttggttgatgcgagtgattttgatgacgagcgtaatggctggcctgttgaacaagtctggaaagaaatgcataagcttttgccattctcaccggattcagtcgtcactcatggtgatttctcacttgataaccttatttttgacgaggggaaattaataggttgtattgatgttggacgagtcggaatcgcagaccgataccaggatcttgccatcctatggaactgcctcggtgagttttctccttcattacagaaacggctttttcaaaaatatggtattgataatcctgatatgaataaattgcagtttcatttgatgctcgatgagtttttctaatcagaattggttaattggttgtaacactggcagagcattacgctgacttgacgggacggcggctttgttgaataaatcgaacttttgctgagttgaaggatcagatcacgcatcttcccgacaacgcagaccgttccgtggcaaagcaaaagttcaaaatcaccaactggtccacctacaacaaagctctcatcaaccgtggctccctcactttctggctggatgatggggcgattcaggcctggtatgagtcagcaacaccttcttcacgaggcagacctcagcgctattctgaccttgccatcacgactgtgctggtcattaaacgcgtattcaggctgaccctgcgcgctgcgcagggctttattgattccatttttacactgatgaatgttccgttgcgctgcccggattacagatcctctagataatgaattcgatgaaaaattcgttgcttcgggactcattctaggaggataagttatttaagtaaaattaaatgtttttaacatagtgatagttaaaaactattaaattcggttttatcgtgcatacaagcttgtgccctgagcttgcgtccctttattttaagtacattaaacaacaataaatatcttgtccctaatttgtgggaattttatgggataaaagtcattttttatttatcgttttttctatttttgatgacaaaaatatgaaattttccctaaaacttgagatattgagctgtttttgttaggatgtttgcaacttaaaaacccaaaaggttaaattatctattttttgaaagcactgcttgcaggtgaacgaacatttgcaggtaagaaattccaaaataaaatcctgtggaagttttctaggcgcttttcttctttagatcctcaagatgttcatttacatcccacagggtcgagtctaatccaaaggacaagtccggaggaatcaatcgtatggtcaagccataagccatccccctgttcgttagattttgctacttctgctgcatttgcaacggtttatgctgatttaagcatgctaggtcgtgaggtttattatcgcttgattgccatagtctttaagtcaatggagacgtttttcatttcatttccattgctgcgattggttgctaatcctatcagcaactcaacaacaaaggtcactcatcatggagagtcataccgaaacctttaattctcataaaacaaaacccaaacctgatattcagttcagaaaaccgacgctggcggatggtgaagccatctatcgcttgattgagcgatgcccgccgttggatttgaactcgagttatctctatttcctgcaggcatcgcattttgccgatacctgtgtggttgcagaaatggacggtgagctggtgggcttcgtttccgcctattacttgcctgaagagccgcgctcattgtttgtttggcagattgccgtagacgaaatcgcgcgaggccaaggcttagcgaagcgattgattcgtcaattactggcgaaccagagcaaaagctatgtcaccgaaattctctgcaccatcagtccatccaacaaggcctcccaagcgttgttcaacggctttgccaatgacgaaggcttgaaggtagtcgttgaaccctttttaaccgaagcgcacttttccagtcttggacacgaggctgaagaactttatcgcttggcagcaccaaagcatcagaacctgtttgcctactggcgataagaaaaactattaaaaatctaaggaaagctaacatgacaacagaaaaattaagtgtatttaatcaatacgaatcggaagtgagaggctatatccgctctttcccaaccctattttcaaaatcgaaaatggcagaaatctgggacgatgacggtaaacgttacgtcgatttctttgccggcgcgggcgcgttgaactacgggcacaacaatccggttatcaacgatgcggtcatcaagtatttgcaggaagacggtatcggccatgcactggatatggcgacagtagcgaaacgcgactttattgagtcgttcgtcaataacatcctcaagccacgaaatctggattacaaaattcaattcgtaggaccaaccggtaccaatgccatcgaaaccgcattgaaaatcgccagaaaggtcaagggtcgtaaacaagtgatgtctttcactaacggcttccatggtatgtcgatgggatcgctgagtatcaccggtaacagttactaccacgacgaaagctatggtgtgccgggttacaccactcaggtgcctttccataactacctgggcgacaaggtcgataccatcgcttatctacacaaaattctagaagatgcttccagtgggacggaactgcctgccgccatcgttttggaaaccattcaggcggaagggggcatcaacgttgccggcgcgccttggctgaaatcgctgagagagatttgtgacaaattcgatatcttgttgatcgtcgatgacattcaagctggtaacggacgctcaagtgatttcttcagcttcgaacgtgctggtatcgtccctgatattgtcactttatcgaaatctgtcgggggtgggcatccgatgtcgattgttttgatgaaaccagagttggacaaatggagtccgggtgaacactcaggaactttccgtgggtttaacttggcgtttgtcgcggcgaaggcagcgattgacaaatattggtcaaacaaagacttccaagcggaaatcaaacaaaaatctgagtgggtgcaacagcgtatgcagcaactggcgttgaaattcccgaaagcgattcgtgaaattcgcggtcacggcatgatctggggtgcggagttcagagaccctgaagtcgcgtcaaaagtctgtgaggcgtcattccatgaaggcttggtggtggaaaccgccggcgcggaaggtgaagtcatcaaattcctcgggcctttgatcatcaccaaagagttgatcgacgaaggtttcgacattctggaatcagcgaccacaaaagtgctcgccaagaaataacccttttagtaaccaatttagacaggagtaaatcatgattgtaagaaatctatacgacgatattatcggaaccgaagcggatgtagatggtgggcaatgggtcagccgccgcttgttgctggggaaagatgggatgggattctctttccatgacaccatcatcaaagaaggtgagatttgccatttttggtataaaaaccatcttgaagcggtgtattgcattgcgggtgaaggggaaatctacgacaaggcgaccggtatcacgcacccgattcgtgaagggacgatctatgcattgaacgagcatgatcgccatatccttagcgccaacaaaggcactgaactgcgtttggtgtgtgccttcaatccaccggtcacggggcgcgaaacccatgatgaagatggttcttatactttggtgaaggaataaggatcctgaagatccaacgctcggttgccgccgggcgttttttattctgcaggagcagaagagcatacatctggaagctttctagaatcgggggcccccggggggattctagaacaatgga

SEQ ID NO: 22 - DNA, 12100 bp, synthetic construct
  source 1..12100: mol_type = other DNA
agtcctcgtctcgccctcgaattagcccgcttaatgagcgggctttttttgaattaattctcgcgagctggcacgacaggtttcccgactggaaagcgggcagtgagcgcaacgcaattaatgtaagttagcgcgaattgcaagctggccgacgcgctgggctacgtcttgctggcgttcgggagcagaagagcatacatctggaagcaaagccaggaaagcggcctatggagctgtgcggcagcgctcagtaggcaatttttcaaaatattgttaagccttttctgagcatggtatttttcatggtattaccaattagcaggaaaataagccattgaatataaaagataaaaatgtcttgtttacaatagagtggggggggtcagcctgccgccttgggccgggtgatgtcgtacttgcccgccgcgaactcggttaccgtccagcccagcgcgaccagctccggcaacgcctcgcgcacccgctggcggcgcttgcgcatggtcgaaccactggcctctgacggccagacatagccgcacaaggtatctatggaagccttgccggttttgccggggtcgatccagccacacagccgctggtgcagcaggcgggcggtttcgctgtccagcgcccgcacctcgtccatgctgatgcgcacatgctggccgccacccatgacggcctgcgcgatcaaggggttcagggccacgtacaggcgcccgtccgcctcgtcgctggcgtactccgacagcagccgaaacccctgccgcttgcggccattctgggcgatgatggataccttccaaaggcgctcgatgcagtcctgtatgtgcttgagcgccccaccactatcgacctctgccccgatttcctttgccagcgcccgatagctacctttgaccaccatggcatcagcggtgacggcctcccacttgggttccaggaacagccggagctgccgtccgccttcggtcttgggttccgggccaagcactaggccattaggcccagccatggccaccagcccttgcaggatgcgcagatcatcagcgcccagcggctccgggccgctgaactcgatccgcttgccgtcgccgtagtcatacgtcacgtccagcttgctgcgcttgcgctcgccccgcttgagggcacggaacaggccgggggccagacagtgcgccgggtcgtgtcggacgtggctgaggctgtgcttgttcttaggcttcaccacggggcacccccttgctcttgcgctgcctctccagcacggcgggcttgagcaccccgccgtcatgccgcctgaaccaccgatcagcgaacggtgcgccatagttggccttgctcacaccgaagcggacgaagaaccggcgctggtcgtcgtccacaccccattcctcggcctcggcgctggtcatgctcgacaggtaggactgccagcggatgttatcgaccagtaccgagctgccccggctggcctgctgctggtcgcctgcgcccatcatggccgcgcccttgctggcatggtgcaggaacacgatagagcacccggtatcggcggcgatggcctccatgcgaccgatgacctgggccatggggccgctggcgttttcttcctcgatgtggaaccggcgcagcgtgtccagcaccatcaggcggcggccctcggcggcgcgcttgaggccgtcgaaccactccggggccatgatgttgggcaggctgccgatcagcggctggatcagcaggccgtcagccacggcttgccgttcctcggcgctgaggtgcgccccaagggcgtgcaggcggtgatgaatggcggtgggcgggtcttcggcgggcaggtagatcaccgggccggtgggcagttcgcccacctccagcagatccggcccgcctgcaatctgtgcggccagttgcagggccagcatggatttaccggcaccaccgggcgacaccagcgccccgaccgtaccggccaccatgttgggcaaaacgtagtccagcggtggcggcgctgctgcgaacgcctccagaatattgataggcttatgggtagccattgattgcctcctttgcaggcagttggtggttaggcgctggcggggtcactacccccgccctgcgccgctctgagttcttccaggcactcgcgcagcgcctcgtattcgtcgtcggtcagccagaacttgcgctgacgcatccctttggccttcatgcgctcggcatatcgcgcttggcgtacagcgtcagggctggccagcaggtcgccggtctgcttgtccttttggtctttcatatcagtcaccgagaaacttgccggggccgaaaggcttgtcttcgcggaacaaggacaaggtgcagccgtcaaggttaaggctggccatatcagcgactgaaaagcggccagcctcggccttgtttgacgtataaccaaagccaccgggcaaccaatagcccttgtcacttttgatcaggtagaccgaccctgaagcgcttttttcgtattccataaaacccccttctgtgcgtgagtactcatagtataacaggcgtgagtaccaacgcaagcactacatgctgaaatctggcccgcccctgtccatgcctcgctggcggggtgccggtgcccgtgccagctcggcccgcgcaagctggacgctgggcagacccatgaccttgctgacggtgcgctcgatgtaatccgcttcgtggccgggcttgcgctctgccagcgctgggctggcctcggccatggccttgccgatttcctcggcactgcggccccggctggccagcttctgcgcggcgataaagtcgcacttgctgaggtcatcaccgaagcgcttgaccagcccggccatctcgctgcggtactcgtccagcgccgtgcgccggtggcggctaagctgccgctcggacagttcgaggctggccagcctgcgggccttctcctgctgccgctgggcctgctcgatctgctggccagcctgctgcaccagcgccgggccagcggtggcggtcttgcccttggattcacgcagcagcacccacggctgataaccggcgcgggtggtgtgcttgtccttgcggttggtgaagcccgccaagcggccatagtggcggctgtcggcgctggccgggtcggcgtcgtactcgctggccagcgtccgggcaatctgcccccgaagttcaccgcctgcggcgtcggccaccttgacccatgcctgatagttcttcgggctggtttccactaccagggcaggctcccggccctcggctttcatgtcatccaggtcaaactcgctgaggtcgtccaccagcaccagaccatgccgctcctgctcggcgggcctgatatacacgtcattgccctgggcattcatccgcttgagccatggcgtgttctggagcacttcggcggctgaccattcccggttcatcatctggccggtggtggcgtccctgacgccgatatcgaagcgctcacagcccatggccttgagctgtcggcctatggcctgcaaagtcctgtcgttcttcatcgggccaccaagcgcagccagatcgagccgtcctcggttgtcagtggcgtcaggtcgagcaagagcaacgatgcgatcagcagcaccaccgtaggcatcatggaagccagcatcacggttagccatagcttccagtgccacccccgcgacgcgctccgggcgctctgcgcggcgctgctcacctcggcggctacctcccgcaactctttggccagctccacccatgccgcccctgtctggcgctgggctttcagccactccgccgcctgcgcctcgctggcctgctgggtctggctcatgacctgccgggcttcgtcggccagtgtcgccatgctctgggccagcggttcgatctgctccgctaactcgttgatgcctctggatttcttcactctgtcgattgcgttcatggtctattgcctcccggtattcctgtaagtcgatgatctgggcgttggcggtgtcgatgttcagggccacgtctgcccggtcggtgcggatgccccggccttccatctccaccacgttcggccccaggtgaacaccgggcaggcgctcgatgccctgcgcctcaagtgttctgtggtcaatgcgggcgtcgtggcctgcccgctctaatgcccggttggcatggtcggcccatgcctcgcgggtctgctcaagccatgccttgggcttgagcgcttcggtcttctgtgccccgcccttctccggggtcttgccgttgtaccgcttgaaccactgagcggcgggccgctcgatgccgtcattgatccgctcggagatcatcaggtggcagtgcgggttctcgccgccaccggcatggatggccagcgtatacggcaggcgctcggcaccggtcaggtgctgggcgaactcggacgccagcgccttctgctggtcgagggtcagctcgaccggcagggcaaattcgacctccttgaacagccgcccattggcgcgttcatacaggtcggcagcatcccagtagtcggcgggccgctcgacgaactccggcatgtgcccggattcggcgtgcaagacttcatccatgtcgcgggcatacttgccttcgcgctggatgaagtcggccttggccctggccgattggccgcccgacctgctgccggttttcgccgtaaggtgataaatcgccatgctgcctcgctgttgcttttgcttttcggctccatgcaatggccctcggagagcgcaccgcccgaagggtggccgttaggccagtttctcgaagagaaaccggtaagtgcgccctcccctacaaagtagggtcgggattgccgccgctgtgcctccatgatagcctacgagacagcacattaacaatggggtgtcaagatggttaaggggagcaacaaggcggcggatcggctggccaagctcgaagaacaacgagcgcgaatcaatgccgaaattcagcgggtgcgggcaagggaacagcagcaagagcgcaagaacgaaacaaggcgcaaggtgctggtgggggccatgattttggccaaggtgaacagcagcgagtggccggaggatcggctcatggcggcaatggatgcgtaccttgaacgcgaccacgaccgcgccttgttcggtctgccgccacgccagaaggatgagccgggctgaatgatcgaccgagacaggccctgcggggctgcacacgcgcccccacccttcgggtagggggaaaggccgctaaagcggctaaaagcgctccagcgtatttctgcggggtttggtgtggggtttagcgggctttgcccgcctttccccctgccgcgcagcggtggggcggtgtgtagcctagcgcagcgaatagaccagctatccggcctctggccgggcatattgggcaagggcagcagcgccccacaagggcgctgataaccgcgcctagtggattattcttagataatcatggatggatttttccaacaccccgccagcccccgcccctgctgggtttgcaggtttgggggcgtgacagttattgcaggggttcgtgacagttattgcaggggggcgtgacagttattgcaggggttcgtgacagttagtacgggagtgacgggcactggctggcaatgtctagcaacggcaggcatttcggctgagggtaaaagaactttccgctaagcgatagactgtatgtaaacacagtattgcaaggacgcggaacatgcctcatgtggcggccctcgcgagaattaattcagataaaaaaaatccttagctttcgctaaggatgatttctagcgatgaccctgctgattggttcgctgaccgtagactggttggcttggtttcatcagccatccgcttgccctcatctgttacgccggcggtagccggccagcctcgcagagcaggattcccgttgagcaccgccaggtgcgaataagggacagtgaagaaggaacacccgctcgcgggtgggcctacttcacctatcctgcccggctgacgccgttggatacaccaaggaaagtctacacgaaccctttggcaaaatcctgtatatcgtgcgacatcgcgcgcgcgcgcgcggatgctagtacgttgtgtctcaaaatctctgatgttacattgcacaagataaaaatatatcatcatgaacaataaaactgtctgcttacataaacagtaatacaaggggtgttatgagccatattcaacgggaaacgtcttgctcgaggccgcgattaaattccaacatggatgctgatttatatgggtataaatgggctcgcgataatgtcgggcaatcaggtgcgacaatctatcgattgtatgggaagcccgatgcgccagagttgtttctgaaacatggcaaaggtagcgttgccaatgatgttacagatgagatggtcagactaaactggctgacggaatttatgcctcttccgaccatcaagcattttatccgtactcctgatgatgcatggttactcaccactgcgatccccgggaaaacagcattccaggtattagaagaatatcctgattcaggtgaaaatattgttgatgcgctggcagtgttcctgcgccggttgcattcgattcctgtttgtaattgtccttttaacagcgatcgcgtatttcgtctcgctcaggcgcaatcacgaatgaataacggtttggttgatgcgagtgattttgatgacgagcgtaatggctggcctgttgaacaagtctggaaagaaatgcataagcttttgccattctcaccggattcagtcgtcactcatggtgatttctcacttgataaccttatttttgacgaggggaaattaataggttgtattgatgttggacgagtcggaatcgcagaccgataccaggatcttgccatcctatggaactgcctcggtgagttttctccttcattacagaaacggctttttcaaaaatatggtattgataatcctgatatgaataaattgcagtttcatttgatgctcgatgagtttttctaatcagaattggttaattggttgtaacactggcagagcattacgctgacttgacgggacggcggctttgttgaataaatcgaacttttgctgagttgaaggatcagatcacgcatcttcccgacaacgcagaccgttccgtggcaaagcaaaagttcaaaatcaccaactggtccacctacaacaaagctctcatcaaccgtggctccctcactttctggctggatgatggggcgattcaggcctggtatgagtcagcaacaccttcttcacgaggcagacctcagcgctattctgaccttgccatcacgactgtgctggtcattaaacgcgtattcaggctgaccctgcgcgctgcgcagggctttattgattccatttttacactgatgaatgttccgttgcgctgcccggattacagatcctctagataatgaattcgatgaaaaattcgttgcttcgggactcattctaggaggataagttatttaagtaaaattaaatgtttttaacatagtgatagttaaaaactattaaattcggttttatcgtgcatacaagcttgtgccctgagcttgcgtccctttattttaagtacattaaacaacaataaatatcttgtccctaatttgtgggaattttatgggataaaagtcattttttatttatcgttttttctatttttgatgacaaaaatatgaaattttccctaaaacttgagatattgagctgtttttgttaggatgtttgcaacttaaaaacccaaaaggttaaattatctattttttgaaagcactgcttgcaggtgaacgaacatttgcaggtaagaaattccaaaataaaatcctgtggaagttttctaggcgcttttcttctttagatcctcaagatgttcatttacatcccacagggtcgagtctaatccaaaggacaagtccggaggaatcaatcgtatggtcaagccataagccatccccctgttcgttagattttgctacttctgctgcatttgcaacggtttatgctgatttaagcatgctaggtcgtgaggtttattatcgcttgattgccatagtctttaagtcaatggagacgtttttcatttcatttccattgctgcgattggttgctaatcctatcagcaactcaacaacaaaggtcactcatcatggagagtcataccgaaacctttaattctcataaaacaaaacccaaacctgatattcagttcagaaaaccgacgctggcggatggtgaagccatctatcgcttgattgagcgatgcccgccgttggatttgaactcgagttatctctatttcctgcaggcatcgcattttgccgatacctgtgtggttgcagaaatggacggtgagctggtgggcttcgtttccgcctattacttgcctgaagagccgcgctcattgtttgtttggcagattgccgtagacgaaatcgcgcgaggccaaggcttagcgaagcgattgattcgtcaattactggcgaaccagagcaaaagctatgtcaccgaaattctctgcaccatcagtccatccaacaaggcctcccaagcgttgttcaacggctttgccaatgacgaaggcttgaaggtagtcgttgaaccctttttaaccgaagcgcacttttccagtcttggacacgaggctgaagaactttatcgcttggcagcaccaaagcatcagaacctgtttgcctactggcgataagaaaaactattaaaaatctaaggaaagctaacatgacaacagaaaaattaagtgtatttaatcaatacgaatcggaagtgagaggctatatccgctctttcccaaccctattttcaaaatcgaaaatggcagaaatctgggacgatgacggtaaacgttacgtcgatttctttgccggcgcgggcgcgttgaactacgggcacaacaatccggttatcaacgatgcggtcatcaagtatttgcaggaagacggtatcggccatgcactggatatggcgacagtagcgaaacgcgactttattgagtcgttcgtcaataacatcctcaagccacgaaatctggattacaaaattcaattcgtaggaccaaccggtaccaatgccatcgaaaccgcattgaaaatcgccagaaaggtcaagggtcgtaaacaagtgatgtctttcactaacggcttccatggtatgtcgatgggatcgctgagtatcaccggtaacagttactaccacgacgaaagctatggtgtgccgggttacaccactcaggtgcctttccataactacctgggcgacaaggtcgataccatcgcttatctacacaaaattctagaagatgcttccagtgggacggaactgcctgccgccatcgttttggaaaccattcaggcggaagggggcatcaacgttgccggcgcgccttggctgaaatcgctgagagagatttgtgacaaattcgatatcttgttgatcgtcgatgacattcaagctggtaacggacgctcaagtgatttcttcagcttcgaacgtgctggtatcgtccctgatattgtcactttatcgaaatctgtcgggggtgggcatccgatgtcgattgttttgatgaaaccagagttggacaaatggagtccgggtgaacactcaggaactttccgtgggtttaacttggcgtttgtcgcggcgaaggcagcgattgacaaatattggtcaaacaaagacttccaagcggaaatcaaacaaaaatctgagtgggtgcaacagcgtatgcagcaactggcgttgaaattcccgaaagcgattcgtgaaattcgcggtcacggcatgatctggggtgcggagttcagagaccctgaagtcgcgtcaaaagtctgtgaggcgtcattccatgaaggcttggtggtggaaaccgccggcgcggaaggtgaagtcatcaaattcctcgggcctttgatcatcaccaaagagttgatcgacgaaggtttcgacattctggaatcagcgaccacaaaagtgctcgccaagaaataacccttttagtaaccaatttagacaggagtaaatcatgattgtaagaaatctatacgacgatattatcggaaccgaagcggatgtagatggtgggcaatgggtcagccgccgcttgttgctggggaaagatgggatgggattctctttccatgacaccatcatcaaagaaggtgagatttgccatttttggtataaaaaccatcttgaagcggtgtattgcattgcgggtgaaggggaaatctacgacaaggcgaccggtatcacgcacccgattcgtgaagggacgatctatgcattgaacgagcatgatcgccatatccttagcgccaacaaaggcactgaactgcgtttggtgtgtgccttcaatccaccggtcacggggcgcgaaacccatgatgaagatggttcttatactttggtgaaggaataagttatcgccatgcagcataagaatgagcagggaaaacctgttgatagaacattgagcgtcgagaaaatcggcggaacctccatgagtgactatcaggcggttagggacaatattgttttctatccgcaaaacccgtatcgacgtattctggtggtgtccgcttacggcggcatgaccaacgacttgttggaacacaagaaaaccgggcaaccgggtgtctatgggttgtttgcatacaatgacgagagtgatgatggtacggagcattcctggcgcgaagctttgcgagacctctcggcaaagatgcaacagttcaacgaagagctgtttgatgaagatgacatgaaagcggcggcaaaccgctttatctccgagcgcattgaacacaccgaaaacttgttgatgcatttgcagaacctttgtcaccatggacatttttcactggaagatcatttgttgacggtgcgtgaactcttagcgagcatcggcgaagcgcacagtgcatggaacctgacgcagttgttgaaatcagaaggcatcaatgcaatttggattgatttgaccggctggcaggacgatgaaaaactgccgctggatgaagtgattcacaacaaattgtgccacctcaattatgacgaagtgctgccgattgtaaccggctatgctcactgcgaagagaacctcatgaacacctttgaccgtggctatagcgaaatgacgttcagtcgtattgcggtgttgtgtcaggcgacgcaagcggtcattcataaggaatatcatttgagtagtgccgacccgcgcttggtgggagaggaacaggcagttcccattggtaagaccaattatgacatcgctgaccagttggcgaaccttggcatggaagcgattcaccccaaagcggcaaaagggttgcgacaagcacagatccctctgttgattaaaaacacctttgagcccgagcaccacggcaccattattcgcgaagactacgtgagcgagttcccgcaagtcgagattatcgccggcaggcagaatttgatcgccgtagaagtgttcgatgccgaaatgatggggcagcagacagactatgagcaagccatttgggaaatcaccaaacgtctcagatgccaggtgctgactaaagatttcaacgccaataccatcaccctgtatctgcaagcatccttgcgaaaagccaaacgacttgccggacaattggaggtgcgtttgccgaccgccaagatttccaccagcaaagtctcattggtttcggcgatgggaagtgatatgcgtatcaaagggcttttggcgcaagctgtacagacgctatttgaagcgggcatcaatattcaagcgttgcatcaaaacctcagacaggtggaaatgcagtttttcgtcaaagagcaagattacgagcgcgcggtcaaacgcctacacgctagtttaatcgaagttcataaccatggaaaagcgatatgggaacactaaagaaggatcctgaagatccaacgctcggttgccgccgggcgttttttattctgcaggagcagaagagcatacatctggaagctttctagaatcgggggcccccggggggattctagaacaatgga

SEQ ID NO: 23 - DNA, 9953 bp, synthetic construct
  source 1..9953: mol_type = other DNA
agtcctcgtctcgccctcgaattagcccgcttaatgagcgggctttttttgaattaattctcgcgagctggcacgacaggtttcccgactggaaagcgggcagtgagcgcaacgcaattaatgtaagttagcgcgaattgcaagctggccgacgcgctgggctacgtcttgctggcgttcgggagcagaagagcatacatctggaagcaaagccaggaaagcggcctatggagctgtgcggcagcgctcagtaggcaatttttcaaaatattgttaagccttttctgagcatggtatttttcatggtattaccaattagcaggaaaataagccattgaatataaaagataaaaatgtcttgtttacaatagagtggggggggtcagcctgccgccttgggccgggtgatgtcgtacttgcccgccgcgaactcggttaccgtccagcccagcgcgaccagctccggcaacgcctcgcgcacccgctggcggcgcttgcgcatggtcgaaccactggcctctgacggccagacatagccgcacaaggtatctatggaagccttgccggttttgccggggtcgatccagccacacagccgctggtgcagcaggcgggcggtttcgctgtccagcgcccgcacctcgtccatgctgatgcgcacatgctggccgccacccatgacggcctgcgcgatcaaggggttcagggccacgtacaggcgcccgtccgcctcgtcgctggcgtactccgacagcagccgaaacccctgccgcttgcggccattctgggcgatgatggataccttccaaaggcgctcgatgcagtcctgtatgtgcttgagcgccccaccactatcgacctctgccccgatttcctttgccagcgcccgatagctacctttgaccaccatggcatcagcggtgacggcctcccacttgggttccaggaacagccggagctgccgtccgccttcggtcttgggttccgggccaagcactaggccattaggcccagccatggccaccagcccttgcaggatgcgcagatcatcagcgcccagcggctccgggccgctgaactcgatccgcttgccgtcgccgtagtcatacgtcacgtccagcttgctgcgcttgcgctcgccccgcttgagggcacggaacaggccgggggccagacagtgcgccgggtcgtgtcggacgtggctgaggctgtgcttgttcttaggcttcaccacggggcacccccttgctcttgcgctgcctctccagcacggcgggcttgagcaccccgccgtcatgccgcctgaaccaccgatcagcgaacggtgcgccatagttggccttgctcacaccgaagcggacgaagaaccggcgctggtcgtcgtccacaccccattcctcggcctcggcgctggtcatgctcgacaggtaggactgccagcggatgttatcgaccagtaccgagctgccccggctggcctgctgctggtcgcctgcgcccatcatggccgcgcccttgctggcatggtgcaggaacacgatagagcacccggtatcggcggcgatggcctccatgcgaccgatgacctgggccatggggccgctggcgttttcttcctcgatgtggaaccggcgcagcgtgtccagcaccatcaggcggcggccctcggcggcgcgcttgaggccgtcgaaccactccggggccatgatgttgggcaggctgccgatcagcggctggatcagcaggccgtcagccacggcttgccgttcctcggcgctgaggtgcgccccaagggcgtgcaggcggtgatgaatggcggtgggcgggtcttcggcgggcaggtagatcaccgggccggtgggcagttcgcccacctccagcagatccggcccgcctgcaatctgtgcggccagttgcagggccagcatggatttaccggcaccaccgggcgacaccagcgccccgaccgtaccggccaccatgttgggcaaaacgtagtccagcggtggcggcgctgctgcgaacgcctccagaatattgataggcttatgggtagccattgattgcctcctttgcaggcagttggtggttaggcgctggcggggtcactacccccgccctgcgccgctctgagttcttccaggcactcgcgcagcgcctcgtattcgtcgtcggtcagccagaacttgcgctgacgcatccctttggccttcatgcgctcggcatatcgcgcttggcgtacagcgtcagggctggccagcaggtcgccggtctgcttgtccttttggtctttcatatcagtcaccgagaaacttgccggggccgaaaggcttgtcttcgcggaacaaggacaaggtgcagccgtcaaggttaaggctggccatatcagcgactgaaaagcggccagcctcggccttgtttgacgtataaccaaagccaccgggcaaccaatagcccttgtcacttttgatcaggtagaccgaccctgaagcgcttttttcgtattccataaaacccccttctgtgcgtgagtactcatagtataacaggcgtgagtaccaacgcaagcactacatgctgaaatctggcccgcccctgtccatgcctcgctggcggggtgccggtgcccgtgccagctcggcccgcgcaagctggacgctgggcagacccatgaccttgctgacggtgcgctcgatgtaatccgcttcgtggccgggcttgcgctctgccagcgctgggctggcctcggccatggccttgccgatttcctcggcactgcggccccggctggccagcttctgcgcggcgataaagtcgcacttgctgaggtcatcaccgaagcgcttgaccagcccggccatctcgctgcggtactcgtccagcgccgtgcgccggtggcggctaagctgccgctcggacagttcgaggctggccagcctgcgggccttctcctgctgccgctgggcctgctcgatctgctggccagcctgctgcaccagcgccgggccagcggtggcggtcttgcccttggattcacgcagcagcacccacggctgataaccggcgcgggtggtgtgcttgtccttgcggttggtgaagcccgccaagcggccatagtggcggctgtcggcgctggccgggtcggcgtcgtactcgctggccagcgtccgggcaatctgcccccgaagttcaccgcctgcggcgtcggccaccttgacccatgcctgatagttcttcgggctggtttccactaccagggcaggctcccggccctcggctttcatgtcatccaggtcaaactcgctgaggtcgtccaccagcaccagaccatgccgctcctgctcggcgggcctgatatacacgtcattgccctgggcattcatccgcttgagccatggcgtgttctggagcacttcggcggctgaccattcccggttcatcatctggccggtggtggcgtccctgacgccgatatcgaagcgctcacagcccatggccttgagctgtcggcctatggcctgcaaagtcctgtcgttcttcatcgggccaccaagcgcagccagatcgagccgtcctcggttgtcagtggcgtcaggtcgagcaagagcaacgatgcgatcagcagcaccaccgtaggcatcatggaagccagcatcacggttagccatagcttccagtgccacccccgcgacgcgctccgggcgctctgcgcggcgctgctcacctcggcggctacctcccgcaactctttggccagctccacccatgccgcccctgtctggcgctgggctttcagccactccgccgcctgcgcctcgctggcctgctgggtctggctcatgacctgccgggcttcgtcggccagtgtcgccatgctctgggccagcggttcgatctgctccgctaactcgttgatgcctctggatttcttcactctgtcgattgcgttcatggtctattgcctcccggtattcctgtaagtcgatgatctgggcgttggcggtgtcgatgttcagggccacgtctgcccggtcggtgcggatgccccggccttccatctccaccacgttcggccccaggtgaacaccgggcaggcgctcgatgccctgcgcctcaagtgttctgtggtcaatgcgggcgtcgtggcctgcccgctctaatgcccggttggcatggtcggcccatgcctcgcgggtctgctcaagccatgccttgggcttgagcgcttcggtcttctgtgccccgcccttctccggggtcttgccgttgtaccgcttgaaccactgagcggcgggccgctcgatgccgtcattgatccgctcggagatcatcaggtggcagtgcgggttctcgccgccaccggcatggatggccagcgtatacggcaggcgctcggcaccggtcaggtgctgggcgaactcggacgccagcgccttctgctggtcgagggtcagctcgaccggcagggcaaattcgacctccttgaacagccgcccattggcgcgttcatacaggtcggcagcatcccagtagtcggcgggccgctcgacgaactccggcatgtgcccggattcggcgtgcaagacttcatccatgtcgcgggcatacttgccttcgcgctggatgaagtcggccttggccctggccgattggccgcccgacctgctgccggttttcgccgtaaggtgataaatcgccatgctgcctcgctgttgcttttgcttttcggctccatgcaatggccctcggagagcgcaccgcccgaagggtggccgttaggccagtttctcgaagagaaaccggtaagtgcgccctcccctacaaagtagggtcgggattgccgccgctgtgcctccatgatagcctacgagacagcacattaacaatggggtgtcaagatggttaaggggagcaacaaggcggcggatcggctggccaagctcgaagaacaacgagcgcgaatcaatgccgaaattcagcgggtgcgggcaagggaacagcagcaagagcgcaagaacgaaacaaggcgcaaggtgctggtgggggccatgattttggccaaggtgaacagcagcgagtggccggaggatcggctcatggcggcaatggatgcgtaccttgaacgcgaccacgaccgcgccttgttcggtctgccgccacgccagaaggatgagccgggctgaatgatcgaccgagacaggccctgcggggctgcacacgcgcccccacccttcgggtagggggaaaggccgctaaagcggctaaaagcgctccagcgtatttctgcggggtttggtgtggggtttagcgggctttgcccgcctttccccctgccgcgcagcggtggggcggtgtgtagcctagcgcagcgaatagaccagctatccggcctctggccgggcatattgggcaagggcagcagcgccccacaagggcgctgataaccgcgcctagtggattattcttagataatcatggatggatttttccaacaccccgccagcccccgcccctgctgggtttgcaggtttgggggcgtgacagttattgcaggggttcgtgacagttattgcaggggggcgtgacagttattgcaggggttcgtgacagttagtacgggagtgacgggcactggctggcaatgtctagcaacggcaggcatttcggctgagggtaaaagaactttccgctaagcgatagactgtatgtaaacacagtattgcaaggacgcggaacatgcctcatgtggcggccctcgcgagaattaattcagataaaaaaaatccttagctttcgctaaggatgatttctagcgatgaccctgctgattggttcgctgaccgtagactggttggcttggtttcatcagccatccgcttgccctcatctgttacgccggcggtagccggccagcctcgcagagcaggattcccgttgagcaccgccaggtgcgaataagggacagtgaagaaggaacacccgctcgcgggtgggcctacttcacctatcctgcccggctgacgccgttggatacaccaaggaaagtctacacgaaccctttggcaaaatcctgtatatcgtgcgacatcgcgcgcgcgcgcgcggatgctagtacgttgtgtctcaaaatctctgatgttacattgcacaagataaaaatatatcatcatgaacaataaaactgtctgcttacataaacagtaatacaaggggtgttatgagccatattcaacgggaaacgtcttgctcgaggccgcgattaaattccaacatggatgctgatttatatgggtataaatgggctcgcgataatgtcgggcaatcaggtgcgacaatctatcgattgtatgggaagcccgatgcgccagagttgtttctgaaacatggcaaaggtagcgttgccaatgatgttacagatgagatggtcagactaaactggctgacggaatttatgcctcttccgaccatcaagcattttatccgtactcctgatgatgcatggttactcaccactgcgatccccgggaaaacagcattccaggtattagaagaatatcctgattcaggtgaaaatattgttgatgcgctggcagtgttcctgcgccggttgcattcgattcctgtttgtaattgtccttttaacagcgatcgcgtatttcgtctcgctcaggcgcaatcacgaatgaataacggtttggttgatgcgagtgattttgatgacgagcgtaatggctggcctgttgaacaagtctggaaagaaatgcataagcttttgccattctcaccggattcagtcgtcactcatggtgatttctcacttgataaccttatttttgacgaggggaaattaataggttgtattgatgttggacgagtcggaatcgcagaccgataccaggatcttgccatcctatggaactgcctcggtgagttttctccttcattacagaaacggctttttcaaaaatatggtattgataatcctgatatgaataaattgcagtttcatttgatgctcgatgagtttttctaatcagaattggttaattggttgtaacactggcagagcattacgctgacttgacgggacggcggctttgttgaataaatcgaacttttgctgagttgaaggatcagatcacgcatcttcccgacaacgcagaccgttccgtggcaaagcaaaagttcaaaatcaccaactggtccacctacaacaaagctctcatcaaccgtggctccctcactttctggctggatgatggggcgattcaggcctggtatgagtcagcaacaccttcttcacgaggcagacctcagcgctattctgaccttgccatcacgactgtgctggtcattaaacgcgtattcaggctgaccctgcgcgctgcgcagggctttattgattccatttttacactgatgaatgttccgttgcgctgcccggattacagatcctctagataatgaattctataggtacctttatggctagctcagtcctaggtacaatgctagcactagagtcacacaggaaaccactagtatggagagtcataccgaaacctttaattctcataaaacaaaacccaaacctgatattcagttcagaaaaccgacgctggcggatggtgaagccatctatcgcttgattgagcgatgcccgccgttggatttgaactcgagttatctctatttcctgcaggcatcgcattttgccgatacctgtgtggttgcagaaatggacggtgagctggtgggcttcgtttccgcctattacttgcctgaagagccgcgctcattgtttgtttggcagattgccgtagacgaaatcgcgcgaggccaaggcttagcgaagcgattgattcgtcaattactggcgaaccagagcaaaagctatgtcaccgaaattctctgcaccatcagtccatccaacaaggcctcccaagcgttgttcaacggctttgccaatgacgaaggcttgaaggtagtcgttgaaccctttttaaccgaagcgcacttttccagtcttggacacgaggctgaagaactttatcgcttggcagcaccaaagcatcagaacctgtttgcctactggcgataagaaaaactattaaaaatctaaggaaagctaacatgacaacagaaaaattaagtgtatttaatcaatacgaatcggaagtgagaggctatatccgctctttcccaaccctattttcaaaatcgaaaatggcagaaatctgggacgatgacggtaaacgttacgtcgatttctttgccggcgcgggcgcgttgaactacgggcacaacaatccggttatcaacgatgcggtcatcaagtatttgcaggaagacggtatcggccatgcactggatatggcgacagtagcgaaacgcgactttattgagtcgttcgtcaataacatcctcaagccacgaaatctggattacaaaattcaattcgtaggaccaaccggtaccaatgccatcgaaaccgcattgaaaatcgccagaaaggtcaagggtcgtaaacaagtgatgtctttcactaacggcttccatggtatgtcgatgggatcgctgagtatcaccggtaacagttactaccacgacgaaagctatggtgtgccgggttacaccactcaggtgcctttccataactacctgggcgacaaggtcgataccatcgcttatctacacaaaattctagaagatgcttccagtgggacggaactgcctgccgccatcgttttggaaaccattcaggcggaagggggcatcaacgttgccggcgcgccttggctgaaatcgctgagagagatttgtgacaaattcgatatcttgttgatcgtcgatgacattcaagctggtaacggacgctcaagtgatttcttcagcttcgaacgtgctggtatcgtccctgatattgtcactttatcgaaatctgtcgggggtgggcatccgatgtcgattgttttgatgaaaccagagttggacaaatggagtccgggtgaacactcaggaactttccgtgggtttaacttggcgtttgtcgcggcgaaggcagcgattgacaaatattggtcaaacaaagacttccaagcggaaatcaaacaaaaatctgagtgggtgcaacagcgtatgcagcaactggcgttgaaattcccgaaagcgattcgtgaaattcgcggtcacggcatgatctggggtgcggagttcagagaccctgaagtcgcgtcaaaagtctgtgaggcgtcattccatgaaggcttggtggtggaaaccgccggcgcggaaggtgaagtcatcaaattcctcgggcctttgatcatcaccaaagagttgatcgacgaaggtttcgacattctggaatcagcgaccacaaaagtgctcgccaagaaataacccttttagtaaccaatttagacaggagtaaatcatgattgtaagaaatctatacgacgatattatcggaaccgaagcggatgtagatggtgggcaatgggtcagccgccgcttgttgctggggaaagatgggatgggattctctttccatgacaccatcatcaaagaaggtgagatttgccatttttggtataaaaaccatcttgaagcggtgtattgcattgcgggtgaaggggaaatctacgacaaggcgaccggtatcacgcacccgattcgtgaagggacgatctatgcattgaacgagcatgatcgccatatccttagcgccaacaaaggcactgaactgcgtttggtgtgtgccttcaatccaccggtcacggggcgcgaaacccatgatgaagatggttcttatactttggtgaaggaataaggatcctgaagatccaacgctcggttgccgccgggcgttttttattctgcaggagcagaagagcatacatctggaagctttctagaatcgggggcccccggggggattctagaacaatgga

SEQ ID NO: 24 - DNA, 14478 bp, synthetic construct
  source 1..14478: mol_type = other DNA
agtcctcgtctcgccctcgaattagcccgcttaatgagcgggctttttttgaattaattctcgcgagctggcacgacaggtttcccgactggaaagcgggcagtgagcgcaacgcaattaatgtaagttagcgcgaattgcaagctggccgacgcgctgggctacgtcttgctggcgttcgggagcagaagagcatacatctggaagcaaagccaggaaagcggcctatggagctgtgcggcagcgctcagtaggcaatttttcaaaatattgttaagccttttctgagcatggtatttttcatggtattaccaattagcaggaaaataagccattgaatataaaagataaaaatgtcttgtttacaatagagtggggggggtcagcctgccgccttgggccgggtgatgtcgtacttgcccgccgcgaactcggttaccgtccagcccagcgcgaccagctccggcaacgcctcgcgcacccgctggcggcgcttgcgcatggtcgaaccactggcctctgacggccagacatagccgcacaaggtatctatggaagccttgccggttttgccggggtcgatccagccacacagccgctggtgcagcaggcgggcggtttcgctgtccagcgcccgcacctcgtccatgctgatgcgcacatgctggccgccacccatgacggcctgcgcgatcaaggggttcagggccacgtacaggcgcccgtccgcctcgtcgctggcgtactccgacagcagccgaaacccctgccgcttgcggccattctgggcgatgatggataccttccaaaggcgctcgatgcagtcctgtatgtgcttgagcgccccaccactatcgacctctgccccgatttcctttgccagcgcccgatagctacctttgaccaccatggcatcagcggtgacggcctcccacttgggttccaggaacagccggagctgccgtccgccttcggtcttgggttccgggccaagcactaggccattaggcccagccatggccaccagcccttgcaggatgcgcagatcatcagcgcccagcggctccgggccgctgaactcgatccgcttgccgtcgccgtagtcatacgtcacgtccagcttgctgcgcttgcgctcgccccgcttgagggcacggaacaggccgggggccagacagtgcgccgggtcgtgtcggacgtggctgaggctgtgcttgttcttaggcttcaccacggggcacccccttgctcttgcgctgcctctccagcacggcgggcttgagcaccccgccgtcatgccgcctgaaccaccgatcagcgaacggtgcgccatagttggccttgctcacaccgaagcggacgaagaaccggcgctggtcgtcgtccacaccccattcctcggcctcggcgctggtcatgctcgacaggtaggactgccagcggatgttatcgaccagtaccgagctgccccggctggcctgctgctggtcgcctgcgcccatcatggccgcgcccttgctggcatggtgcaggaacacgatagagcacccggtatcggcggcgatggcctccatgcgaccgatgacctgggccatggggccgctggcgttttcttcctcgatgtggaaccggcgcagcgtgtccagcaccatcaggcggcggccctcggcggcgcgcttgaggccgtcgaaccactccggggccatgatgttgggcaggctgccgatcagcggctggatcagcaggccgtcagccacggcttgccgttcctcggcgctgaggtgcgccccaagggcgtgcaggcggtgatgaatggcggtgggcgggtcttcggcgggcaggtagatcaccgggccggtgggcagttcgcccacctccagcagatccggcccgcctgcaatctgtgcggccagttgcagggccagcatggatttaccggcaccaccgggcgacaccagcgccccgaccgtaccggccaccatgttgggcaaaacgtagtccagcggtggcggcgctgctgcgaacgcctccagaatattgataggcttatgggtagccattgattgcctcctttgcaggcagttggtggttaggcgctggcggggtcactacccccgccctgcgccgctctgagttcttccaggcactcgcgcagcgcctcgtattcgtcgtcggtcagccagaacttgcgctgacgcatccctttggccttcatgcgctcggcatatcgcgcttggcgtacagcgtcagggctggccagcaggtcgccggtctgcttgtccttttggtctttcatatcagtcaccgagaaacttgccggggccgaaaggcttgtcttcgcggaacaaggacaaggtgcagccgtcaaggttaaggctggccatatcagcgactgaaaagcggccagcctcggccttgtttgacgtataaccaaagccaccgggcaaccaatagcccttgtcacttttgatcaggtagaccgaccctgaagcgcttttttcgtattccataaaacccccttctgtgcgtgagtactcatagtataacaggcgtgagtaccaacgcaagcactacatgctgaaatctggcccgcccctgtccatgcctcgctggcggggtgccggtgcccgtgccagctcggcccgcgcaagctggacgctgggcagacccatgaccttgctgacggtgcgctcgatgtaatccgcttcgtggccgggcttgcgctctgccagcgctgggctggcctcggccatggccttgccgatttcctcggcactgcggccccggctggccagcttctgcgcggcgataaagtcgcacttgctgaggtcatcaccgaagcgcttgaccagcccggccatctcgctgcggtactcgtccagcgccgtgcgccggtggcggctaagctgccgctcggacagttcgaggctggccagcctgcgggccttctcctgctgccgctgggcctgctcgatctgctggccagcctgctgcaccagcgccgggccagcggtggcggtcttgcccttggattcacgcagcagcacccacggctgataaccggcgcgggtggtgtgcttgtccttgcggttggtgaagcccgccaagcggccatagtggcggctgtcggcgctggccgggtcggcgtcgtactcgctggccagcgtccgggcaatctgcccccgaagttcaccgcctgcggcgtcggccaccttgacccatgcctgatagttcttcgggctggtttccactaccagggcaggctcccggccctcggctttcatgtcatccaggtcaaactcgctgaggtcgtccaccagcaccagaccatgccgctcctgctcggcgggcctgatatacacgtcattgccctgggcattcatccgcttgagccatggcgtgttctggagcacttcggcggctgaccattcccggttcatcatctggccggtggtggcgtccctgacgccgatatcgaagcgctcacagcccatggccttgagctgtcggcctatggcctgcaaagtcctgtcgttcttcatcgggccaccaagcgcagccagatcgagccgtcctcggttgtcagtggcgtcaggtcgagcaagagcaacgatgcgatcagcagcaccaccgtaggcatcatggaagccagcatcacggttagccatagcttccagtgccacccccgcgacgcgctccgggcgctctgcgcggcgctgctcacctcggcggctacctcccgcaactctttggccagctccacccatgccgcccctgtctggcgctgggctttcagccactccgccgcctgcgcctcgctggcctgctgggtctggctcatgacctgccgggcttcgtcggccagtgtcgccatgctctgggccagcggttcgatctgctccgctaactcgttgatgcctctggatttcttcactctgtcgattgcgttcatggtctattgcctcccggtattcctgtaagtcgatgatctgggcgttggcggtgtcgatgttcagggccacgtctgcccggtcggtgcggatgccccggccttccatctccaccacgttcggccccaggtgaacaccgggcaggcgctcgatgccctgcgcctcaagtgttctgtggtcaatgcgggcgtcgtggcctgcccgctctaatgcccggttggcatggtcggcccatgcctcgcgggtctgctcaagccatgccttgggcttgagcgcttcggtcttctgtgccccgcccttctccggggtcttgccgttgtaccgcttgaaccactgagcggcgggccgctcgatgccgtcattgatccgctcggagatcatcaggtggcagtgcgggttctcgccgccaccggcatggatggccagcgtatacggcaggcgctcggcaccggtcaggtgctgggcgaactcggacgccagcgccttctgctggtcgagggtcagctcgaccggcagggcaaattcgacctccttgaacagccgcccattggcgcgttcatacaggtcggcagcatcccagtagtcggcgggccgctcgacgaactccggcatgtgcccggattcggcgtgcaagacttcatccatgtcgcgggcatacttgccttcgcgctggatgaagtcggccttggccctggccgattggccgcccgacctgctgccggttttcgccgtaaggtgataaatcgccatgctgcctcgctgttgcttttgcttttcggctccatgcaatggccctcggagagcgcaccgcccgaagggtggccgttaggccagtttctcgaagagaaaccggtaagtgcgccctcccctacaaagtagggtcgggattgccgccgctgtgcctccatgatagcctacgagacagcacattaacaatggggtgtcaagatggttaaggggagcaacaaggcggcggatcggctggccaagctcgaagaacaacgagcgcgaatcaatgccgaaattcagcgggtgcgggcaagggaacagcagcaagagcgcaagaacgaaacaaggcgcaaggtgctggtgggggccatgattttggccaaggtgaacagcagcgagtggccggaggatcggctcatggcggcaatggatgcgtaccttgaacgcgaccacgaccgcgccttgttcggtctgccgccacgccagaaggatgagccgggctgaatgatcgaccgagacaggccctgcggggctgcacacgcgcccccacccttcgggtagggggaaaggccgctaaagcggctaaaagcgctccagcgtatttctgcggggtttggtgtggggtttagcgggctttgcccgcctttccccctgccgcgcagcggtggggcggtgtgtagcctagcgcagcgaatagaccagctatccggcctctggccgggcatattgggcaagggcagcagcgccccacaagggcgctgataaccgcgcctagtggattattcttagataatcatggatggatttttccaacaccccgccagcccccgcccctgctgggtttgcaggtttgggggcgtgacagttattgcaggggttcgtgacagttattgcaggggggcgtgacagttattgcaggggttcgtgacagttagtacgggagtgacgggcactggctggcaatgtctagcaacggcaggcatttcggctgagggtaaaagaactttccgctaagcgatagactgtatgtaaacacagtattgcaaggacgcggaacatgcctcatgtggcggccctcgcgagaattaattcagataaaaaaaatccttagctttcgctaaggatgatttctagcgatgaccctgctgattggttcgctgaccgtagactggttggcttggtttcatcagccatccgcttgccctcatctgttacgccggcggtagccggccagcctcgcagagcaggattcccgttgagcaccgccaggtgcgaataagggacagtgaagaaggaacacccgctcgcgggtgggcctacttcacctatcctgcccggctgacgccgttggatacaccaaggaaagtctacacgaaccctttggcaaaatcctgtatatcgtgcgacatcgcgcgcgcgcgcgcggatgctagtacgttgtgtctcaaaatctctgatgttacattgcacaagataaaaatatatcatcatgaacaataaaactgtctgcttacataaacagtaatacaaggggtgttatgagccatattcaacgggaaacgtcttgctcgaggccgcgattaaattccaacatggatgctgatttatatgggtataaatgggctcgcgataatgtcgggcaatcaggtgcgacaatctatcgattgtatgggaagcccgatgcgccagagttgtttctgaaacatggcaaaggtagcgttgccaatgatgttacagatgagatggtcagactaaactggctgacggaatttatgcctcttccgaccatcaagcattttatccgtactcctgatgatgcatggttactcaccactgcgatccccgggaaaacagcattccaggtattagaagaatatcctgattcaggtgaaaatattgttgatgcgctggcagtgttcctgcgccggttgcattcgattcctgtttgtaattgtccttttaacagcgatcgcgtatttcgtctcgctcaggcgcaatcacgaatgaataacggtttggttgatgcgagtgattttgatgacgagcgtaatggctggcctgttgaacaagtctggaaagaaatgcataagcttttgccattctcaccggattcagtcgtcactcatggtgatttctcacttgataaccttatttttgacgaggggaaattaataggttgtattgatgttggacgagtcggaatcgcagaccgataccaggatcttgccatcctatggaactgcctcggtgagttttctccttcattacagaaacggctttttcaaaaatatggtattgataatcctgatatgaataaattgcagtttcatttgatgctcgatgagtttttctaatcagaattggttaattggttgtaacactggcagagcattacgctgacttgacgggacggcggctttgttgaataaatcgaacttttgctgagttgaaggatcagatcacgcatcttcccgacaacgcagaccgttccgtggcaaagcaaaagttcaaaatcaccaactggtccacctacaacaaagctctcatcaaccgtggctccctcactttctggctggatgatggggcgattcaggcctggtatgagtcagcaacaccttcttcacgaggcagacctcagcgctattctgaccttgccatcacgactgtgctggtcattaaacgcgtattcaggctgaccctgcgcgctgcgcagggctttattgattccatttttacactgatgaatgttccgttgcgctgcccggattacagatcctctagataatgaattcgatgaaaaattcgttgcttcgggactcattctaggaggataagttatttaagtaaaattaaatgtttttaacatagtgatagttaaaaactattaaattcggttttatcgtgcatacaagcttgtgccctgagcttgcgtccctttattttaagtacattaaacaacaataaatatcttgtccctaatttgtgggaattttatgggataaaagtcattttttatttatcgttttttctatttttgatgacaaaaatatgaaattttccctaaaacttgagatattgagctgtttttgttaggatgtttgcaacttaaaaacccaaaaggttaaattatctattttttgaaagcactgcttgcaggtgaacgaacatttgcaggtaagaaattccaaaataaaatcctgtggaagttttctaggcgcttttcttctttagatcctcaagatgttcatttacatcccacagggtcgagtctaatccaaaggacaagtccggaggaatcaatcgtatggtcaagccataagccatccccctgttcgttagattttgctacttctgctgcatttgcaacggtttatgctgatttaagcatgctaggtcgtgaggtttattatcgcttgattgccatagtctttaagtcaatggagacgtttttcatttcatttccattgctgcgattggttgctaatcctatcagcaactcaacaacaaaggtcactcatcatggagagtcataccgaaacctttaattctcataaaacaaaacccaaacctgatattcagttcagaaaaccgacgctggcggatggtgaagccatctatcgcttgattgagcgatgcccgccgttggatttgaactcgagttatctctatttcctgcaggcatcgcattttgccgatacctgtgtggttgcagaaatggacggtgagctggtgggcttcgtttccgcctattacttgcctgaagagccgcgctcattgtttgtttggcagattgccgtagacgaaatcgcgcgaggccaaggcttagcgaagcgattgattcgtcaattactggcgaaccagagcaaaagctatgtcaccgaaattctctgcaccatcagtccatccaacaaggcctcccaagcgttgttcaacggctttgccaatgacgaaggcttgaaggtagtcgttgaaccctttttaaccgaagcgcacttttccagtcttggacacgaggctgaagaactttatcgcttggcagcaccaaagcatcagaacctgtttgcctactggcgataagaaaaactattaaaaatctaaggaaagctaacatgacaacagaaaaattaagtgtatttaatcaatacgaatcggaagtgagaggctatatccgctctttcccaaccctattttcaaaatcgaaaatggcagaaatctgggacgatgacggtaaacgttacgtcgatttctttgccggcgcgggcgcgttgaactacgggcacaacaatccggttatcaacgatgcggtcatcaagtatttgcaggaagacggtatcggccatgcactggatatggcgacagtagcgaaacgcgactttattgagtcgttcgtcaataacatcctcaagccacgaaatctggattacaaaattcaattcgtaggaccaaccggtaccaatgccatcgaaaccgcattgaaaatcgccagaaaggtcaagggtcgtaaacaagtgatgtctttcactaacggcttccatggtatgtcgatgggatcgctgagtatcaccggtaacagttactaccacgacgaaagctatggtgtgccgggttacaccactcaggtgcctttccataactacctgggcgacaaggtcgataccatcgcttatctacacaaaattctagaagatgcttccagtgggacggaactgcctgccgccatcgttttggaaaccattcaggcggaagggggcatcaacgttgccggcgcgccttggctgaaatcgctgagagagatttgtgacaaattcgatatcttgttgatcgtcgatgacattcaagctggtaacggacgctcaagtgatttcttcagcttcgaacgtgctggtatcgtccctgatattgtcactttatcgaaatctgtcgggggtgggcatccgatgtcgattgttttgatgaaaccagagttggacaaatggagtccgggtgaacactcaggaactttccgtgggtttaacttggcgtttgtcgcggcgaaggcagcgattgacaaatattggtcaaacaaagacttccaagcggaaatcaaacaaaaatctgagtgggtgcaacagcgtatgcagcaactggcgttgaaattcccgaaagcgattcgtgaaattcgcggtcacggcatgatctggggtgcggagttcagagaccctgaagtcgcgtcaaaagtctgtgaggcgtcattccatgaaggcttggtggtggaaaccgccggcgcggaaggtgaagtcatcaaattcctcgggcctttgatcatcaccaaagagttgatcgacgaaggtttcgacattctggaatcagcgaccacaaaagtgctcgccaagaaataacccttttagtaaccaatttagacaggagtaaatcatgattgtaagaaatctatacgacgatattatcggaaccgaagcggatgtagatggtgggcaatgggtcagccgccgcttgttgctggggaaagatgggatgggattctctttccatgacaccatcatcaaagaaggtgagatttgccatttttggtataaaaaccatcttgaagcggtgtattgcattgcgggtgaaggggaaatctacgacaaggcgaccggtatcacgcacccgattcgtgaagggacgatctatgcattgaacgagcatgatcgccatatccttagcgccaacaaaggcactgaactgcgtttggtgtgtgccttcaatccaccggtcacggggcgcgaaacccatgatgaagatggttcttatactttggtgaaggaataagttatcgccatgcagcataagaatgagcagggaaaacctgttgatagaacattgagcgtcgagaaaatcggcggaacctccatgagtgactatcaggcggttagggacaatattgttttctatccgcaaaacccgtatcgacgtattctggtggtgtccgcttacggcggcatgaccaacgacttgttggaacacaagaaaaccgggcaaccgggtgtctatgggttgtttgcatacaatgacgagagtgatgatggtacggagcattcctggcgcgaagctttgcgagacctctcggcaaagatgcaacagttcaacgaagagctgtttgatgaagatgacatgaaagcggcggcaaaccgctttatctccgagcgcattgaacacaccgaaaacttgttgatgcatttgcagaacctttgtcaccatggacatttttcactggaagatcatttgttgacggtgcgtgaactcttagcgagcatcggcgaagcgcacagtgcatggaacctgacgcagttgttgaaatcagaaggcatcaatgcaatttggattgatttgaccggctggcaggacgatgaaaaactgccgctggatgaagtgattcacaacaaattgtgccacctcaattatgacgaagtgctgccgattgtaaccggctatgctcactgcgaagagaacctcatgaacacctttgaccgtggctatagcgaaatgacgttcagtcgtattgcggtgttgtgtcaggcgacgcaagcggtcattcataaggaatatcatttgagtagtgccgacccgcgcttggtgggagaggaacaggcagttcccattggtaagaccaattatgacatcgctgaccagttggcgaaccttggcatggaagcgattcaccccaaagcggcaaaagggttgcgacaagcacagatccctctgttgattaaaaacacctttgagcccgagcaccacggcaccattattcgcgaagactacgtgagcgagttcccgcaagtcgagattatcgccggcaggcagaatttgatcgccgtagaagtgttcgatgccgaaatgatggggcagcagacagactatgagcaagccatttgggaaatcaccaaacgtctcagatgccaggtgctgactaaagatttcaacgccaataccatcaccctgtatctgcaagcatccttgcgaaaagccaaacgacttgccggacaattggaggtgcgtttgccgaccgccaagatttccaccagcaaagtctcattggtttcggcgatgggaagtgatatgcgtatcaaagggcttttggcgcaagctgtacagacgctatttgaagcgggcatcaatattcaagcgttgcatcaaaacctcagacaggtggaaatgcagtttttcgtcaaagagcaagattacgagcgcgcggtcaaacgcctacacgctagtttaatcgaagttcataaccatggaaaagcgatatgggaacactaaagaaaatctgccaggttgggggagtgttagctttgttgctgatggctcaaccggtgtttgccgaggatacagccgccaagccagaggcgtctcaagaagccaagatggaacaaaccgtcgataagctcaaggcgcctttatatacgccgttcatcgaacgctatgtcttggacgacctaaagcagttgcgcatcgacatgaatcacttgcaggttaatatgaccaagcaagtgaccgatcgggagctgacagcgaccaatcgggctgtgtcctatgccaccgataccgtcacctatttcttttacctgattgccggaatcagttccgtgctcttactggtgggttggacctctttgaaagatgttaaagagcgtgttcataattttgccgacaccaaagtgaataaagtgatttccgaatatgagcagcggttggcaaaacttgaagaagaattgaatcataaatccgtcggtattcagagcgcccagaaacgtctcacgcgttatgaagatattcatagcctatggttgaaagcggcgcaggagcaggtgccgaccagacgtctggatttgtatgatcagattctacgcttagatcgcgacaatgccgaagcattaacctataaagccgatgtggttctggagatgaacgaaccgcaatgggcaatcaacctctgtcagcaagcattagaaattgatcctgataactcccatgccttttatcaattggcgggagcctatgcgttgttgaatcaacctcatgacgccatcgtcaatttggagttgtctctaaaggacacggaaggcatggttgaccaagtgcttaaagatcctatttttgaaggtctgtcggaaaatgctgagttcaaagaattgctgaaacgaaaaggggtggtttgatgaaatctccacaaggaaaacaccttatcggaaggttcattaaatgatattgacgacttttcttggctttctactgttgtttttcctgataggggtttcaagctattttttctcccgaaaaaccacttcagattatttggtagcggggaaaagcgtttctcccgctttggtagggctatcggctatcgctaccaataatagcggcttcatgttcattgggatgatcggcgcaacctacaccatgggcttgtcgtccatttggttgatgattggctggatttttggggatttcattgctcagaaactggcggtgaaacagattcagcgccacgcgcaggcagatacagtgcattcgtttggcggactcattgtccactggttggtaagggattctgagggaaaaacttcgatgactcaagttttccgacttcgacaattgattggtgttctgacgttggtgtttctggtggtttacgctgctgcccagttaaaagcgggcacgaaagccactcaagtgctgctcggctggtcacctgaaaccggcatctatctcgcggcgatgattattttcgtttatagcctgatgggcggattgcgggcatcgatatggacggatgtcgcccagtcgattgtgatgttgtttggtatggcttccctggcgatattcggcattttgtcgctgatgtcatctgagcaaagtgtgtgggaacaactggcgaatgccgctccccattatatgaactggcttccatcggatatgacatcaacagcagccattttgtttgtcatcggctggattttcggcggtatgggggtgatagggcagccgcaaatcgtcataaggtttatgacgctgcacccggaacgcacgcccggtgagatgcaagcatactactatgcgtggtttgttaccttttacagtttgacggtttttgtcgggttgttaagtcgcctgttgattcctgtgaccgcaggtttcgatgcggaaactgcattgcccacattagcgaccgagttgatgccgaagatatttgccgggttgatactggcagcgttgtttgcagcaaccatgtctactgtcgattcattggtactttcctgttcggcggctttgacacgcgacttgactcggaagccctcgcaaagtctttatttcaccaagtttgcgacctttaccatcctagtggtagcggttttgattgctatttccaacaatcaaaccgtgttcaaaatggtattggatgcctggggactgcttggctctgctttcggaccattgattatctggctttcaatcggtaagcgcgtaacgcagaaccaggcaatattgatgattttgtccggcattgccgcatttgttctgttttcttattttgattggatggccgaggtttacccggttgcatttggtatgttgactgggttgatagtcgcatttttgacgtctgctgttccaagccttcaaaagcaagctagtaactagggatcctgaagatccaacgctcggttgccgccgggcgttttttattctgcaggagcagaagagcatacatctggaagctttctagaatcgggggcccccggggggattctagaacaatgga

SEQ ID NO: 25 - DNA, 8941 bp, synthetic construct
  source 1..8941: mol_type = other DNA
agtcctcgtctcgccctcgaattagcccgcttaatgagcgggctttttttgaattaattctcgcgagctggcacgacaggtttcccgactggaaagcgggcagtgagcgcaacgcaattaatgtaagttagcgcgaattgcaagctggccgacgcgctgggctacgtcttgctggcgttcgggagcagaagagcatacatctggaagcaaagccaggaaagcggcctatggagctgtgcggcagcgctcagtaggcaatttttcaaaatattgttaagccttttctgagcatggtatttttcatggtattaccaattagcaggaaaataagccattgaatataaaagataaaaatgtcttgtttacaatagagtggggggggtcagcctgccgccttgggccgggtgatgtcgtacttgcccgccgcgaactcggttaccgtccagcccagcgcgaccagctccggcaacgcctcgcgcacccgctggcggcgcttgcgcatggtcgaaccactggcctctgacggccagacatagccgcacaaggtatctatggaagccttgccggttttgccggggtcgatccagccacacagccgctggtgcagcaggcgggcggtttcgctgtccagcgcccgcacctcgtccatgctgatgcgcacatgctggccgccacccatgacggcctgcgcgatcaaggggttcagggccacgtacaggcgcccgtccgcctcgtcgctggcgtactccgacagcagccgaaacccctgccgcttgcggccattctgggcgatgatggataccttccaaaggcgctcgatgcagtcctgtatgtgcttgagcgccccaccactatcgacctctgccccgatttcctttgccagcgcccgatagctacctttgaccaccatggcatcagcggtgacggcctcccacttgggttccaggaacagccggagctgccgtccgccttcggtcttgggttccgggccaagcactaggccattaggcccagccatggccaccagcccttgcaggatgcgcagatcatcagcgcccagcggctccgggccgctgaactcgatccgcttgccgtcgccgtagtcatacgtcacgtccagcttgctgcgcttgcgctcgccccgcttgagggcacggaacaggccgggggccagacagtgcgccgggtcgtgtcggacgtggctgaggctgtgcttgttcttaggcttcaccacggggcacccccttgctcttgcgctgcctctccagcacggcgggcttgagcaccccgccgtcatgccgcctgaaccaccgatcagcgaacggtgcgccatagttggccttgctcacaccgaagcggacgaagaaccggcgctggtcgtcgtccacaccccattcctcggcctcggcgctggtcatgctcgacaggtaggactgccagcggatgttatcgaccagtaccgagctgccccggctggcctgctgctggtcgcctgcgcccatcatggccgcgcccttgctggcatggtgcaggaacacgatagagcacccggtatcggcggcgatggcctccatgcgaccgatgacctgggccatggggccgctggcgttttcttcctcgatgtggaaccggcgcagcgtgtccagcaccatcaggcggcggccctcggcggcgcgcttgaggccgtcgaaccactccggggccatgatgttgggcaggctgccgatcagcggctggatcagcaggccgtcagccacggcttgccgttcctcggcgctgaggtgcgccccaagggcgtgcaggcggtgatgaatggcggtgggcgggtcttcggcgggcaggtagatcaccgggccggtgggcagttcgcccacctccagcagatccggcccgcctgcaatctgtgcggccagttgcagggccagcatggatttaccggcaccaccgggcgacaccagcgccccgaccgtaccggccaccatgttgggcaaaacgtagtccagcggtggcggcgctgctgcgaacgcctccagaatattgataggcttatgggtagccattgattgcctcctttgcaggcagttggtggttaggcgctggcggggtcactacccccgccctgcgccgctctgagttcttccaggcactcgcgcagcgcctcgtattcgtcgtcggtcagccagaacttgcgctgacgcatccctttggccttcatgcgctcggcatatcgcgcttggcgtacagcgtcagggctggccagcaggtcgccggtctgcttgtccttttggtctttcatatcagtcaccgagaaacttgccggggccgaaaggcttgtcttcgcggaacaaggacaaggtgcagccgtcaaggttaaggctggccatatcagcgactgaaaagcggccagcctcggccttgtttgacgtataaccaaagccaccgggcaaccaatagcccttgtcacttttgatcaggtagaccgaccctgaagcgcttttttcgtattccataaaacccccttctgtgcgtgagtactcatagtataacaggcgtgagtaccaacgcaagcactacatgctgaaatctggcccgcccctgtccatgcctcgctggcggggtgccggtgcccgtgccagctcggcccgcgcaagctggacgctgggcagacccatgaccttgctgacggtgcgctcgatgtaatccgcttcgtggccgggcttgcgctctgccagcgctgggctggcctcggccatggccttgccgatttcctcggcactgcggccccggctggccagcttctgcgcggcgataaagtcgcacttgctgaggtcatcaccgaagcgcttgaccagcccggccatctcgctgcggtactcgtccagcgccgtgcgccggtggcggctaagctgccgctcggacagttcgaggctggccagcctgcgggccttctcctgctgccgctgggcctgctcgatctgctggccagcctgctgcaccagcgccgggccagcggtggcggtcttgcccttggattcacgcagcagcacccacggctgataaccggcgcgggtggtgtgcttgtccttgcggttggtgaagcccgccaagcggccatagtggcggctgtcggcgctggccgggtcggcgtcgtactcgctggccagcgtccgggcaatctgcccccgaagttcaccgcctgcggcgtcggccaccttgacccatgcctgatagttcttcgggctggtttccactaccagggcaggctcccggccctcggctttcatgtcatccaggtcaaactcgctgaggtcgtccaccagcaccagaccatgccgctcctgctcggcgggcctgatatacacgtcattgccctgggcattcatccgcttgagccatggcgtgttctggagcacttcggcggctgaccattcccggttcatcatctggccggtggtggcgtccctgacgccgatatcgaagcgctcacagcccatggccttgagctgtcggcctatggcctgcaaagtcctgtcgttcttcatcgggccaccaagcgcagccagatcgagccgtcctcggttgtcagtggcgtcaggtcgagcaagagcaacgatgcgatcagcagcaccaccgtaggcatcatggaagccagcatcacggttagccatagcttccagtgccacccccgcgacgcgctccgggcgctctgcgcggcgctgctcacctcggcggctacctcccgcaactctttggccagctccacccatgccgcccctgtctggcgctgggctttcagccactccgccgcctgcgcctcgctggcctgctgggtctggctcatgacctgccgggcttcgtcggccagtgtcgccatgctctgggccagcggttcgatctgctccgctaactcgttgatgcctctggatttcttcactctgtcgattgcgttcatggtctattgcctcccggtattcctgtaagtcgatgatctgggcgttggcggtgtcgatgttcagggccacgtctgcccggtcggtgcggatgccccggccttccatctccaccacgttcggccccaggtgaacaccgggcaggcgctcgatgccctgcgcctcaagtgttctgtggtcaatgcgggcgtcgtggcctgcccgctctaatgcccggttggcatggtcggcccatgcctcgcgggtctgctcaagccatgccttgggcttgagcgcttcggtcttctgtgccccgcccttctccggggtcttgccgttgtaccgcttgaaccactgagcggcgggccgctcgatgccgtcattgatccgctcggagatcatcaggtggcagtgcgggttctcgccgccaccggcatggatggccagcgtatacggcaggcgctcggcaccggtcaggtgctgggcgaactcggacgccagcgccttctgctggtcgagggtcagctcgaccggcagggcaaattcgacctccttgaacagccgcccattggcgcgttcatacaggtcggcagcatcccagtagtcggcgggccgctcgacgaactccggcatgtgcccggattcggcgtgcaagacttcatccatgtcgcgggcatacttgccttcgcgctggatgaagtcggccttggccctggccgattggccgcccgacctgctgccggttttcgccgtaaggtgataaatcgccatgctgcctcgctgttgcttttgcttttcggctccatgcaatggccctcggagagcgcaccgcccgaagggtggccgttaggccagtttctcgaagagaaaccggtaagtgcgccctcccctacaaagtagggtcgggattgccgccgctgtgcctccatgatagcctacgagacagcacattaacaatggggtgtcaagatggttaaggggagcaacaaggcggcggatcggctggccaagctcgaagaacaacgagcgcgaatcaatgccgaaattcagcgggtgcgggcaagggaacagcagcaagagcgcaagaacgaaacaaggcgcaaggtgctggtgggggccatgattttggccaaggtgaacagcagcgagtggccggaggatcggctcatggcggcaatggatgcgtaccttgaacgcgaccacgaccgcgccttgttcggtctgccgccacgccagaaggatgagccgggctgaatgatcgaccgagacaggccctgcggggctgcacacgcgcccccacccttcgggtagggggaaaggccgctaaagcggctaaaagcgctccagcgtatttctgcggggtttggtgtggggtttagcgggctttgcccgcctttccccctgccgcgcagcggtggggcggtgtgtagcctagcgcagcgaatagaccagctatccggcctctggccgggcatattgggcaagggcagcagcgccccacaagggcgctgataaccgcgcctagtggattattcttagataatcatggatggatttttccaacaccccgccagcccccgcccctgctgggtttgcaggtttgggggcgtgacagttattgcaggggttcgtgacagttattgcaggggggcgtgacagttattgcaggggttcgtgacagttagtacgggagtgacgggcactggctggcaatgtctagcaacggcaggcatttcggctgagggtaaaagaactttccgctaagcgatagactgtatgtaaacacagtattgcaaggacgcggaacatgcctcatgtggcggccctcgcgagaattaattcagataaaaaaaatccttagctttcgctaaggatgatttctagcgatgaccctgctgattggttcgctgaccgtagactggttggcttggtttcatcagccatccgcttgccctcatctgttacgccggcggtagccggccagcctcgcagagcaggattcccgttgagcaccgccaggtgcgaataagggacagtgaagaaggaacacccgctcgcgggtgggcctacttcacctatcctgcccggctgacgccgttggatacaccaaggaaagtctacacgaaccctttggcaaaatcctgtatatcgtgcgacatcgcgcgcgcgcgcgcggatgctagtacgttgtgtctcaaaatctctgatgttacattgcacaagataaaaatatatcatcatgaacaataaaactgtctgcttacataaacagtaatacaaggggtgttatgagccatattcaacgggaaacgtcttgctcgaggccgcgattaaattccaacatggatgctgatttatatgggtataaatgggctcgcgataatgtcgggcaatcaggtgcgacaatctatcgattgtatgggaagcccgatgcgccagagttgtttctgaaacatggcaaaggtagcgttgccaatgatgttacagatgagatggtcagactaaactggctgacggaatttatgcctcttccgaccatcaagcattttatccgtactcctgatgatgcatggttactcaccactgcgatccccgggaaaacagcattccaggtattagaagaatatcctgattcaggtgaaaatattgttgatgcgctggcagtgttcctgcgccggttgcattcgattcctgtttgtaattgtccttttaacagcgatcgcgtatttcgtctcgctcaggcgcaatcacgaatgaataacggtttggttgatgcgagtgattttgatgacgagcgtaatggctggcctgttgaacaagtctggaaagaaatgcataagcttttgccattctcaccggattcagtcgtcactcatggtgatttctcacttgataaccttatttttgacgaggggaaattaataggttgtattgatgttggacgagtcggaatcgcagaccgataccaggatcttgccatcctatggaactgcctcggtgagttttctccttcattacagaaacggctttttcaaaaatatggtattgataatcctgatatgaataaattgcagtttcatttgatgctcgatgagtttttctaatcagaattggttaattggttgtaacactggcagagcattacgctgacttgacgggacggcggctttgttgaataaatcgaacttttgctgagttgaaggatcagatcacgcatcttcccgacaacgcagaccgttccgtggcaaagcaaaagttcaaaatcaccaactggtccacctacaacaaagctctcatcaaccgtggctccctcactttctggctggatgatggggcgattcaggcctggtatgagtcagcaacaccttcttcacgaggcagacctcagcgctattctgaccttgccatcacgactgtgctggtcattaaacgcgtattcaggctgaccctgcgcgctgcgcagggctttattgattccatttttacactgatgaatgttccgttgcgctgcccggattacagatcctctagataatgaattctataggtaccttgacggctagctcagtcctaggtatagtgctagcactagagaaagaggggaaatactagtatgaaaacttttgaactgaatgaatccagggttcgcagctactgccgttccttccccgtggtcttcaagcaggcccagggcgccgaactggtcactcaggacggcaagcgctacatcgacttcctcgctggtgccggcacgctcaactacgggcacaaccacccggtgctcaagcaggcgctgctcgagtacatcgagagcgacggcatcacccacggcctggacatgtacaccgaagccaaggagcgtttcctcgaaaccttcaaccggctgatcctcgagccgcgcggcatgggcgactaccgcatgcagttcaccggcccgaccggcaccaacgcggtcgaggcggcgatgaagctggcgcgcaaggtcaccgggcgcaacaacatcatcagtttcaccaacggcttccacggctgcagcattggcgcgctggccgccaccggcaaccagcatcaccgcggcggctccggcatcggcctcaccgatgtcagccgcatgccgtacgccaactatttcggcgacaagaccaacactatcggcatgatggacaagctcttgtccgacccatccagcgggatcgacaagcccgccgcggtgatcgtcgaggtggtgcagggcgaaggcggcctgaacaccgcgtcggccgaatggatgcgcaagctcgagaagctctgccgcaagcacgaaatgctgctgatcgtcgatgacatccaggccggctgcggccgcaccgggactttcttcagcttcgaagagatgggcatccagccggatatcgtaacgctgtccaagtcgctgtccggctacggcctgccgttcgccatggtgttgctgcgccaggagctggaccagtggaagcccggcgaacacaacggcaccttccgcggcaacaaccatgcattcgtcacggcggccgcggcggtcgagcacttctggcagaacgacacgttcgccaacagcgtgaaggccaagggcaagcgcatcgccgacggcatgcagcgcatcatccgtcgccacggcccggattcgctgtttctcaagggccgcgggatgatgatcggcattagctgccccgatggcgagattgccgccgcagtgtgccgccatgccttcgaaaacggcctggtgatcgagaccagcggcgcccacagcgaagtggtcaagtgcctctgcccgctgatcatcagcgatgagcagatcgacaaggcgctttccatcctcgacaaggcctttgccgccgtgatgagcgagcagaccgagaaccaagcttcctgaggatcctgaagatccaacgctcggttgccgccgggcgttttttattctgcaggagcagaagagcatacatctggaagctttctagaatcgggggcccccggggggattctagaacaatgga

SEQ ID NO: 26 - DNA, 8942 bp, synthetic construct
  source 1..8942: mol_type = other DNA
agtcctcgtctcgccctcgaattagcccgcttaatgagcgggctttttttgaattaattctcgcgagctggcacgacaggtttcccgactggaaagcgggcagtgagcgcaacgcaattaatgtaagttagcgcgaattgcaagctggccgacgcgctgggctacgtcttgctggcgttcgggagcagaagagcatacatctggaagcaaagccaggaaagcggcctatggagctgtgcggcagcgctcagtaggcaatttttcaaaatattgttaagccttttctgagcatggtatttttcatggtattaccaattagcaggaaaataagccattgaatataaaagataaaaatgtcttgtttacaatagagtggggggggtcagcctgccgccttgggccgggtgatgtcgtacttgcccgccgcgaactcggttaccgtccagcccagcgcgaccagctccggcaacgcctcgcgcacccgctggcggcgcttgcgcatggtcgaaccactggcctctgacggccagacatagccgcacaaggtatctatggaagccttgccggttttgccggggtcgatccagccacacagccgctggtgcagcaggcgggcggtttcgctgtccagcgcccgcacctcgtccatgctgatgcgcacatgctggccgccacccatgacggcctgcgcgatcaaggggttcagggccacgtacaggcgcccgtccgcctcgtcgctggcgtactccgacagcagccgaaacccctgccgcttgcggccattctgggcgatgatggataccttccaaaggcgctcgatgcagtcctgtatgtgcttgagcgccccaccactatcgacctctgccccgatttcctttgccagcgcccgatagctacctttgaccaccatggcatcagcggtgacggcctcccacttgggttccaggaacagccggagctgccgtccgccttcggtcttgggttccgggccaagcactaggccattaggcccagccatggccaccagcccttgcaggatgcgcagatcatcagcgcccagcggctccgggccgctgaactcgatccgcttgccgtcgccgtagtcatacgtcacgtccagcttgctgcgcttgcgctcgccccgcttgagggcacggaacaggccgggggccagacagtgcgccgggtcgtgtcggacgtggctgaggctgtgcttgttcttaggcttcaccacggggcacccccttgctcttgcgctgcctctccagcacggcgggcttgagcaccccgccgtcatgccgcctgaaccaccgatcagcgaacggtgcgccatagttggccttgctcacaccgaagcggacgaagaaccggcgctggtcgtcgtccacaccccattcctcggcctcggcgctggtcatgctcgacaggtaggactgccagcggatgttatcgaccagtaccgagctgccccggctggcctgctgctggtcgcctgcgcccatcatggccgcgcccttgctggcatggtgcaggaacacgatagagcacccggtatcggcggcgatggcctccatgcgaccgatgacctgggccatggggccgctggcgttttcttcctcgatgtggaaccggcgcagcgtgtccagcaccatcaggcggcggccctcggcggcgcgcttgaggccgtcgaaccactccggggccatgatgttgggcaggctgccgatcagcggctggatcagcaggccgtcagccacggcttgccgttcctcggcgctgaggtgcgccccaagggcgtgcaggcggtgatgaatggcggtgggcgggtcttcggcgggcaggtagatcaccgggccggtgggcagttcgcccacctccagcagatccggcccgcctgcaatctgtgcggccagttgcagggccagcatggatttaccggcaccaccgggcgacaccagcgccccgaccgtaccggccaccatgttgggcaaaacgtagtccagcggtggcggcgctgctgcgaacgcctccagaatattgataggcttatgggtagccattgattgcctcctttgcaggcagttggtggttaggcgctggcggggtcactacccccgccctgcgccgctctgagttcttccaggcactcgcgcagcgcctcgtattcgtcgtcggtcagccagaacttgcgctgacgcatccctttggccttcatgcgctcggcatatcgcgcttggcgtacagcgtcagggctggccagcaggtcgccggtctgcttgtccttttggtctttcatatcagtcaccgagaaacttgccggggccgaaaggcttgtcttcgcggaacaaggacaaggtgcagccgtcaaggttaaggctggccatatcagcgactgaaaagcggccagcctcggccttgtttgacgtataaccaaagccaccgggcaaccaatagcccttgtcacttttgatcaggtagaccgaccctgaagcgcttttttcgtattccataaaacccccttctgtgcgtgagtactcatagtataacaggcgtgagtaccaacgcaagcactacatgctgaaatctggcccgcccctgtccatgcctcgctggcggggtgccggtgcccgtgccagctcggcccgcgcaagctggacgctgggcagacccatgaccttgctgacggtgcgctcgatgtaatccgcttcgtggccgggcttgcgctctgccagcgctgggctggcctcggccatggccttgccgatttcctcggcactgcggccccggctggccagcttctgcgcggcgataaagtcgcacttgctgaggtcatcaccgaagcgcttgaccagcccggccatctcgctgcggtactcgtccagcgccgtgcgccggtggcggctaagctgccgctcggacagttcgaggctggccagcctgcgggccttctcctgctgccgctgggcctgctcgatctgctggccagcctgctgcaccagcgccgggccagcggtggcggtcttgcccttggattcacgcagcagcacccacggctgataaccggcgcgggtggtgtgcttgtccttgcggttggtgaagcccgccaagcggccatagtggcggctgtcggcgctggccgggtcggcgtcgtactcgctggccagcgtccgggcaatctgcccccgaagttcaccgcctgcggcgtcggccaccttgacccatgcctgatagttcttcgggctggtttccactaccagggcaggctcccggccctcggctttcatgtcatccaggtcaaactcgctgaggtcgtccaccagcaccagaccatgccgctcctgctcggcgggcctgatatacacgtcattgccctgggcattcatccgcttgagccatggcgtgttctggagcacttcggcggctgaccattcccggttcatcatctggccggtggtggcgtccctgacgccgatatcgaagcgctcacagcccatggccttgagctgtcggcctatggcctgcaaagtcctgtcgttcttcatcgggccaccaagcgcagccagatcgagccgtcctcggttgtcagtggcgtcaggtcgagcaagagcaacgatgcgatcagcagcaccaccgtaggcatcatggaagccagcatcacggttagccatagcttccagtgccacccccgcgacgcgctccgggcgctctgcgcggcgctgctcacctcggcggctacctcccgcaactctttggccagctccacccatgccgcccctgtctggcgctgggctttcagccactccgccgcctgcgcctcgctggcctgctgggtctggctcatgacctgccgggcttcgtcggccagtgtcgccatgctctgggccagcggttcgatctgctccgctaactcgttgatgcctctggatttcttcactctgtcgattgcgttcatggtctattgcctcccggtattcctgtaagtcgatgatctgggcgttggcggtgtcgatgttcagggccacgtctgcccggtcggtgcggatgccccggccttccatctccaccacgttcggccccaggtgaacaccgggcaggcgctcgatgccctgcgcctcaagtgttctgtggtcaatgcgggcgtcgtggcctgcccgctctaatgcccggttggcatggtcggcccatgcctcgcgggtctgctcaagccatgccttgggcttgagcgcttcggtcttctgtgccccgcccttctccggggtcttgccgttgtaccgcttgaaccactgagcggcgggccgctcgatgccgtcattgatccgctcggagatcatcaggtggcagtgcgggttctcgccgccaccggcatggatggccagcgtatacggcaggcgctcggcaccggtcaggtgctgggcgaactcggacgccagcgccttctgctggtcgagggtcagctcgaccggcagggcaaattcgacctccttgaacagccgcccattggcgcgttcatacaggtcggcagcatcccagtagtcggcgggccgctcgacgaactccggcatgtgcccggattcggcgtgcaagacttcatccatgtcgcgggcatacttgccttcgcgctggatgaagtcggccttggccctggccgattggccgcccgacctgctgccggttttcgccgtaaggtgataaatcgccatgctgcctcgctgttgcttttgcttttcggctccatgcaatggccctcggagagcgcaccgcccgaagggtggccgttaggccagtttctcgaagagaaaccggtaagtgcgccctcccctacaaagtagggtcgggattgccgccgctgtgcctccatgatagcctacgagacagcacattaacaatggggtgtcaagatggttaaggggagcaacaaggcggcggatcggctggccaagctcgaagaacaacgagcgcgaatcaatgccgaaattcagcgggtgcgggcaagggaacagcagcaagagcgcaagaacgaaacaaggcgcaaggtgctggtgggggccatgattttggccaaggtgaacagcagcgagtggccggaggatcggctcatggcggcaatggatgcgtaccttgaacgcgaccacgaccgcgccttgttcggtctgccgccacgccagaaggatgagccgggctgaatgatcgaccgagacaggccctgcggggctgcacacgcgcccccacccttcgggtagggggaaaggccgctaaagcggctaaaagcgctccagcgtatttctgcggggtttggtgtggggtttagcgggctttgcccgcctttccccctgccgcgcagcggtggggcggtgtgtagcctagcgcagcgaatagaccagctatccggcctctggccgggcatattgggcaagggcagcagcgccccacaagggcgctgataaccgcgcctagtggattattcttagataatcatggatggatttttccaacaccccgccagcccccgcccctgctgggtttgcaggtttgggggcgtgacagttattgcaggggttcgtgacagttattgcaggggggcgtgacagttattgcaggggttcgtgacagttagtacgggagtgacgggcactggctggcaatgtctagcaacggcaggcatttcggctgagggtaaaagaactttccgctaagcgatagactgtatgtaaacacagtattgcaaggacgcggaacatgcctcatgtggcggccctcgcgagaattaattcagataaaaaaaatccttagctttcgctaaggatgatttctagcgatgaccctgctgattggttcgctgaccgtagactggttggcttggtttcatcagccatccgcttgccctcatctgttacgccggcggtagccggccagcctcgcagagcaggattcccgttgagcaccgccaggtgcgaataagggacagtgaagaaggaacacccgctcgcgggtgggcctacttcacctatcctgcccggctgacgccgttggatacaccaaggaaagtctacacgaaccctttggcaaaatcctgtatatcgtgcgacatcgcgcgcgcgcgcgcggatgctagtacgttgtgtctcaaaatctctgatgttacattgcacaagataaaaatatatcatcatgaacaataaaactgtctgcttacataaacagtaatacaaggggtgttatgagccatattcaacgggaaacgtcttgctcgaggccgcgattaaattccaacatggatgctgatttatatgggtataaatgggctcgcgataatgtcgggcaatcaggtgcgacaatctatcgattgtatgggaagcccgatgcgccagagttgtttctgaaacatggcaaaggtagcgttgccaatgatgttacagatgagatggtcagactaaactggctgacggaatttatgcctcttccgaccatcaagcattttatccgtactcctgatgatgcatggttactcaccactgcgatccccgggaaaacagcattccaggtattagaagaatatcctgattcaggtgaaaatattgttgatgcgctggcagtgttcctgcgccggttgcattcgattcctgtttgtaattgtccttttaacagcgatcgcgtatttcgtctcgctcaggcgcaatcacgaatgaataacggtttggttgatgcgagtgattttgatgacgagcgtaatggctggcctgttgaacaagtctggaaagaaatgcataagcttttgccattctcaccggattcagtcgtcactcatggtgatttctcacttgataaccttatttttgacgaggggaaattaataggttgtattgatgttggacgagtcggaatcgcagaccgataccaggatcttgccatcctatggaactgcctcggtgagttttctccttcattacagaaacggctttttcaaaaatatggtattgataatcctgatatgaataaattgcagtttcatttgatgctcgatgagtttttctaatcagaattggttaattggttgtaacactggcagagcattacgctgacttgacgggacggcggctttgttgaataaatcgaacttttgctgagttgaaggatcagatcacgcatcttcccgacaacgcagaccgttccgtggcaaagcaaaagttcaaaatcaccaactggtccacctacaacaaagctctcatcaaccgtggctccctcactttctggctggatgatggggcgattcaggcctggtatgagtcagcaacaccttcttcacgaggcagacctcagcgctattctgaccttgccatcacgactgtgctggtcattaaacgcgtattcaggctgaccctgcgcgctgcgcagggctttattgattccatttttacactgatgaatgttccgttgcgctgcccggattacagatcctctagataatgaattctataggtacctttatggctagctcagtcctaggtacaatgctagcactagagtcacacaggaaaccactagtatgaaaacttttgaactgaatgaatccagggttcgcagctactgccgttccttccccgtggtcttcaagcaggcccagggcgccgaactggtcactcaggacggcaagcgctacatcgacttcctcgctggtgccggcacgctcaactacgggcacaaccacccggtgctcaagcaggcgctgctcgagtacatcgagagcgacggcatcacccacggcctggacatgtacaccgaagccaaggagcgtttcctcgaaaccttcaaccggctgatcctcgagccgcgcggcatgggcgactaccgcatgcagttcaccggcccgaccggcaccaacgcggtcgaggcggcgatgaagctggcgcgcaaggtcaccgggcgcaacaacatcatcagtttcaccaacggcttccacggctgcagcattggcgcgctggccgccaccggcaaccagcatcaccgcggcggctccggcatcggcctcaccgatgtcagccgcatgccgtacgccaactatttcggcgacaagaccaacactatcggcatgatggacaagctcttgtccgacccatccagcgggatcgacaagcccgccgcggtgatcgtcgaggtggtgcagggcgaaggcggcctgaacaccgcgtcggccgaatggatgcgcaagctcgagaagctctgccgcaagcacgaaatgctgctgatcgtcgatgacatccaggccggctgcggccgcaccgggactttcttcagcttcgaagagatgggcatccagccggatatcgtaacgctgtccaagtcgctgtccggctacggcctgccgttcgccatggtgttgctgcgccaggagctggaccagtggaagcccggcgaacacaacggcaccttccgcggcaacaaccatgcattcgtcacggcggccgcggcggtcgagcacttctggcagaacgacacgttcgccaacagcgtgaaggccaagggcaagcgcatcgccgacggcatgcagcgcatcatccgtcgccacggcccggattcgctgtttctcaagggccgcgggatgatgatcggcattagctgccccgatggcgagattgccgccgcagtgtgccgccatgccttcgaaaacggcctggtgatcgagaccagcggcgcccacagcgaagtggtcaagtgcctctgcccgctgatcatcagcgatgagcagatcgacaaggcgctttccatcctcgacaaggcctttgccgccgtgatgagcgagcagaccgagaaccaagcttcctgaggatcctgaagatccaacgctcggttgccgccgggcgttttttattctgcaggagcagaagagcatacatctggaagctttctagaatcgggggcccccggggggattctagaacaatgga

SEQ ID NO: 27 - DNA, 727 bp, Hydrogenovibrio marinus
  source 1..727: mol_type = genomic DNA
gatgaaaaattcgttgcttcgggactcattctaggaggataagttatttaagtaaaattaaatgtttttaacatagtgatagttaaaaactattaaattcggttttatcgtgcatacaagcttgtgccctgagcttgcgtccctttattttaagtacattaaacaacaataaatatcttgtccctaatttgtgggaattttatgggataaaagtcattttttatttatcgttttttctatttttgatgacaaaaatatgaaattttccctaaaacttgagatattgagctgtttttgttaggatgtttgcaacttaaaaacccaaaaggttaaattatctattttttgaaagcactgcttgcaggtgaacgaacatttgcaggtaagaaattccaaaataaaatcctgtggaagttttctaggcgcttttcttctttagatcctcaagatgttcatttacatcccacagggtcgagtctaatccaaaggacaagtccggaggaatcaatcgtatggtcaagccataagccatccccctgttcgttagattttgctacttctgctgcatttgcaacggtttatgctgatttaagcatgctaggtcgtgaggtttattatcgcttgattgccatagtctttaagtcaatggagacgtttttcatttcatttccattgctgcgattggttgctaatcctatcagcaactcaacaacaaaggtcactcatc

SEQ ID NO: 28 - DNA, 6159 bp, Hydrogenovibrio marinus
  source 1..6159: mol_type = genomic DNA
atggagagtcataccgaaacctttaattctcataaaacaaaacccaaacctgatattcagttcagaaaaccgacgctggcggatggtgaagccatctatcgcttgattgagcgatgcccgccgttggatttgaactcgagttatctctatttcctgcaggcatcgcattttgccgatacctgtgtggttgcagaaatggacggtgagctggtgggcttcgtttccgcctattacttgcctgaagagccgcgctcattgtttgtttggcagattgccgtagacgaaatcgcgcgaggccaaggcttagcgaagcgattgattcgtcaattactggcgaaccagagcaaaagctatgtcaccgaaattctctgcaccatcagtccatccaacaaggcctcccaagcgttgttcaacggctttgccaatgacgaaggcttgaaggtagtcgttgaaccctttttaaccgaagcgcacttttccagtcttggacacgaggctgaagaactttatcgcttggcagcaccaaagcatcagaacctgtttgcctactggcgataagaaaaactattaaaaatctaaggaaagctaacatgacaacagaaaaattaagtgtatttaatcaatacgaatcggaagtgagaggctatatccgctctttcccaaccctattttcaaaatcgaaaatggcagaaatctgggacgatgacggtaaacgttacgtcgatttctttgccggcgcgggcgcgttgaactacgggcacaacaatccggttatcaacgatgcggtcatcaagtatttgcaggaagacggtatcggccatgcactggatatggcgacagtagcgaaacgcgactttattgagtcgttcgtcaataacatcctcaagccacgaaatctggattacaaaattcaattcgtaggaccaaccggtaccaatgccatcgaaaccgcattgaaaatcgccagaaaggtcaagggtcgtaaacaagtgatgtctttcactaacggcttccatggtatgtcgatgggatcgctgagtatcaccggtaacagttactaccacgacgaaagctatggtgtgccgggttacaccactcaggtgcctttccataactacctgggcgacaaggtcgataccatcgcttatctacacaaaattctagaagatgcttccagtgggacggaactgcctgccgccatcgttttggaaaccattcaggcggaagggggcatcaacgttgccggcgcgccttggctgaaatcgctgagagagatttgtgacaaattcgatatcttgttgatcgtcgatgacattcaagctggtaacggacgctcaagtgatttcttcagcttcgaacgtgctggtatcgtccctgatattgtcactttatcgaaatctgtcgggggtgggcatccgatgtcgattgttttgatgaaaccagagttggacaaatggagtccgggtgaacactcaggaactttccgtgggtttaacttggcgtttgtcgcggcgaaggcagcgattgacaaatattggtcaaacaaagacttccaagcggaaatcaaacaaaaatctgagtgggtgcaacagcgtatgcagcaactggcgttgaaattcccgaaagcgattcgtgaaattcgcggtcacggcatgatctggggtgcggagttcagagaccctgaagtcgcgtcaaaagtctgtgaggcgtcattccatgaaggcttggtggtggaaaccgccggcgcggaaggtgaagtcatcaaattcctcgggcctttgatcatcaccaaagagttgatcgacgaaggtttcgacattctggaatcagcgaccacaaaagtgctcgccaagaaataacccttttagtaaccaatttagacaggagtaaatcatgattgtaagaaatctatacgacgatattatcggaaccgaagcggatgtagatggtgggcaatgggtcagccgccgcttgttgctggggaaagatgggatgggattctctttccatgacaccatcatcaaagaaggtgagatttgccatttttggtataaaaaccatcttgaagcggtgtattgcattgcgggtgaaggggaaatctacgacaaggcgaccggtatcacgcacccgattcgtgaagggacgatctatgcattgaacgagcatgatcgccatatccttagcgccaacaaaggcactgaactgcgtttggtgtgtgccttcaatccaccggtcacggggcgcgaaacccatgatgaagatggttcttatactttggtgaaggaataagttatcgccatgcagcataagaatgagcagggaaaacctgttgatagaacattgagcgtcgagaaaatcggcggaacctccatgagtgactatcaggcggttagggacaatattgttttctatccgcaaaacccgtatcgacgtattctggtggtgtccgcttacggcggcatgaccaacgacttgttggaacacaagaaaaccgggcaaccgggtgtctatgggttgtttgcatacaatgacgagagtgatgatggtacggagcattcctggcgcgaagctttgcgagacctctcggcaaagatgcaacagttcaacgaagagctgtttgatgaagatgacatgaaagcggcggcaaaccgctttatctccgagcgcattgaacacaccgaaaacttgttgatgcatttgcagaacctttgtcaccatggacatttttcactggaagatcatttgttgacggtgcgtgaactcttagcgagcatcggcgaagcgcacagtgcatggaacctgacgcagttgttgaaatcagaaggcatcaatgcaatttggattgatttgaccggctggcaggacgatgaaaaactgccgctggatgaagtgattcacaacaaattgtgccacctcaattatgacgaagtgctgccgattgtaaccggctatgctcactgcgaagagaacctcatgaacacctttgaccgtggctatagcgaaatgacgttcagtcgtattgcggtgttgtgtcaggcgacgcaagcggtcattcataaggaatatcatttgagtagtgccgacccgcgcttggtgggagaggaacaggcagttcccattggtaagaccaattatgacatcgctgaccagttggcgaaccttggcatggaagcgattcaccccaaagcggcaaaagggttgcgacaagcacagatccctctgttgattaaaaacacctttgagcccgagcaccacggcaccattattcgcgaagactacgtgagcgagttcccgcaagtcgagattatcgccggcaggcagaatttgatcgccgtagaagtgttcgatgccgaaatgatggggcagcagacagactatgagcaagccatttgggaaatcaccaaacgtctcagatgccaggtgctgactaaagatttcaacgccaataccatcaccctgtatctgcaagcatccttgcgaaaagccaaacgacttgccggacaattggaggtgcgtttgccgaccgccaagatttccaccagcaaagtctcattggtttcggcgatgggaagtgatatgcgtatcaaagggcttttggcgcaagctgtacagacgctatttgaagcgggcatcaatattcaagcgttgcatcaaaacctcagacaggtggaaatgcagtttttcgtcaaagagcaagattacgagcgcgcggtcaaacgcctacacgctagtttaatcgaagttcataaccatggaaaagcgatatgggaacactaaagaaaatctgccaggttgggggagtgttagctttgttgctgatggctcaaccggtgtttgccgaggatacagccgccaagccagaggcgtctcaagaagccaagatggaacaaaccgtcgataagctcaaggcgcctttatatacgccgttcatcgaacgctatgtcttggacgacctaaagcagttgcgcatcgacatgaatcacttgcaggttaatatgaccaagcaagtgaccgatcgggagctgacagcgaccaatcgggctgtgtcctatgccaccgataccgtcacctatttcttttacctgattgccggaatcagttccgtgctcttactggtgggttggacctctttgaaagatgttaaagagcgtgttcataattttgccgacaccaaagtgaataaagtgatttccgaatatgagcagcggttggcaaaacttgaagaagaattgaatcataaatccgtcggtattcagagcgcccagaaacgtctcacgcgttatgaagatattcatagcctatggttgaaagcggcgcaggagcaggtgccgaccagacgtctggatttgtatgatcagattctacgcttagatcgcgacaatgccgaagcattaacctataaagccgatgtggttctggagatgaacgaaccgcaatgggcaatcaacctctgtcagcaagcattagaaattgatcctgataactcccatgccttttatcaattggcgggagcctatgcgttgttgaatcaacctcatgacgccatcgtcaatttggagttgtctctaaaggacacggaaggcatggttgaccaagtgcttaaagatcctatttttgaaggtctgtcggaaaatgctgagttcaaagaattgctgaaacgaaaaggggtggtttgatgaaatctccacaaggaaaacaccttatcggaaggttcattaaatgatattgacgacttttcttggctttctactgttgtttttcctgataggggtttcaagctattttttctcccgaaaaaccacttcagattatttggtagcggggaaaagcgtttctcccgctttggtagggctatcggctatcgctaccaataatagcggcttcatgttcattgggatgatcggcgcaacctacaccatgggcttgtcgtccatttggttgatgattggctggatttttggggatttcattgctcagaaactggcggtgaaacagattcagcgccacgcgcaggcagatacagtgcattcgtttggcggactcattgtccactggttggtaagggattctgagggaaaaacttcgatgactcaagttttccgacttcgacaattgattggtgttctgacgttggtgtttctggtggtttacgctgctgcccagttaaaagcgggcacgaaagccactcaagtgctgctcggctggtcacctgaaaccggcatctatctcgcggcgatgattattttcgtttatagcctgatgggcggattgcgggcatcgatatggacggatgtcgcccagtcgattgtgatgttgtttggtatggcttccctggcgatattcggcattttgtcgctgatgtcatctgagcaaagtgtgtgggaacaactggcgaatgccgctccccattatatgaactggcttccatcggatatgacatcaacagcagccattttgtttgtcatcggctggattttcggcggtatgggggtgatagggcagccgcaaatcgtcataaggtttatgacgctgcacccggaacgcacgcccggtgagatgcaagcatactactatgcgtggtttgttaccttttacagtttgacggtttttgtcgggttgttaagtcgcctgttgattcctgtgaccgcaggtttcgatgcggaaactgcattgcccacattagcgaccgagttgatgccgaagatatttgccgggttgatactggcagcgttgtttgcagcaaccatgtctactgtcgattcattggtactttcctgttcggcggctttgacacgcgacttgactcggaagccctcgcaaagtctttatttcaccaagtttgcgacctttaccatcctagtggtagcggttttgattgctatttccaacaatcaaaccgtgttcaaaatggtattggatgcctggggactgcttggctctgctttcggaccattgattatctggctttcaatcggtaagcgcgtaacgcagaaccaggcaatattgatgattttgtccggcattgccgcatttgttctgttttcttattttgattggatggccgaggtttacccggttgcatttggtatgttgactgggttgatagtcgcatttttgacgtctgctgttccaagccttcaaaagcaagctagtaactag

SEQ ID NO: 29 - DNA, 558 bp, Hydrogenovibrio marinus
  source 1..558: mol_type = genomic DNA
atggagagtcataccgaaacctttaattctcataaaacaaaacccaaacctgatattcagttcagaaaaccgacgctggcggatggtgaagccatctatcgcttgattgagcgatgcccgccgttggatttgaactcgagttatctctatttcctgcaggcatcgcattttgccgatacctgtgtggttgcagaaatggacggtgagctggtgggcttcgtttccgcctattacttgcctgaagagccgcgctcattgtttgtttggcagattgccgtagacgaaatcgcgcgaggccaaggcttagcgaagcgattgattcgtcaattactggcgaaccagagcaaaagctatgtcaccgaaattctctgcaccatcagtccatccaacaaggcctcccaagcgttgttcaacggctttgccaatgacgaaggcttgaaggtagtcgttgaaccctttttaaccgaagcgcacttttccagtcttggacacgaggctgaagaactttatcgcttggcagcaccaaagcatcagaacctgtttgcctactggcgataa

SEQ ID NO: 30 - DNA, 1269 bp, Hydrogenovibrio marinus
  source 1..1269: mol_type = genomic DNA
atgacaacagaaaaattaagtgtatttaatcaatacgaatcggaagtgagaggctatatccgctctttcccaaccctattttcaaaatcgaaaatggcagaaatctgggacgatgacggtaaacgttacgtcgatttctttgccggcgcgggcgcgttgaactacgggcacaacaatccggttatcaacgatgcggtcatcaagtatttgcaggaagacggtatcggccatgcactggatatggcgacagtagcgaaacgcgactttattgagtcgttcgtcaataacatcctcaagccacgaaatctggattacaaaattcaattcgtaggaccaaccggtaccaatgccatcgaaaccgcattgaaaatcgccagaaaggtcaagggtcgtaaacaagtgatgtctttcactaacggcttccatggtatgtcgatgggatcgctgagtatcaccggtaacagttactaccacgacgaaagctatggtgtgccgggttacaccactcaggtgcctttccataactacctgggcgacaaggtcgataccatcgcttatctacacaaaattctagaagatgcttccagtgggacggaactgcctgccgccatcgttttggaaaccattcaggcggaagggggcatcaacgttgccggcgcgccttggctgaaatcgctgagagagatttgtgacaaattcgatatcttgttgatcgtcgatgacattcaagctggtaacggacgctcaagtgatttcttcagcttcgaacgtgctggtatcgtccctgatattgtcactttatcgaaatctgtcgggggtgggcatccgatgtcgattgttttgatgaaaccagagttggacaaatggagtccgggtgaacactcaggaactttccgtgggtttaacttggcgtttgtcgcggcgaaggcagcgattgacaaatattggtcaaacaaagacttccaagcggaaatcaaacaaaaatctgagtgggtgcaacagcgtatgcagcaactggcgttgaaattcccgaaagcgattcgtgaaattcgcggtcacggcatgatctggggtgcggagttcagagaccctgaagtcgcgtcaaaagtctgtgaggcgtcattccatgaaggcttggtggtggaaaccgccggcgcggaaggtgaagtcatcaaattcctcgggcctttgatcatcaccaaagagttgatcgacgaaggtttcgacattctggaatcagcgaccacaaaagtgctcgccaagaaataa

SEQ ID NO: 31 - DNA, 396 bp, Hydrogenovibrio marinus
  source 1..396: mol_type = genomic DNA
atgattgtaagaaatctatacgacgatattatcggaaccgaagcggatgtagatggtgggcaatgggtcagccgccgcttgttgctggggaaagatgggatgggattctctttccatgacaccatcatcaaagaaggtgagatttgccatttttggtataaaaaccatcttgaagcggtgtattgcattgcgggtgaaggggaaatctacgacaaggcgaccggtatcacgcacccgattcgtgaagggacgatctatgcattgaacgagcatgatcgccatatccttagcgccaacaaaggcactgaactgcgtttggtgtgtgccttcaatccaccggtcacggggcgcgaaacccatgatgaagatggttcttatactttggtgaaggaataa

SEQ ID NO: 32 - DNA, 6650 bp, Pseudomonas stutzeri
  source 1..6650: mol_type = genomic DNA
atgctccgtcgcccaaccgacggcgacggttacaaccttcatcagctggtggcgcgctgccagcccctcgataccaattcggtctactgcaacctgctgcagtgttccgatttcgctgacaccgccatcgccgcagagaacgcccaaggcgagctggtcggtttcatctcgggttaccgccccccttcgcggccggacacgctgttcgtctggcaggtcgccgtcgacagctcgatgcgcggtcaggggctggccctgcgcatgctgctggcactgaccgcccgggtcgctcgcgagtacggcgtgcgttacatggaaaccaccatctcgccggacaacggggcgtcacaggcgctgttcaagcgggccttcgaccgcctcgatgccaactgcacgacgcgcacgctgttcgcccgcgacacgcatttcgccggtcagcacgaggacgaggtgctctaccgcgccggcccgttcaccgtttcccatctagaagaagagctcaaggagcacgcatgaaaacttttgaactgaatgaatccagggttcgcagctactgccgttccttccccgtggtcttcaagcaggcccagggcgccgaactggtcactcaggacggcaagcgctacatcgacttcctcgctggtgccggcacgctcaactacgggcacaaccacccggtgctcaagcaggcgctgctcgagtacatcgagagcgacggcatcacccacggcctggacatgtacaccgaagccaaggagcgtttcctcgaaaccttcaaccggctgatcctcgagccgcgcggcatgggcgactaccgcatgcagttcaccggcccgaccggcaccaacgcggtcgaggcggcgatgaagctggcgcgcaaggtcaccgggcgcaacaacatcatcagtttcaccaacggcttccacggctgcagcattggcgcgctggccgccaccggcaaccagcatcaccgcggcggctccggcatcggcctcaccgatgtcagccgcatgccgtacgccaactatttcggcgacaagaccaacactatcggcatgatggacaagctcttgtccgacccatccagcgggatcgacaagcccgccgcggtgatcgtcgaggtggtgcagggcgaaggcggcctgaacaccgcgtcggccgaatggatgcgcaagctcgagaagctctgccgcaagcacgaaatgctgctgatcgtcgatgacatccaggccggctgcggccgcaccgggactttcttcagcttcgaagagatgggcatccagccggatatcgtaacgctgtccaagtcgctgtccggctacggcctgccgttcgccatggtgttgctgcgccaggagctggaccagtggaagcccggcgaacacaacggcaccttccgcggcaacaaccatgcattcgtcacggcggccgcggcggtcgagcacttctggcagaacgacacgttcgccaacagcgtgaaggccaagggcaagcgcatcgccgacggcatgcagcgcatcatccgtcgccacggcccggattcgctgtttctcaagggccgcgggatgatgatcggcattagctgccccgatggcgagattgccgccgcagtgtgccgccatgccttcgaaaacggcctggtgatcgagaccagcggcgcccacagcgaagtggtcaagtgcctctgcccgctgatcatcagcgatgagcagatcgacaaggcgctttccatcctcgacaaggcctttgccgccgtgatgagcgagcagaccgagaaccaagcttcctgaggtatccgcaatgatcgtcagaaccctcgccgagtgcgaaaagaccgaccgcaaggtccacagccagaccggcacttgggacagcacgcgcatgctgctcaaggacgacaaggtgggattctccttccacatcaccaccatctacgccggcagcgagacgcacatccactaccagaaccacttcgagtcggtgtactgcatcagcggcaatggcgagatcgaaaccatcgccgacggcaagatttacaagatcgagccgggcacgctgtacgtgctggacaagcatgacgagcacctgctgcgcggtggcagcgaagacatgaagctggcctgcgtcttcaacccgccgctcaacgggcgcgaagtgcatgacgaaagcggcgtctatccgctggaggccgaaaccgtctgataccggttcaaccggggcggccaccgcgccgccccgccattacaagaaaggaggtaagcgtgaaccctatgcaagccgacctgtatccctcgcgccaggaagaccagcccagctggcaggaacgcctggatccggtcgtctaccgcagcgacctggagaatgcgccaatcgcggcagagctggtcgaacgcttcgagcgcgacggctacctggtcatccccaatctgttcagcgccgacgaagtcgcgctgtttcgcgccgaactcgagcgcatgcgccaggacccggccgtcgccggttccggcaagaccatcaaggaacccgacagcggtgcgatccgctcggtgttcgccatccacaaggacaacgagctgttcgcccgcgtcgcagccgacgagcgcaccgccggcatcgcccgcttcatccttggcggcgacctgtacgtgcatcagtcgcgaatgaacttcaagcccggcttcaccggcaaggagttctactggcactcggatttcgagacctggcacatcgaggacggcatgccgcgcatgcgctgcctgtcctgctcgatcctcttgaccgacaacgagccgcacaacggcccgctgatgctgatgcccggctcgcacaagcactacgtgcgctgtgtcggagccacaccggaaaatcactacgagaagtccctgcgcaagcaggagatcggcatccccgaccagaacagcctgagcgagctggccagccgcttcggcatcgactgcgccaccggccccgccggcagcgtggtgctcttcgactgcaacaccatgcacggctccaacggcaacatcacgcccagcgcgcggagcaatctgttctacgtctacaaccacgtggataatgccgtgcaggctccgttctgcgagcagaaaccgcgcccggcctttgtcgccgaacgcgagaatttcaagccgctggacattcggccgcaacagtatctctgaggcgatggggcgcgtctgatgacgggccccttcccccggcttggccgatcgctaccggcccagggaaattcactccagctcgttgatcgacaggtgcgccagccgcgcgccgggcccgtcaacggcctgccagattcggacgctataaaaagatgcataccgtggaaaagatcggcggcacgtcgatgagccgcttcgaggaagttctcgacaatatcttcatcggccgccgggaaggcgcagcgctttaccagcgtatcttcgtcgtctcggcctacagcggcatgaccaacctgctgctggagcacaagaagaccggcgagcccggcgtctaccaacgcttcgccgatgcgcagagcgaaggtgcctggcgcgaagcgctggagggtgtgcgccagcgcatgctcgccaagaacgccgagctgttcagttccgagtacgaactgcacgccgccaaccagttcatcaactcgcgcatcgacgatgccagcgagtgcatgcacagcctgcagaagctgtgcgcctacggccacttccagctctccgaacacctgatgaaggtgcgcgagatgctcgcttccctcggcgaagcccacagcgccttcaactcggtgctggcgctcaagcagcgcggcgtcaacgcgcgcctggccgacctcaccggctggcagcaggaagcaccgctgccgttcgaggagatgatttccagccacttcgccggcttcgacttcagccgcgaactggtggtcgccaccggttacacccattgcgccgaaggcctgatgaacaccttcgatcgcggctacagcgagatcaccttcgcccagatcgccgccgccaccggcgcacgcgaggccatcatccacaaggaatttcacctctcctcggccgacccgaatctggtgggtgccgacaaagtggtcaccatcggccgcaccaactacgacgtcgccgaccagctgtcgaacctcggcatggaggcgatccacccgcgcgccgccaagaccctgcgtcgcgccggcgtcgaactgcgcatcaagaatgccttcgagcccgagcatggcggcacgctgatcagccaggactacaagtccgagaagccctgcgtcgagatcatcgccgggcgcaaggacgtcttcggcatcgaggtgttcgaccaggacatgctcggcgacatcggctacgacatggagatcagcaagctgctcaagcagctcaagctctatgtggtgaacaaggattccgacgccaacagcatcacctactacgcctccggttcgcgcaagctgatcaatcgcgccgcgcggctgatcgaggagcagtacccggccgccgaggtcaccgtgcacaacctggccatcgtttcggccatcggctccgacctcaaggtcaagggcattctggccaagaccgtggccgctctggccgaggccggcatcagcatccaggcgatccaccagtcaatccgtcaggtggagatgcagtgcgtggtcaacgaggaagactacgacgccgccatcgccgcgctgcaccgcgcactgatcgagccggaaaaccacggcgatgtgatcgcagcggcctgatcgacgcttcattggaaaacgccgggctcgtcccggcgttttgctgtctggacgctgacgccgatcaatactgccggcaacgcgcaggatgactatggagacaagaagcacgtcacactttacccgctgaggcctgacctgctcgccggcttatccaccatgcaggagttgccatgttccccgagtaccgcgatctgatcacccgtctcaaggctgaaaacaagacctttgcccgcctgttcgacgagcacaacgacctcgaccagcgggtgaagaacatcgaggcgcacatcgtgccgggcaccgacagcgaggtggaaaacctgaagaagcagaagctgcagctcaaggatcgcctctacgacatgctcaaggaggcatccgtcgcctgacctctgcgcgccccgctcgcggggcgctacctgccgcgtcgttgcggacaacgctcgacgcgcaatcgccgggcaagcgcagtaaaatgccgcgctttcgatacccctgcgagtcccgcgccatgaacacccccaaccgcaccgagctgctgtcgcctgccggcacgctgaaatccatgcgctacgccttcgcctacggcgccgatgcggtgtacgccgggcagccacgctacagcctgcgcgtacgcaacaacgagttcgaccacgccaacctgaaggtcggcatcgacgaggcccacgcgctgggcaagcagttctacgtggtggtcaacatcgccccgcacaacgccaagctcaagaccttcatcaaggacctggagccggtggtggcgatgggcccggacgcgctgatcatgtccgacccgggcctgatcatgctggtgcgccagcattttccgcagcagaccatccacctctcggtacaggccaacgcggtgaactgggcgacggtgaagttctgggaaagccagggcgtctcccgggtgatcctctcccgcgagctgtcgctggaggagatcggcgagatacgcgagcaggtgccgggcatggagctggaagtgttcgtccatggtgcgctgtgcatggcctattccggtcgctgcctgctgtcgggctacatcaacaagcgcgaccccaaccagggcacctgcaccaatgcctgccgctgggaatacaagacccacgaggcaaaggaggacgaactgggcaactcggtgcacctctacgagcccatcgccgtgcagcaggtcgaggcgcagggcaacccgaccctgggcgtcggagcgcccaccgacaaggtgttcctgctcgaggatgtctcgcggcccggcgagttcatggaggcgaccgaggacgagcacggcacctacatcatgaactccaaggacctgcgcgccgtgcagcatgtcgagcggctggtgcagatgggcgtgcactcgctgaagatcgaaggccgcaccaagagccactactacgtggcgcgcaccgcgcaggtctaccgcaaggccatcgatgatgcactggccggccggccgttcgacaagtcgttgatggacaccctcgaatccctggcccaccgcggctataccgagggtttcctgcgccgtcacgtgcacgacgaataccagaactacgagcgcggcttctcgctctccgagcgccagcagttcgtcggcgagctgaccggcgagcggcgcaacggcctggccgaagtgaaagtgaaaaaccgcttcgcggtcggcgacaggctggagctgatgacaccgcagggcaatctcaacctgcgcctggagaccctggaaagcagccgcggcgaagccatcgaggttgcgccgggcgacggccacaccgtctatctgccggtcccgcaggacgtggacctgcacttcggcctgctgatgcgcgagctggagggcggcagcagcacccgcggctga

SEQ ID NO: 33 - DNA, 516 bp, Pseudomonas stutzeri
  source 1..516: mol_type = genomic DNA
atgctccgtcgcccaaccgacggcgacggttacaaccttcatcagctggtggcgcgctgccagcccctcgataccaattcggtctactgcaacctgctgcagtgttccgatttcgctgacaccgccatcgccgcagagaacgcccaaggcgagctggtcggtttcatctcgggttaccgccccccttcgcggccggacacgctgttcgtctggcaggtcgccgtcgacagctcgatgcgcggtcaggggctggccctgcgcatgctgctggcactgaccgcccgggtcgctcgcgagtacggcgtgcgttacatggaaaccaccatctcgccggacaacggggcgtcacaggcgctgttcaagcgggccttcgaccgcctcgatgccaactgcacgacgcgcacgctgttcgcccgcgacacgcatttcgccggtcagcacgaggacgaggtgctctaccgcgccggcccgttcaccgtttcccatctagaagaagagctcaaggagcacgcatga

SEQ ID NO: 34 - DNA, 1278 bp, Pseudomonas stutzeri
  source 1..1278: mol_type = genomic DNA
atgaaaacttttgaactgaatgaatccagggttcgcagctactgccgttccttccccgtggtcttcaagcaggcccagggcgccgaactggtcactcaggacggcaagcgctacatcgacttcctcgctggtgccggcacgctcaactacgggcacaaccacccggtgctcaagcaggcgctgctcgagtacatcgagagcgacggcatcacccacggcctggacatgtacaccgaagccaaggagcgtttcctcgaaaccttcaaccggctgatcctcgagccgcgcggcatgggcgactaccgcatgcagttcaccggcccgaccggcaccaacgcggtcgaggcggcgatgaagctggcgcgcaaggtcaccgggcgcaacaacatcatcagtttcaccaacggcttccacggctgcagcattggcgcgctggccgccaccggcaaccagcatcaccgcggcggctccggcatcggcctcaccgatgtcagccgcatgccgtacgccaactatttcggcgacaagaccaacactatcggcatgatggacaagctcttgtccgacccatccagcgggatcgacaagcccgccgcggtgatcgtcgaggtggtgcagggcgaaggcggcctgaacaccgcgtcggccgaatggatgcgcaagctcgagaagctctgccgcaagcacgaaatgctgctgatcgtcgatgacatccaggccggctgcggccgcaccgggactttcttcagcttcgaagagatgggcatccagccggatatcgtaacgctgtccaagtcgctgtccggctacggcctgccgttcgccatggtgttgctgcgccaggagctggaccagtggaagcccggcgaacacaacggcaccttccgcggcaacaaccatgcattcgtcacggcggccgcggcggtcgagcacttctggcagaacgacacgttcgccaacagcgtgaaggccaagggcaagcgcatcgccgacggcatgcagcgcatcatccgtcgccacggcccggattcgctgtttctcaagggccgcgggatgatgatcggcattagctgccccgatggcgagattgccgccgcagtgtgccgccatgccttcgaaaacggcctggtgatcgagaccagcggcgcccacagcgaagtggtcaagtgcctctgcccgctgatcatcagcgatgagcagatcgacaaggcgctttccatcctcgacaaggcctttgccgccgtgatgagcgagcagaccgagaaccaagcttcctga

SEQ ID NO: 35 - DNA, 402 bp, Pseudomonas stutzeri
  source 1..402: mol_type = genomic DNA
atgatcgtcagaaccctcgccgagtgcgaaaagaccgaccgcaaggtccacagccagaccggcacttgggacagcacgcgcatgctgctcaaggacgacaaggtgggattctccttccacatcaccaccatctacgccggcagcgagacgcacatccactaccagaaccacttcgagtcggtgtactgcatcagcggcaatggcgagatcgaaaccatcgccgacggcaagatttacaagatcgagccgggcacgctgtacgtgctggacaagcatgacgagcacctgctgcgcggtggcagcgaagacatgaagctggcctgcgtcttcaacccgccgctcaacgggcgcgaagtgcatgacgaaagcggcgtctatccgctggaggccgaaaccgtctga